European Patent Specification EP 3 352 760 B1, published March 11, 2026. Title: CD3 BINDING POLYPEPTIDES. Applicant: APTEVO RESEARCH AND DEVELOPMENT LLC Tan, Philip Blankenship, John W. The sequence listing filed with the application follows.

SEQUENCE LISTING (222 sequences)

SEQ ID NO: 1 - DNA, 1560 bp, Artificial Sequence
  Fc DRA222 (TSC311 or TSC312) CD3-binding domain
atggaagcaccagcgcagcttctcttcctcctgctactctggctcccagataccaccggtgagcccaaatcttctgacaaaactcacacatgcccaccgtgcccagcacctgaagccgcgggtgcaccgtcagtcttcctcttccccccaaaacccaaggacaccctcatgatctcccggacccctgaggtcacatgcgtggtggtggacgtgagccacgaagaccctgaggtcaagttcaactggtacgtggacggcgtggaggtgcataatgccaagacaaagccgcgggaggagcagtacaacagcacgtaccgtgtggtcagcgtcctcaccgtcctgcaccaggactggctgaatggcaaggcatacgcgtgcgcggtctccaacaaagccctcccagcccccatcgagaaaaccatctccaaagccaaagggcagccccgagaaccacaggtgtacaccctgcccccatcccgggatgagctgaccaagaaccaggtcagcctgacctgcctggtcaaaggcttctatccaagcgacatcgccgtggagtgggagagcaatgggcagccggagaacaactacaagaccacgcctcccgtgctggactccgacggctccttcttcctctacagcaagctcaccgtggacaagagcaggtggcagcaggggaacgtcttctcatgctccgtgatgcatgaggctctgcacaaccactacacgcagaagagcctctccctgtctccgggtcagaggcacaacaattcttccctgaatacaggaactcagatggcaggtcattctccgaattctcaggtccagctggtggagtctgggggcggagtggtgcagcctgggcggtcactgaggctgtcctgcaaggcttctggctacacctttactagatctacgatgcactgggtaaggcaggcccctggacaaggtctggaatggattggatacattaatcctagcagtgcttatactaattacaatcagaaattcaaggacaggttcacaatcagcgcagacaaatccaagagcacagccttcctgcagatggacagcctgaggcccgaggacaccggcgtctatttctgtgcacggccccaagtccactatgattacaacgggtttccttactggggccaagggactcccgtcactgtctctagcggtggcggagggtctgggggtggcggatccggaggtggtggctctgcacaagacatccagatgacccagtctccaagcagcctgtctgcaagcgtgggggacagggtcaccatgacctgcagtgccagctcaagtgtaagttacatgaactggtaccagcagaagccgggcaaggcccccaaaagatggatttatgactcatccaaactggcttctggagtccctgctcgcttcagtggcagtgggtctgggaccgactataccctcacaatcagcagcctgcagcccgaagatttcgccacttattactgccagcagtggagtcgtaacccacccacgttcggaggggggaccaagctacaaattacatcctccagctaa

SEQ ID NO: 2 - protein, 499 aa, Artificial Sequence
  Fc DRA222 (TSC311 or TSC312) CD3-binding domain
EPKSSDKTHTCPPCPAPEAAGAPSVFLFPPKPKDTLMISRTPEVTCVVVDVSHEDPEVKFNWYVDGVEVHNAKTKPREEQYNSTYRVVSVLTVLHQDWLNGKAYACAVSNKALPAPIEKTISKAKGQPREPQVYTLPPSRDELTKNQVSLTCLVKGFYPSDIAVEWESNGQPENNYKTTPPVLDSDGSFFLYSKLTVDKSRWQQGNVFSCSVMHEALHNHYTQKSLSLSPGQRHNNSSLNTGTQMAGHSPNSQVQLVESGGGVVQPGRSLRLSCKASGYTFTRSTMHWVRQAPGQGLEWIGYINPSSAYTNYNQKFKDRFTISADKSKSTAFLQMDSLRPEDTGVYFCARPQVHYDYNGFPYWGQGTPVTVSSGGGGSGGGGSGGGGSAQDIQMTQSPSSLSASVGDRVTMTCSASSSVSYMNWYQQKPGKAPKRWIYDSSKLASGVPARFSGSGSGTDYTLTISSLQPEDFATYYCQQWSRNPPTFGGGTKLQITSSS

SEQ ID NO: 3 - DNA, 1569 bp, Artificial Sequence
  Fc H7L1 (TSC313) CD3-binding domain
atggaagcaccagcgcagcttctcttcctcctgctactctggctcccagataccaccggtgagcccaaatcttctgacaaaactcacacatgcccaccgtgcccagcacctgaagccgcgggtgcaccgtcagtcttcctcttccccccaaaacccaaggacaccctcatgatctcccggacccctgaggtcacatgcgtggtggtggacgtgagccacgaagaccctgaggtcaagttcaactggtacgtggacggcgtggaggtgcataatgccaagacaaagccgcgggaggagcagtacaacagcacgtaccgtgtggtcagcgtcctcaccgtcctgcaccaggactggctgaatggcaaggcatacgcgtgcgcggtctccaacaaagccctcccagcccccatcgagaaaaccatctccaaagccaaagggcagccccgagaaccacaggtgtacaccctgcccccatcccgggatgagctgaccaagaaccaggtcagcctgacctgcctggtcaaaggcttctatccaagcgacatcgccgtggagtgggagagcaatgggcagccggagaacaactacaagaccacgcctcccgtgctggactccgacggctccttcttcctctacagcaagctcaccgtggacaagagcaggtggcagcaggggaacgtcttctcatgctccgtgatgcatgaggctctgcacaaccactacacgcagaagagcctctccctgtctccgggtcagaggcacaacaattcttccctgaatacaggaactcagatggcaggtcattctccgaattctcaggtgcagctggtgcagtctggggctgaggtgaagaagcctggggcctcagtgaaggtctcctgcaaggcttctggatacaccttcaccagatctacgatgcactgggtgcgacaggcccctggacaagggcttgagtggatgggatacattaatcctagcagtgcttatactaattacaatcagaaattcaaggacagggtcaccatgaccagggacacgtccatcagcacagcctacatggagctgagcaggctgagatctgacgacacggccgtgtattactgtgcgagaccccaagtccactatgattacaacgggtttccttactggggccaaggaaccctggtcaccgtctcctcaggtggaggcggttcaggcggaggtggatccggcggtggcggatcgggtggcggcggatctgacatccagatgacccagtctccaagcagcctgtctgcaagcgtgggggacagggtcaccatgacctgcagtgccagctcaagtgtaagttacatgaactggtaccagcagaagccgggcaaggcccccaaaagatggatttatgactcatccaaactggcttctggagtccctgctcgcttcagtggcagtgggtctgggaccgactataccctcacaatcagcagcctgcagcccgaagatttcgccacttattactgccagcagtggagtcgtaacccacccacgttcggaggggggaccaagctacaaattacatcctccagctaa

SEQ ID NO: 4 - protein, 502 aa, Artificial Sequence
  Fc H7L1 (TSC313) CD3-binding domain
EPKSSDKTHTCPPCPAPEAAGAPSVFLFPPKPKDTLMISRTPEVTCVVVDVSHEDPEVKFNWYVDGVEVHNAKTKPREEQYNSTYRVVSVLTVLHQDWLNGKAYACAVSNKALPAPIEKTISKAKGQPREPQVYTLPPSRDELTKNQVSLTCLVKGFYPSDIAVEWESNGQPENNYKTTPPVLDSDGSFFLYSKLTVDKSRWQQGNVFSCSVMHEALHNHYTQKSLSLSPGQRHNNSSLNTGTQMAGHSPNSQVQLVQSGAEVKKPGASVKVSCKASGYTFTRSTMHWVRQAPGQGLEWMGYINPSSAYTNYNQKFKDRVTMTRDTSISTAYMELSRLRSDDTAVYYCARPQVHYDYNGFPYWGQGTLVTVSSGGGGSGGGGSGGGGSGGGGSDIQMTQSPSSLSASVGDRVTMTCSASSSVSYMNWYQQKPGKAPKRWIYDSSKLASGVPARFSGSGSGTDYTLTISSLQPEDFATYYCQQWSRNPPTFGGGTKLQITSSS

SEQ ID NO: 5 - DNA, 1572 bp, Artificial Sequence
  H7L4 (TSC314) CD3-binding domain
atggaagcaccagcgcagcttctcttcctcctgctactctggctcccagataccaccggtgagcccaaatcttctgacaaaactcacacatgcccaccgtgcccagcacctgaagccgcgggtgcaccgtcagtcttcctcttccccccaaaacccaaggacaccctcatgatctcccggacccctgaggtcacatgcgtggtggtggacgtgagccacgaagaccctgaggtcaagttcaactggtacgtggacggcgtggaggtgcataatgccaagacaaagccgcgggaggagcagtacaacagcacgtaccgtgtggtcagcgtcctcaccgtcctgcaccaggactggctgaatggcaaggcatacgcgtgcgcggtctccaacaaagccctcccagcccccatcgagaaaaccatctccaaagccaaagggcagccccgagaaccacaggtgtacaccctgcccccatcccgggatgagctgaccaagaaccaggtcagcctgacctgcctggtcaaaggcttctatccaagcgacatcgccgtggagtgggagagcaatgggcagccggagaacaactacaagaccacgcctcccgtgctggactccgacggctccttcttcctctacagcaagctcaccgtggacaagagcaggtggcagcaggggaacgtcttctcatgctccgtgatgcatgaggctctgcacaaccactacacgcagaagagcctctccctgtctccgggtcagaggcacaacaattcttccctgaatacaggaactcagatggcaggtcattctccgaattctcaggtgcagctggtgcagtctggggctgaggtgaagaagcctggggcctcagtgaaggtctcctgcaaggcttctggatacaccttcaccagatctacgatgcactgggtgcgacaggcccctggacaagggcttgagtggatgggatacattaatcctagcagtgcttatactaattacaatcagaaattcaaggacagggtcaccatgaccagggacacgtccatcagcacagcctacatggagctgagcaggctgagatctgacgacacggccgtgtattactgtgcgagaccccaagtccactatgattacaacgggtttccttactggggccaaggaaccctggtcaccgtctcctcaggtggaggcggttcaggcggaggtggatccggcggtggcggatcgggtggcggcggatctgaaattgtgttgacacagtctccagccaccctgtctttgtctccaggggaaagagccaccctctcctgcagtgccagctcaagtgtaagttacatgaactggtaccaacagaaacctggccaggctcccaggctcctcatctatgactcatccaaactggcttctggcatcccagccaggttcagtggcagtgggtctgggacagacttcactctcaccatcagcagcctagagcctgaagattttgcagtttattactgtcagcagtggagtcgtaacccacccactttcggcggagggaccaaggtggagatcaaacggtcctccagctaa

SEQ ID NO: 6 - protein, 503 aa, Artificial Sequence
  Fc H7L4 (TSC314) CD3-binding domain
EPKSSDKTHTCPPCPAPEAAGAPSVFLFPPKPKDTLMISRTPEVTCVVVDVSHEDPEVKFNWYVDGVEVHNAKTKPREEQYNSTYRVVSVLTVLHQDWLNGKAYACAVSNKALPAPIEKTISKAKGQPREPQVYTLPPSRDELTKNQVSLTCLVKGFYPSDIAVEWESNGQPENNYKTTPPVLDSDGSFFLYSKLTVDKSRWQQGNVFSCSVMHEALHNHYTQKSLSLSPGQRHNNSSLNTGTQMAGHSPNSQVQLVQSGAEVKKPGASVKVSCKASGYTFTRSTMHWVRQAPGQGLEWMGYINPSSAYTNYNQKFKDRVTMTRDTSISTAYMELSRLRSDDTAVYYCARPQVHYDYNGFPYWGQGTLVTVSSGGGGSGGGGSGGGGSGGGGSEIVLTQSPATLSLSPGERATLSCSASSSVSYMNWYQQKPGQAPRLLIYDSSKLASGIPARFSGSGSGTDFTLTISSLEPEDFAVYYCQQWSRNPPTFGGGTKVEIKRSSS

SEQ ID NO: 7 - DNA, 1572 bp, Artificial Sequence
  Fc H7L5 (TSC315) CD3-binding domain
atggaagcaccagcgcagcttctcttcctcctgctactctggctcccagataccaccggtgagcccaaatcttctgacaaaactcacacatgcccaccgtgcccagcacctgaagccgcgggtgcaccgtcagtcttcctcttccccccaaaacccaaggacaccctcatgatctcccggacccctgaggtcacatgcgtggtggtggacgtgagccacgaagaccctgaggtcaagttcaactggtacgtggacggcgtggaggtgcataatgccaagacaaagccgcgggaggagcagtacaacagcacgtaccgtgtggtcagcgtcctcaccgtcctgcaccaggactggctgaatggcaaggcatacgcgtgcgcggtctccaacaaagccctcccagcccccatcgagaaaaccatctccaaagccaaagggcagccccgagaaccacaggtgtacaccctgcccccatcccgggatgagctgaccaagaaccaggtcagcctgacctgcctggtcaaaggcttctatccaagcgacatcgccgtggagtgggagagcaatgggcagccggagaacaactacaagaccacgcctcccgtgctggactccgacggctccttcttcctctacagcaagctcaccgtggacaagagcaggtggcagcaggggaacgtcttctcatgctccgtgatgcatgaggctctgcacaaccactacacgcagaagagcctctccctgtctccgggtcagaggcacaacaattcttccctgaatacaggaactcagatggcaggtcattctccgaattctcaggtgcagctggtgcagtctggggctgaggtgaagaagcctggggcctcagtgaaggtctcctgcaaggcttctggatacaccttcaccagatctacgatgcactgggtgcgacaggcccctggacaagggcttgagtggatgggatacattaatcctagcagtgcttatactaattacaatcagaaattcaaggacagggtcaccatgaccagggacacgtccatcagcacagcctacatggagctgagcaggctgagatctgacgacacggccgtgtattactgtgcgagaccccaagtccactatgattacaacgggtttccttactggggccaaggaaccctggtcaccgtctcctcaggtggaggcggttcaggcggaggtggatccggcggtggcggatcgggtggcggcggatctgacatccagatgacccagtctccatcctccctgtctgcatctgtaggagacagagtcaccatcacttgcagtgccagctcaagtgtaagttacatgaactggtatcagcagaaaccagggaaagcccctaagctcctgatctatgactcatccaaactggcttctggggtcccatcaaggttcagtggcagtggatctgggacagatttcactctcaccatcagcagtctgcaacctgaagattttgcaacttactactgtcaacagtggagtcgtaacccacccactttcggcggagggaccaaggtggagatcaaacggtcctccagctaa

SEQ ID NO: 8 - protein, 503 aa, Artificial Sequence
  Fc H7L5 (TSC315) CD3-binding domain
EPKSSDKTHTCPPCPAPEAAGAPSVFLFPPKPKDTLMISRTPEVTCVVVDVSHEDPEVKFNWYVDGVEVHNAKTKPREEQYNSTYRVVSVLTVLHQDWLNGKAYACAVSNKALPAPIEKTISKAKGQPREPQVYTLPPSRDELTKNQVSLTCLVKGFYPSDIAVEWESNGQPENNYKTTPPVLDSDGSFFLYSKLTVDKSRWQQGNVFSCSVMHEALHNHYTQKSLSLSPGQRHNNSSLNTGTQMAGHSPNSQVQLVQSGAEVKKPGASVKVSCKASGYTFTRSTMHWVRQAPGQGLEWMGYINPSSAYTNYNQKFKDRVTMTRDTSISTAYMELSRLRSDDTAVYYCARPQVHYDYNGFPYWGQGTLVTVSSGGGGSGGGGSGGGGSGGGGSDIQMTQSPSSLSASVGDRVTITCSASSSVSYMNWYQQKPGKAPKLLIYDSSKLASGVPSRFSGSGSGTDFTLTISSLQPEDFATYYCQQWSRNPPTFGGGTKVEIKRSSS

SEQ ID NO: 9 - DNA, 1569 bp, Artificial Sequence
  Fc H8L1 (TSC316) CD3-binding domain
atggaagcaccagcgcagcttctcttcctcctgctactctggctcccagataccaccggtgagcccaaatcttctgacaaaactcacacatgcccaccgtgcccagcacctgaagccgcgggtgcaccgtcagtcttcctcttccccccaaaacccaaggacaccctcatgatctcccggacccctgaggtcacatgcgtggtggtggacgtgagccacgaagaccctgaggtcaagttcaactggtacgtggacggcgtggaggtgcataatgccaagacaaagccgcgggaggagcagtacaacagcacgtaccgtgtggtcagcgtcctcaccgtcctgcaccaggactggctgaatggcaaggcatacgcgtgcgcggtctccaacaaagccctcccagcccccatcgagaaaaccatctccaaagccaaagggcagccccgagaaccacaggtgtacaccctgcccccatcccgggatgagctgaccaagaaccaggtcagcctgacctgcctggtcaaaggcttctatccaagcgacatcgccgtggagtgggagagcaatgggcagccggagaacaactacaagaccacgcctcccgtgctggactccgacggctccttcttcctctacagcaagctcaccgtggacaagagcaggtggcagcaggggaacgtcttctcatgctccgtgatgcatgaggctctgcacaaccactacacgcagaagagcctctccctgtctccgggtcagaggcacaacaattcttccctgaatacaggaactcagatggcaggtcattctccgaattctcaggtgcagctggtgcagtctggggctgaggtgaagaagcctggggcctcagtgaaggtttcctgcaaggcatctggatacaccttcaccagatctacgatgcactgggtgcgacaggcccctggacaagggcttgagtggatgggatacattaatcctagcagtgcttatactaattacaatcagaaattcaaggacagagtcaccatgaccagggacacgtccacgagcacagtctacatggagctgagcagcctgagatctgaggacacggccgtgtattactgtgctagaccccaagtccactatgattacaacgggtttccttactggggccaaggaaccctggtcaccgtctcctcaggtggaggcggttcaggcggaggtggatccggcggtggcggatcgggtggcggcggatctgacatccagatgacccagtctccaagcagcctgtctgcaagcgtgggggacagggtcaccatgacctgcagtgccagctcaagtgtaagttacatgaactggtaccagcagaagccgggcaaggcccccaaaagatggatttatgactcatccaaactggcttctggagtccctgctcgcttcagtggcagtgggtctgggaccgactataccctcacaatcagcagcctgcagcccgaagatttcgccacttattactgccagcagtggagtcgtaacccacccacgttcggaggggggaccaagctacaaattacatcctccagctaa

SEQ ID NO: 10 - protein, 502 aa, Artificial Sequence
  Fc H8L1 (TSC316) CD3-binding domain
EPKSSDKTHTCPPCPAPEAAGAPSVFLFPPKPKDTLMISRTPEVTCVVVDVSHEDPEVKFNWYVDGVEVHNAKTKPREEQYNSTYRVVSVLTVLHQDWLNGKAYACAVSNKALPAPIEKTISKAKGQPREPQVYTLPPSRDELTKNQVSLTCLVKGFYPSDIAVEWESNGQPENNYKTTPPVLDSDGSFFLYSKLTVDKSRWQQGNVFSCSVMHEALHNHYTQKSLSLSPGQRHNNSSLNTGTQMAGHSPNSQVQLVQSGAEVKKPGASVKVSCKASGYTFTRSTMHWVRQAPGQGLEWMGYINPSSAYTNYNQKFKDRVTMTRDTSTSTVYMELSSLRSEDTAVYYCARPQVHYDYNGFPYWGQGTLVTVSSGGGGSGGGGSGGGGSGGGGSDIQMTQSPSSLSASVGDRVTMTCSASSSVSYMNWYQQKPGKAPKRWIYDSSKLASGVPARFSGSGSGTDYTLTISSLQPEDFATYYCQQWSRNPPTFGGGTKLQITSSS

SEQ ID NO: 11 - DNA, 1572 bp, Artificial Sequence
  Fc H8L4 (TSC317) CD3-binding domain
atggaagcaccagcgcagcttctcttcctcctgctactctggctcccagataccaccggtgagcccaaatcttctgacaaaactcacacatgcccaccgtgcccagcacctgaagccgcgggtgcaccgtcagtcttcctcttccccccaaaacccaaggacaccctcatgatctcccggacccctgaggtcacatgcgtggtggtggacgtgagccacgaagaccctgaggtcaagttcaactggtacgtggacggcgtggaggtgcataatgccaagacaaagccgcgggaggagcagtacaacagcacgtaccgtgtggtcagcgtcctcaccgtcctgcaccaggactggctgaatggcaaggcatacgcgtgcgcggtctccaacaaagccctcccagcccccatcgagaaaaccatctccaaagccaaagggcagccccgagaaccacaggtgtacaccctgcccccatcccgggatgagctgaccaagaaccaggtcagcctgacctgcctggtcaaaggcttctatccaagcgacatcgccgtggagtgggagagcaatgggcagccggagaacaactacaagaccacgcctcccgtgctggactccgacggctccttcttcctctacagcaagctcaccgtggacaagagcaggtggcagcaggggaacgtcttctcatgctccgtgatgcatgaggctctgcacaaccactacacgcagaagagcctctccctgtctccgggtcagaggcacaacaattcttccctgaatacaggaactcagatggcaggtcattctccgaattctcaggtgcagctggtgcagtctggggctgaggtgaagaagcctggggcctcagtgaaggtttcctgcaaggcatctggatacaccttcaccagatctacgatgcactgggtgcgacaggcccctggacaagggcttgagtggatgggatacattaatcctagcagtgcttatactaattacaatcagaaattcaaggacagagtcaccatgaccagggacacgtccacgagcacagtctacatggagctgagcagcctgagatctgaggacacggccgtgtattactgtgctagaccccaagtccactatgattacaacgggtttccttactggggccaaggaaccctggtcaccgtctcctcaggtggaggcggttcaggcggaggtggatccggcggtggcggatcgggtggcggcggatctgaaattgtgttgacacagtctccagccaccctgtctttgtctccaggggaaagagccaccctctcctgcagtgccagctcaagtgtaagttacatgaactggtaccaacagaaacctggccaggctcccaggctcctcatctatgactcatccaaactggcttctggcatcccagccaggttcagtggcagtgggtctgggacagacttcactctcaccatcagcagcctagagcctgaagattttgcagtttattactgtcagcagtggagtcgtaacccacccactttcggcggagggaccaaggtggagatcaaacggtcctccagctaa

SEQ ID NO: 12 - protein, 503 aa, Artificial Sequence
  Fc H8L4 (TSC317) CD3-binding domain
EPKSSDKTHTCPPCPAPEAAGAPSVFLFPPKPKDTLMISRTPEVTCVVVDVSHEDPEVKFNWYVDGVEVHNAKTKPREEQYNSTYRVVSVLTVLHQDWLNGKAYACAVSNKALPAPIEKTISKAKGQPREPQVYTLPPSRDELTKNQVSLTCLVKGFYPSDIAVEWESNGQPENNYKTTPPVLDSDGSFFLYSKLTVDKSRWQQGNVFSCSVMHEALHNHYTQKSLSLSPGQRHNNSSLNTGTQMAGHSPNSQVQLVQSGAEVKKPGASVKVSCKASGYTFTRSTMHWVRQAPGQGLEWMGYINPSSAYTNYNQKFKDRVTMTRDTSTSTVYMELSSLRSEDTAVYYCARPQVHYDYNGFPYWGQGTLVTVSSGGGGSGGGGSGGGGSGGGGSEIVLTQSPATLSLSPGERATLSCSASSSVSYMNWYQQKPGQAPRLLIYDSSKLASGIPARFSGSGSGTDFTLTISSLEPEDFAVYYCQQWSRNPPTFGGGTKVEIKRSSS

SEQ ID NO: 13 - DNA, 1572 bp, Artificial Sequence
  Fc H8L5 (TSC318) CD3-binding domain
atggaagcaccagcgcagcttctcttcctcctgctactctggctcccagataccaccggtgagcccaaatcttctgacaaaactcacacatgcccaccgtgcccagcacctgaagccgcgggtgcaccgtcagtcttcctcttccccccaaaacccaaggacaccctcatgatctcccggacccctgaggtcacatgcgtggtggtggacgtgagccacgaagaccctgaggtcaagttcaactggtacgtggacggcgtggaggtgcataatgccaagacaaagccgcgggaggagcagtacaacagcacgtaccgtgtggtcagcgtcctcaccgtcctgcaccaggactggctgaatggcaaggcatacgcgtgcgcggtctccaacaaagccctcccagcccccatcgagaaaaccatctccaaagccaaagggcagccccgagaaccacaggtgtacaccctgcccccatcccgggatgagctgaccaagaaccaggtcagcctgacctgcctggtcaaaggcttctatccaagcgacatcgccgtggagtgggagagcaatgggcagccggagaacaactacaagaccacgcctcccgtgctggactccgacggctccttcttcctctacagcaagctcaccgtggacaagagcaggtggcagcaggggaacgtcttctcatgctccgtgatgcatgaggctctgcacaaccactacacgcagaagagcctctccctgtctccgggtcagaggcacaacaattcttccctgaatacaggaactcagatggcaggtcattctccgaattctcaggtgcagctggtgcagtctggggctgaggtgaagaagcctggggcctcagtgaaggtttcctgcaaggcatctggatacaccttcaccagatctacgatgcactgggtgcgacaggcccctggacaagggcttgagtggatgggatacattaatcctagcagtgcttatactaattacaatcagaaattcaaggacagagtcaccatgaccagggacacgtccacgagcacagtctacatggagctgagcagcctgagatctgaggacacggccgtgtattactgtgctagaccccaagtccactatgattacaacgggtttccttactggggccaaggaaccctggtcaccgtctcctcaggtggaggcggttcaggcggaggtggatccggcggtggcggatcgggtggcggcggatctgacatccagatgacccagtctccatcctccctgtctgcatctgtaggagacagagtcaccatcacttgcagtgccagctcaagtgtaagttacatgaactggtatcagcagaaaccagggaaagcccctaagctcctgatctatgactcatccaaactggcttctggggtcccatcaaggttcagtggcagtggatctgggacagatttcactctcaccatcagcagtctgcaacctgaagattttgcaacttactactgtcaacagtggagtcgtaacccacccactttcggcggagggaccaaggtggagatcaaacggtcctccagctaa

SEQ ID NO: 14 - protein, 503 aa, Artificial Sequence
  Fc H8L5 (TSC318) CD3-binding domain
EPKSSDKTHTCPPCPAPEAAGAPSVFLFPPKPKDTLMISRTPEVTCVVVDVSHEDPEVKFNWYVDGVEVHNAKTKPREEQYNSTYRVVSVLTVLHQDWLNGKAYACAVSNKALPAPIEKTISKAKGQPREPQVYTLPPSRDELTKNQVSLTCLVKGFYPSDIAVEWESNGQPENNYKTTPPVLDSDGSFFLYSKLTVDKSRWQQGNVFSCSVMHEALHNHYTQKSLSLSPGQRHNNSSLNTGTQMAGHSPNSQVQLVQSGAEVKKPGASVKVSCKASGYTFTRSTMHWVRQAPGQGLEWMGYINPSSAYTNYNQKFKDRVTMTRDTSTSTVYMELSSLRSEDTAVYYCARPQVHYDYNGFPYWGQGTLVTVSSGGGGSGGGGSGGGGSGGGGSDIQMTQSPSSLSASVGDRVTITCSASSSVSYMNWYQQKPGKAPKLLIYDSSKLASGVPSRFSGSGSGTDFTLTISSLQPEDFATYYCQQWSRNPPTFGGGTKVEIKRSSS

SEQ ID NO: 15 - DNA, 1569 bp, Artificial Sequence
  Fc H9L1 (TSC319) CD3-binding domain
atggaagcaccagcgcagcttctcttcctcctgctactctggctcccagataccaccggtgagcccaaatcttctgacaaaactcacacatgcccaccgtgcccagcacctgaagccgcgggtgcaccgtcagtcttcctcttccccccaaaacccaaggacaccctcatgatctcccggacccctgaggtcacatgcgtggtggtggacgtgagccacgaagaccctgaggtcaagttcaactggtacgtggacggcgtggaggtgcataatgccaagacaaagccgcgggaggagcagtacaacagcacgtaccgtgtggtcagcgtcctcaccgtcctgcaccaggactggctgaatggcaaggcatacgcgtgcgcggtctccaacaaagccctcccagcccccatcgagaaaaccatctccaaagccaaagggcagccccgagaaccacaggtgtacaccctgcccccatcccgggatgagctgaccaagaaccaggtcagcctgacctgcctggtcaaaggcttctatccaagcgacatcgccgtggagtgggagagcaatgggcagccggagaacaactacaagaccacgcctcccgtgctggactccgacggctccttcttcctctacagcaagctcaccgtggacaagagcaggtggcagcaggggaacgtcttctcatgctccgtgatgcatgaggctctgcacaaccactacacgcagaagagcctctccctgtctccgggtcagaggcacaacaattcttccctgaatacaggaactcagatggcaggtcattctccgaattctcaggtccagcttgtgcagtctggggctgaggtgaagaagcctggggcctcagtgaaggtttcctgcaaggcttctggctacacctttactagatctacgatgcattgggtgcgccaggcccccggacaaaggcttgagtggatgggatacattaatcctagcagtgcttatactaattacaatcagaaattcaaggacagggtcaccattaccagggacacatccgcgagcacagcctacatggagctgagcagcctgagatctgaagacacggctgtgtattactgtgcgagaccccaagtccactatgattacaacgggtttccttactggggccaaggaaccctggtcaccgtctcctcaggtggaggcggttcaggcggaggtggatccggcggtggcggatcgggtggcggcggatctgacatccagatgacccagtctccaagcagcctgtctgcaagcgtgggggacagggtcaccatgacctgcagtgccagctcaagtgtaagttacatgaactggtaccagcagaagccgggcaaggcccccaaaagatggatttatgactcatccaaactggcttctggagtccctgctcgcttcagtggcagtgggtctgggaccgactataccctcacaatcagcagcctgcagcccgaagatttcgccacttattactgccagcagtggagtcgtaacccacccacgttcggaggggggaccaagctacaaattacatcctccagctaa

SEQ ID NO: 16 - protein, 502 aa, Artificial Sequence
  Fc H9L1 (TSC319) CD3-binding domain
EPKSSDKTHTCPPCPAPEAAGAPSVFLFPPKPKDTLMISRTPEVTCVVVDVSHEDPEVKFNWYVDGVEVHNAKTKPREEQYNSTYRVVSVLTVLHQDWLNGKAYACAVSNKALPAPIEKTISKAKGQPREPQVYTLPPSRDELTKNQVSLTCLVKGFYPSDIAVEWESNGQPENNYKTTPPVLDSDGSFFLYSKLTVDKSRWQQGNVFSCSVMHEALHNHYTQKSLSLSPGQRHNNSSLNTGTQMAGHSPNSQVQLVQSGAEVKKPGASVKVSCKASGYTFTRSTMHWVRQAPGQRLEWMGYINPSSAYTNYNQKFKDRVTITRDTSASTAYMELSSLRSEDTAVYYCARPQVHYDYNGFPYWGQGTLVTVSSGGGGSGGGGSGGGGSGGGGSDIQMTQSPSSLSASVGDRVTMTCSASSSVSYMNWYQQKPGKAPKRWIYDSSKLASGVPARFSGSGSGTDYTLTISSLQPEDFATYYCQQWSRNPPTFGGGTKLQITSSS

SEQ ID NO: 17 - DNA, 1572 bp, Artificial Sequence
  Fc H9L4 (TSC320) CD3-binding domain
atggaagcaccagcgcagcttctcttcctcctgctactctggctcccagataccaccggtgagcccaaatcttctgacaaaactcacacatgcccaccgtgcccagcacctgaagccgcgggtgcaccgtcagtcttcctcttccccccaaaacccaaggacaccctcatgatctcccggacccctgaggtcacatgcgtggtggtggacgtgagccacgaagaccctgaggtcaagttcaactggtacgtggacggcgtggaggtgcataatgccaagacaaagccgcgggaggagcagtacaacagcacgtaccgtgtggtcagcgtcctcaccgtcctgcaccaggactggctgaatggcaaggcatacgcgtgcgcggtctccaacaaagccctcccagcccccatcgagaaaaccatctccaaagccaaagggcagccccgagaaccacaggtgtacaccctgcccccatcccgggatgagctgaccaagaaccaggtcagcctgacctgcctggtcaaaggcttctatccaagcgacatcgccgtggagtgggagagcaatgggcagccggagaacaactacaagaccacgcctcccgtgctggactccgacggctccttcttcctctacagcaagctcaccgtggacaagagcaggtggcagcaggggaacgtcttctcatgctccgtgatgcatgaggctctgcacaaccactacacgcagaagagcctctccctgtctccgggtcagaggcacaacaattcttccctgaatacaggaactcagatggcaggtcattctccgaattctcaggtccagcttgtgcagtctggggctgaggtgaagaagcctggggcctcagtgaaggtttcctgcaaggcttctggctacacctttactagatctacgatgcattgggtgcgccaggcccccggacaaaggcttgagtggatgggatacattaatcctagcagtgcttatactaattacaatcagaaattcaaggacagggtcaccattaccagggacacatccgcgagcacagcctacatggagctgagcagcctgagatctgaagacacggctgtgtattactgtgcgagaccccaagtccactatgattacaacgggtttccttactggggccaaggaaccctggtcaccgtctcctcaggtggaggcggttcaggcggaggtggatccggcggtggcggatcgggtggcggcggatctgaaattgtgttgacacagtctccagccaccctgtctttgtctccaggggaaagagccaccctctcctgcagtgccagctcaagtgtaagttacatgaactggtaccaacagaaacctggccaggctcccaggctcctcatctatgactcatccaaactggcttctggcatcccagccaggttcagtggcagtgggtctgggacagacttcactctcaccatcagcagcctagagcctgaagattttgcagtttattactgtcagcagtggagtcgtaacccacccactttcggcggagggaccaaggtggagatcaaacggtcctccagctaa

SEQ ID NO: 18 - protein, 503 aa, Artificial Sequence
  Fc H9L4 (TSC320) CD3-binding domain
EPKSSDKTHTCPPCPAPEAAGAPSVFLFPPKPKDTLMISRTPEVTCVVVDVSHEDPEVKFNWYVDGVEVHNAKTKPREEQYNSTYRVVSVLTVLHQDWLNGKAYACAVSNKALPAPIEKTISKAKGQPREPQVYTLPPSRDELTKNQVSLTCLVKGFYPSDIAVEWESNGQPENNYKTTPPVLDSDGSFFLYSKLTVDKSRWQQGNVFSCSVMHEALHNHYTQKSLSLSPGQRHNNSSLNTGTQMAGHSPNSQVQLVQSGAEVKKPGASVKVSCKASGYTFTRSTMHWVRQAPGQRLEWMGYINPSSAYTNYNQKFKDRVTITRDTSASTAYMELSSLRSEDTAVYYCARPQVHYDYNGFPYWGQGTLVTVSSGGGGSGGGGSGGGGSGGGGSEIVLTQSPATLSLSPGERATLSCSASSSVSYMNWYQQKPGQAPRLLIYDSSKLASGIPARFSGSGSGTDFTLTISSLEPEDFAVYYCQQWSRNPPTFGGGTKVEIKRSSS

SEQ ID NO: 19 - DNA, 1572 bp, Artificial Sequence
  Fc H9L5 (TSC321) CD3-binding domain
atggaagcaccagcgcagcttctcttcctcctgctactctggctcccagataccaccggtgagcccaaatcttctgacaaaactcacacatgcccaccgtgcccagcacctgaagccgcgggtgcaccgtcagtcttcctcttccccccaaaacccaaggacaccctcatgatctcccggacccctgaggtcacatgcgtggtggtggacgtgagccacgaagaccctgaggtcaagttcaactggtacgtggacggcgtggaggtgcataatgccaagacaaagccgcgggaggagcagtacaacagcacgtaccgtgtggtcagcgtcctcaccgtcctgcaccaggactggctgaatggcaaggcatacgcgtgcgcggtctccaacaaagccctcccagcccccatcgagaaaaccatctccaaagccaaagggcagccccgagaaccacaggtgtacaccctgcccccatcccgggatgagctgaccaagaaccaggtcagcctgacctgcctggtcaaaggcttctatccaagcgacatcgccgtggagtgggagagcaatgggcagccggagaacaactacaagaccacgcctcccgtgctggactccgacggctccttcttcctctacagcaagctcaccgtggacaagagcaggtggcagcaggggaacgtcttctcatgctccgtgatgcatgaggctctgcacaaccactacacgcagaagagcctctccctgtctccgggtcagaggcacaacaattcttccctgaatacaggaactcagatggcaggtcattctccgaattctcaggtccagcttgtgcagtctggggctgaggtgaagaagcctggggcctcagtgaaggtttcctgcaaggcttctggctacacctttactagatctacgatgcattgggtgcgccaggcccccggacaaaggcttgagtggatgggatacattaatcctagcagtgcttatactaattacaatcagaaattcaaggacagggtcaccattaccagggacacatccgcgagcacagcctacatggagctgagcagcctgagatctgaagacacggctgtgtattactgtgcgagaccccaagtccactatgattacaacgggtttccttactggggccaaggaaccctggtcaccgtctcctcaggtggaggcggttcaggcggaggtggatccggcggtggcggatcgggtggcggcggatctgacatccagatgacccagtctccatcctccctgtctgcatctgtaggagacagagtcaccatcacttgcagtgccagctcaagtgtaagttacatgaactggtatcagcagaaaccagggaaagcccctaagctcctgatctatgactcatccaaactggcttctggggtcccatcaaggttcagtggcagtggatctgggacagatttcactctcaccatcagcagtctgcaacctgaagattttgcaacttactactgtcaacagtggagtcgtaacccacccactttcggcggagggaccaaggtggagatcaaacggtcctccagctaa

SEQ ID NO: 20 - protein, 503 aa, Artificial Sequence
  Fc H9L5 (TSC321) CD3-binding domain
EPKSSDKTHTCPPCPAPEAAGAPSVFLFPPKPKDTLMISRTPEVTCVVVDVSHEDPEVKFNWYVDGVEVHNAKTKPREEQYNSTYRVVSVLTVLHQDWLNGKAYACAVSNKALPAPIEKTISKAKGQPREPQVYTLPPSRDELTKNQVSLTCLVKGFYPSDIAVEWESNGQPENNYKTTPPVLDSDGSFFLYSKLTVDKSRWQQGNVFSCSVMHEALHNHYTQKSLSLSPGQRHNNSSLNTGTQMAGHSPNSQVQLVQSGAEVKKPGASVKVSCKASGYTFTRSTMHWVRQAPGQRLEWMGYINPSSAYTNYNQKFKDRVTITRDTSASTAYMELSSLRSEDTAVYYCARPQVHYDYNGFPYWGQGTLVTVSSGGGGSGGGGSGGGGSGGGGSDIQMTQSPSSLSASVGDRVTITCSASSSVSYMNWYQQKPGKAPKLLIYDSSKLASGVPSRFSGSGSGTDFTLTISSLQPEDFATYYCQQWSRNPPTFGGGTKVEIKRSSS

SEQ ID NO: 21 - DNA, 1569 bp, Artificial Sequence
  Fc H10L1 (TSC322) CD3-binding domain
atggaagcaccagcgcagcttctcttcctcctgctactctggctcccagataccaccggtgagcccaaatcttctgacaaaactcacacatgcccaccgtgcccagcacctgaagccgcgggtgcaccgtcagtcttcctcttccccccaaaacccaaggacaccctcatgatctcccggacccctgaggtcacatgcgtggtggtggacgtgagccacgaagaccctgaggtcaagttcaactggtacgtggacggcgtggaggtgcataatgccaagacaaagccgcgggaggagcagtacaacagcacgtaccgtgtggtcagcgtcctcaccgtcctgcaccaggactggctgaatggcaaggcatacgcgtgcgcggtctccaacaaagccctcccagcccccatcgagaaaaccatctccaaagccaaagggcagccccgagaaccacaggtgtacaccctgcccccatcccgggatgagctgaccaagaaccaggtcagcctgacctgcctggtcaaaggcttctatccaagcgacatcgccgtggagtgggagagcaatgggcagccggagaacaactacaagaccacgcctcccgtgctggactccgacggctccttcttcctctacagcaagctcaccgtggacaagagcaggtggcagcaggggaacgtcttctcatgctccgtgatgcatgaggctctgcacaaccactacacgcagaagagcctctccctgtctccgggtcagaggcacaacaattcttccctgaatacaggaactcagatggcaggtcattctccgaattctcaggtccagctggtgcaatctggggctgaggtgaagaagcctgggtcctcggtgaaggtctcctgcaaggcttctggaggcaccttcagcagatctacgatgcactgggtgcgacaggcccctggacaagggcttgagtggatgggatacattaatcctagcagtgcttatactaattacaatcagaaattcaaggacagagtcacgattaccgcggacaaatccacgagcacagcctacatggagctgagcagcctgagatctgaggacacggccgtgtattactgtgcgagaccccaagtccactatgattacaacgggtttccttactggggccaaggaaccctggtcaccgtctcctcaggtggaggcggttcaggcggaggtggatccggcggtggcggatcgggtggcggcggatctgacatccagatgacccagtctccaagcagcctgtctgcaagcgtgggggacagggtcaccatgacctgcagtgccagctcaagtgtaagttacatgaactggtaccagcagaagccgggcaaggcccccaaaagatggatttatgactcatccaaactggcttctggagtccctgctcgcttcagtggcagtgggtctgggaccgactataccctcacaatcagcagcctgcagcccgaagatttcgccacttattactgccagcagtggagtcgtaacccacccacgttcggaggggggaccaagctacaaattacatcctccagctaa

SEQ ID NO: 22 - protein, 502 aa, Artificial Sequence
  Fc H10L1 (TSC322) CD3-binding domain
EPKSSDKTHTCPPCPAPEAAGAPSVFLFPPKPKDTLMISRTPEVTCVVVDVSHEDPEVKFNWYVDGVEVHNAKTKPREEQYNSTYRVVSVLTVLHQDWLNGKAYACAVSNKALPAPIEKTISKAKGQPREPQVYTLPPSRDELTKNQVSLTCLVKGFYPSDIAVEWESNGQPENNYKTTPPVLDSDGSFFLYSKLTVDKSRWQQGNVFSCSVMHEALHNHYTQKSLSLSPGQRHNNSSLNTGTQMAGHSPNSQVQLVQSGAEVKKPGSSVKVSCKASGGTFSRSTMHWVRQAPGQGLEWMGYINPSSAYTNYNQKFKDRVTITADKSTSTAYMELSSLRSEDTAVYYCARPQVHYDYNGFPYWGQGTLVTVSSGGGGSGGGGSGGGGSGGGGSDIQMTQSPSSLSASVGDRVTMTCSASSSVSYMNWYQQKPGKAPKRWIYDSSKLASGVPARFSGSGSGTDYTLTISSLQPEDFATYYCQQWSRNPPTFGGGTKLQITSSS

SEQ ID NO: 23 - DNA, 1572 bp, Artificial Sequence
  Fc H10L4 (TSC323) CD3-binding domain
atggaagcaccagcgcagcttctcttcctcctgctactctggctcccagataccaccggtgagcccaaatcttctgacaaaactcacacatgcccaccgtgcccagcacctgaagccgcgggtgcaccgtcagtcttcctcttccccccaaaacccaaggacaccctcatgatctcccggacccctgaggtcacatgcgtggtggtggacgtgagccacgaagaccctgaggtcaagttcaactggtacgtggacggcgtggaggtgcataatgccaagacaaagccgcgggaggagcagtacaacagcacgtaccgtgtggtcagcgtcctcaccgtcctgcaccaggactggctgaatggcaaggcatacgcgtgcgcggtctccaacaaagccctcccagcccccatcgagaaaaccatctccaaagccaaagggcagccccgagaaccacaggtgtacaccctgcccccatcccgggatgagctgaccaagaaccaggtcagcctgacctgcctggtcaaaggcttctatccaagcgacatcgccgtggagtgggagagcaatgggcagccggagaacaactacaagaccacgcctcccgtgctggactccgacggctccttcttcctctacagcaagctcaccgtggacaagagcaggtggcagcaggggaacgtcttctcatgctccgtgatgcatgaggctctgcacaaccactacacgcagaagagcctctccctgtctccgggtcagaggcacaacaattcttccctgaatacaggaactcagatggcaggtcattctccgaattctcaggtccagctggtgcaatctggggctgaggtgaagaagcctgggtcctcggtgaaggtctcctgcaaggcttctggaggcaccttcagcagatctacgatgcactgggtgcgacaggcccctggacaagggcttgagtggatgggatacattaatcctagcagtgcttatactaattacaatcagaaattcaaggacagagtcacgattaccgcggacaaatccacgagcacagcctacatggagctgagcagcctgagatctgaggacacggccgtgtattactgtgcgagaccccaagtccactatgattacaacgggtttccttactggggccaaggaaccctggtcaccgtctcctcaggtggaggcggttcaggcggaggtggatccggcggtggcggatcgggtggcggcggatctgaaattgtgttgacacagtctccagccaccctgtctttgtctccaggggaaagagccaccctctcctgcagtgccagctcaagtgtaagttacatgaactggtaccaacagaaacctggccaggctcccaggctcctcatctatgactcatccaaactggcttctggcatcccagccaggttcagtggcagtgggtctgggacagacttcactctcaccatcagcagcctagagcctgaagattttgcagtttattactgtcagcagtggagtcgtaacccacccactttcggcggagggaccaaggtggagatcaaacggtcctccagctaa

SEQ ID NO: 24 - protein, 503 aa, Artificial Sequence
  Fc H10L4 (TSC323) CD3-binding domain
EPKSSDKTHTCPPCPAPEAAGAPSVFLFPPKPKDTLMISRTPEVTCVVVDVSHEDPEVKFNWYVDGVEVHNAKTKPREEQYNSTYRVVSVLTVLHQDWLNGKAYACAVSNKALPAPIEKTISKAKGQPREPQVYTLPPSRDELTKNQVSLTCLVKGFYPSDIAVEWESNGQPENNYKTTPPVLDSDGSFFLYSKLTVDKSRWQQGNVFSCSVMHEALHNHYTQKSLSLSPGQRHNNSSLNTGTQMAGHSPNSQVQLVQSGAEVKKPGSSVKVSCKASGGTFSRSTMHWVRQAPGQGLEWMGYINPSSAYTNYNQKFKDRVTITADKSTSTAYMELSSLRSEDTAVYYCARPQVHYDYNGFPYWGQGTLVTVSSGGGGSGGGGSGGGGSGGGGSEIVLTQSPATLSLSPGERATLSCSASSSVSYMNWYQQKPGQAPRLLIYDSSKLASGIPARFSGSGSGTDFTLTISSLEPEDFAVYYCQQWSRNPPTFGGGTKVEIKRSSS

SEQ ID NO: 25 - DNA, 1572 bp, Artificial Sequence
  Fc H10L5 (TSC324) CD3-binding domain
atggaagcaccagcgcagcttctcttcctcctgctactctggctcccagataccaccggtgagcccaaatcttctgacaaaactcacacatgcccaccgtgcccagcacctgaagccgcgggtgcaccgtcagtcttcctcttccccccaaaacccaaggacaccctcatgatctcccggacccctgaggtcacatgcgtggtggtggacgtgagccacgaagaccctgaggtcaagttcaactggtacgtggacggcgtggaggtgcataatgccaagacaaagccgcgggaggagcagtacaacagcacgtaccgtgtggtcagcgtcctcaccgtcctgcaccaggactggctgaatggcaaggcatacgcgtgcgcggtctccaacaaagccctcccagcccccatcgagaaaaccatctccaaagccaaagggcagccccgagaaccacaggtgtacaccctgcccccatcccgggatgagctgaccaagaaccaggtcagcctgacctgcctggtcaaaggcttctatccaagcgacatcgccgtggagtgggagagcaatgggcagccggagaacaactacaagaccacgcctcccgtgctggactccgacggctccttcttcctctacagcaagctcaccgtggacaagagcaggtggcagcaggggaacgtcttctcatgctccgtgatgcatgaggctctgcacaaccactacacgcagaagagcctctccctgtctccgggtcagaggcacaacaattcttccctgaatacaggaactcagatggcaggtcattctccgaattctcaggtccagctggtgcaatctggggctgaggtgaagaagcctgggtcctcggtgaaggtctcctgcaaggcttctggaggcaccttcagcagatctacgatgcactgggtgcgacaggcccctggacaagggcttgagtggatgggatacattaatcctagcagtgcttatactaattacaatcagaaattcaaggacagagtcacgattaccgcggacaaatccacgagcacagcctacatggagctgagcagcctgagatctgaggacacggccgtgtattactgtgcgagaccccaagtccactatgattacaacgggtttccttactggggccaaggaaccctggtcaccgtctcctcaggtggaggcggttcaggcggaggtggatccggcggtggcggatcgggtggcggcggatctgacatccagatgacccagtctccatcctccctgtctgcatctgtaggagacagagtcaccatcacttgcagtgccagctcaagtgtaagttacatgaactggtatcagcagaaaccagggaaagcccctaagctcctgatctatgactcatccaaactggcttctggggtcccatcaaggttcagtggcagtggatctgggacagatttcactctcaccatcagcagtctgcaacctgaagattttgcaacttactactgtcaacagtggagtcgtaacccacccactttcggcggagggaccaaggtggagatcaaacggtcctccagctaa

SEQ ID NO: 26 - protein, 503 aa, Artificial Sequence
  Fc H10L5 (TSC324) CD3-binding domain
EPKSSDKTHTCPPCPAPEAAGAPSVFLFPPKPKDTLMISRTPEVTCVVVDVSHEDPEVKFNWYVDGVEVHNAKTKPREEQYNSTYRVVSVLTVLHQDWLNGKAYACAVSNKALPAPIEKTISKAKGQPREPQVYTLPPSRDELTKNQVSLTCLVKGFYPSDIAVEWESNGQPENNYKTTPPVLDSDGSFFLYSKLTVDKSRWQQGNVFSCSVMHEALHNHYTQKSLSLSPGQRHNNSSLNTGTQMAGHSPNSQVQLVQSGAEVKKPGSSVKVSCKASGGTFSRSTMHWVRQAPGQGLEWMGYINPSSAYTNYNQKFKDRVTITADKSTSTAYMELSSLRSEDTAVYYCARPQVHYDYNGFPYWGQGTLVTVSSGGGGSGGGGSGGGGSGGGGSDIQMTQSPSSLSASVGDRVTITCSASSSVSYMNWYQQKPGKAPKLLIYDSSKLASGVPSRFSGSGSGTDFTLTISSLQPEDFATYYCQQWSRNPPTFGGGTKVEIKRSSS

SEQ ID NO: 27 - DNA, 1572 bp, Artificial Sequence
  Fc H7L6 (TSC334) CD3-binding domain
atggaagcaccagcgcagcttctcttcctcctgctactctggctcccagataccaccggtgagcccaaatcttctgacaaaactcacacatgcccaccgtgcccagcacctgaagccgcgggtgcaccgtcagtcttcctcttccccccaaaacccaaggacaccctcatgatctcccggacccctgaggtcacatgcgtggtggtggacgtgagccacgaagaccctgaggtcaagttcaactggtacgtggacggcgtggaggtgcataatgccaagacaaagccgcgggaggagcagtacaacagcacgtaccgtgtggtcagcgtcctcaccgtcctgcaccaggactggctgaatggcaaggcatacgcatgcgcggtctccaacaaagccctcccagcccccatcgagaaaaccatctccaaagccaaagggcagccccgagaaccacaggtgtacaccctgcccccatcccgggatgagctgaccaagaaccaggtcagcctgacctgcctggtcaaaggcttctatccaagcgacatcgccgtggagtgggagagcaatgggcagccggagaacaactacaagaccacgcctcccgtgctggactccgacggctccttcttcctctacagcaagctcaccgtggacaagagcaggtggcagcaggggaacgtcttctcatgctccgtgatgcatgaggctctgcacaaccactacacgcagaagagcctctccctgtctccgggtcagaggcacaacaattcttccctgaatacaggaactcagatggcaggtcattctccgaattctcaggtgcagctggtgcagtctggggctgaggtgaagaagcctggggcctcagtgaaggtctcctgcaaggcttctggatacaccttcaccagatctacgatgcactgggtgcgacaggcccctggacaagggcttgagtggatgggatacattaatcctagcagtgcttatactaattacaatcagaaattcaaggacagggtcaccatgaccagggacacgtccatcagcacagcctacatggagctgagcaggctgagatctgacgacacggccgtgtattactgtgcgagaccccaagtccactatgattacaacgggtttccttactggggccaaggaaccctggtcaccgtctcctcaggtggaggcggttcaggcggaggtggatccggcggtggcggatcgggtggcggcggatctgacatccagatgacccagtctccatcctccctgtctgcatctgtaggagacagagtcaccatcacttgcagtgccagctcaagtgtaagttacatgaactggtatcagcagaaaccagggaaagcccctaagagatggatttatgactcatccaaactggcttctggggtcccatcaaggttcagtggcagtggatctgggacagatttcactctcaccatcagcagtctgcaacctgaagattttgcaacttactactgtcaacagtggagtcgtaacccacccactttcggcggagggaccaaggtggagatcaaacggtcctccagctaa

SEQ ID NO: 28 - protein, 503 aa, Artificial Sequence
  Fc H7L6 (TSC334) CD3-binding domain
EPKSSDKTHTCPPCPAPEAAGAPSVFLFPPKPKDTLMISRTPEVTCVVVDVSHEDPEVKFNWYVDGVEVHNAKTKPREEQYNSTYRVVSVLTVLHQDWLNGKAYACAVSNKALPAPIEKTISKAKGQPREPQVYTLPPSRDELTKNQVSLTCLVKGFYPSDIAVEWESNGQPENNYKTTPPVLDSDGSFFLYSKLTVDKSRWQQGNVFSCSVMHEALHNHYTQKSLSLSPGQRHNNSSLNTGTQMAGHSPNSQVQLVQSGAEVKKPGASVKVSCKASGYTFTRSTMHWVRQAPGQGLEWMGYINPSSAYTNYNQKFKDRVTMTRDTSISTAYMELSRLRSDDTAVYYCARPQVHYDYNGFPYWGQGTLVTVSSGGGGSGGGGSGGGGSGGGGSDIQMTQSPSSLSASVGDRVTITCSASSSVSYMNWYQQKPGKAPKRWIYDSSKLASGVPSRFSGSGSGTDFTLTISSLQPEDFATYYCQQWSRNPPTFGGGTKVEIKRSSS

SEQ ID NO: 29 - DNA, 1572 bp, Artificial Sequence
  Fc H7L7 (TSC335) CD3-binding domain
atggaagcaccagcgcagcttctcttcctcctgctactctggctcccagataccaccggtgagcccaaatcttctgacaaaactcacacatgcccaccgtgcccagcacctgaagccgcgggtgcaccgtcagtcttcctcttccccccaaaacccaaggacaccctcatgatctcccggacccctgaggtcacatgcgtggtggtggacgtgagccacgaagaccctgaggtcaagttcaactggtacgtggacggcgtggaggtgcataatgccaagacaaagccgcgggaggagcagtacaacagcacgtaccgtgtggtcagcgtcctcaccgtcctgcaccaggactggctgaatggcaaggcatacgcatgcgcggtctccaacaaagccctcccagcccccatcgagaaaaccatctccaaagccaaagggcagccccgagaaccacaggtgtacaccctgcccccatcccgggatgagctgaccaagaaccaggtcagcctgacctgcctggtcaaaggcttctatccaagcgacatcgccgtggagtgggagagcaatgggcagccggagaacaactacaagaccacgcctcccgtgctggactccgacggctccttcttcctctacagcaagctcaccgtggacaagagcaggtggcagcaggggaacgtcttctcatgctccgtgatgcatgaggctctgcacaaccactacacgcagaagagcctctccctgtctccgggtcagaggcacaacaattcttccctgaatacaggaactcagatggcaggtcattctccgaattctcaggtgcagctggtgcagtctggggctgaggtgaagaagcctggggcctcagtgaaggtctcctgcaaggcttctggatacaccttcaccagatctacgatgcactgggtgcgacaggcccctggacaagggcttgagtggatgggatacattaatcctagcagtgcttatactaattacaatcagaaattcaaggacagggtcaccatgaccagggacacgtccatcagcacagcctacatggagctgagcaggctgagatctgacgacacggccgtgtattactgtgcgagaccccaagtccactatgattacaacgggtttccttactggggccaaggaaccctggtcaccgtctcctcaggtggaggcggttcaggcggaggtggatccggcggtggcggatcgggtggcggcggatctgaaattgtgttgacgcagtctccagccaccctgtctttgtctccaggggaaagagccaccctctcctgcagtgccagctcaagtgtaagttacatgaactggtaccagcagaaacctggcctggcgcccaggagatggatttatgactcatccaaactggcttctggcatcccagacaggttcagtggcagtgggtctgggacagacttcactctcaccatcagcagactggagcctgaagattttgcagtgtattactgtcagcagtggagtcgtaacccacccactttcggcggagggaccaaggtggagatcaaacggtcctccagctaa

SEQ ID NO: 30 - protein, 503 aa, Artificial Sequence
  Fc H7L7 (TSC335) CD3-binding domain
EPKSSDKTHTCPPCPAPEAAGAPSVFLFPPKPKDTLMISRTPEVTCVVVDVSHEDPEVKFNWYVDGVEVHNAKTKPREEQYNSTYRVVSVLTVLHQDWLNGKAYACAVSNKALPAPIEKTISKAKGQPREPQVYTLPPSRDELTKNQVSLTCLVKGFYPSDIAVEWESNGQPENNYKTTPPVLDSDGSFFLYSKLTVDKSRWQQGNVFSCSVMHEALHNHYTQKSLSLSPGQRHNNSSLNTGTQMAGHSPNSQVQLVQSGAEVKKPGASVKVSCKASGYTFTRSTMHWVRQAPGQGLEWMGYINPSSAYTNYNQKFKDRVTMTRDTSISTAYMELSRLRSDDTAVYYCARPQVHYDYNGFPYWGQGTLVTVSSGGGGSGGGGSGGGGSGGGGSEIVLTQSPATLSLSPGERATLSCSASSSVSYMNWYQQKPGLAPRRWIYDSSKLASGIPDRFSGSGSGTDFTLTISRLEPEDFAVYYCQQWSRNPPTFGGGTKVEIKRSSS

SEQ ID NO: 31 - DNA, 1572 bp, Artificial Sequence
  Fc H7L8 (TSC336) CD3-binding domain
atggaagcaccagcgcagcttctcttcctcctgctactctggctcccagataccaccggtgagcccaaatcttctgacaaaactcacacatgcccaccgtgcccagcacctgaagccgcgggtgcaccgtcagtcttcctcttccccccaaaacccaaggacaccctcatgatctcccggacccctgaggtcacatgcgtggtggtggacgtgagccacgaagaccctgaggtcaagttcaactggtacgtggacggcgtggaggtgcataatgccaagacaaagccgcgggaggagcagtacaacagcacgtaccgtgtggtcagcgtcctcaccgtcctgcaccaggactggctgaatggcaaggcatacgcatgcgcggtctccaacaaagccctcccagcccccatcgagaaaaccatctccaaagccaaagggcagccccgagaaccacaggtgtacaccctgcccccatcccgggatgagctgaccaagaaccaggtcagcctgacctgcctggtcaaaggcttctatccaagcgacatcgccgtggagtgggagagcaatgggcagccggagaacaactacaagaccacgcctcccgtgctggactccgacggctccttcttcctctacagcaagctcaccgtggacaagagcaggtggcagcaggggaacgtcttctcatgctccgtgatgcatgaggctctgcacaaccactacacgcagaagagcctctccctgtctccgggtcagaggcacaacaattcttccctgaatacaggaactcagatggcaggtcattctccgaattctcaggtgcagctggtgcagtctggggctgaggtgaagaagcctggggcctcagtgaaggtctcctgcaaggcttctggatacaccttcaccagatctacgatgcactgggtgcgacaggcccctggacaagggcttgagtggatgggatacattaatcctagcagtgcttatactaattacaatcagaaattcaaggacagggtcaccatgaccagggacacgtccatcagcacagcctacatggagctgagcaggctgagatctgacgacacggccgtgtattactgtgcgagaccccaagtccactatgattacaacgggtttccttactggggccaaggaaccctggtcaccgtctcctcaggtggaggcggttcaggcggaggtggatccggcggtggcggatcgggtggcggcggatctgacatccagatgacccagtctccttccaccctgtctgcatctgtaggagacagagtcaccatcacttgcagtgccagctcaagtgtaagttacatgaactggtatcagcagaaaccagggaaagcccctaagagatggatttatgactcatccaaactggcttctggggtcccatcaaggttcagcggcagtggatctgggacagaattcactctcaccatcagcagcctgcagcctgatgattttgcaacttattactgccaacagtggagtcgtaacccacccactttcggcggagggaccaaggtggagatcaaacggtcctccagctaa

SEQ ID NO: 32 - protein, 503 aa, Artificial Sequence
  Fc H7L8 (TSC336) CD3-binding domain
EPKSSDKTHTCPPCPAPEAAGAPSVFLFPPKPKDTLMISRTPEVTCVVVDVSHEDPEVKFNWYVDGVEVHNAKTKPREEQYNSTYRVVSVLTVLHQDWLNGKAYACAVSNKALPAPIEKTISKAKGQPREPQVYTLPPSRDELTKNQVSLTCLVKGFYPSDIAVEWESNGQPENNYKTTPPVLDSDGSFFLYSKLTVDKSRWQQGNVFSCSVMHEALHNHYTQKSLSLSPGQRHNNSSLNTGTQMAGHSPNSQVQLVQSGAEVKKPGASVKVSCKASGYTFTRSTMHWVRQAPGQGLEWMGYINPSSAYTNYNQKFKDRVTMTRDTSISTAYMELSRLRSDDTAVYYCARPQVHYDYNGFPYWGQGTLVTVSSGGGGSGGGGSGGGGSGGGGSDIQMTQSPSTLSASVGDRVTITCSASSSVSYMNWYQQKPGKAPKRWIYDSSKLASGVPSRFSGSGSGTEFTLTISSLQPDDFATYYCQQWSRNPPTFGGGTKVEIKRSSS

SEQ ID NO: 33 - DNA, 1572 bp, Artificial Sequence
  Fc H8L6 (TSC337) CD3-binding domain
atggaagcaccagcgcagcttctcttcctcctgctactctggctcccagataccaccggtgagcccaaatcttctgacaaaactcacacatgcccaccgtgcccagcacctgaagccgcgggtgcaccgtcagtcttcctcttccccccaaaacccaaggacaccctcatgatctcccggacccctgaggtcacatgcgtggtggtggacgtgagccacgaagaccctgaggtcaagttcaactggtacgtggacggcgtggaggtgcataatgccaagacaaagccgcgggaggagcagtacaacagcacgtaccgtgtggtcagcgtcctcaccgtcctgcaccaggactggctgaatggcaaggcatacgcatgcgcggtctccaacaaagccctcccagcccccatcgagaaaaccatctccaaagccaaagggcagccccgagaaccacaggtgtacaccctgcccccatcccgggatgagctgaccaagaaccaggtcagcctgacctgcctggtcaaaggcttctatccaagcgacatcgccgtggagtgggagagcaatgggcagccggagaacaactacaagaccacgcctcccgtgctggactccgacggctccttcttcctctacagcaagctcaccgtggacaagagcaggtggcagcaggggaacgtcttctcatgctccgtgatgcatgaggctctgcacaaccactacacgcagaagagcctctccctgtctccgggtcagaggcacaacaattcttccctgaatacaggaactcagatggcaggtcattctccgaattctcaggtgcagctggtgcagtctggggctgaggtgaagaagcctggggcctcagtgaaggtttcctgcaaggcatctggatacaccttcaccagatctacgatgcactgggtgcgacaggcccctggacaagggcttgagtggatgggatacattaatcctagcagtgcttatactaattacaatcagaaattcaaggacagagtcaccatgaccagggacacgtccacgagcacagtctacatggagctgagcagcctgagatctgaggacacggccgtgtattactgtgctagaccccaagtccactatgattacaacgggtttccttactggggccaaggaaccctggtcaccgtctcctcaggtggaggcggttcaggcggaggtggatccggcggtggcggatcgggtggcggcggatctgacatccagatgacccagtctccatcctccctgtctgcatctgtaggagacagagtcaccatcacttgcagtgccagctcaagtgtaagttacatgaactggtatcagcagaaaccagggaaagcccctaagagatggatttatgactcatccaaactggcttctggggtcccatcaaggttcagtggcagtggatctgggacagatttcactctcaccatcagcagtctgcaacctgaagattttgcaacttactactgtcaacagtggagtcgtaacccacccactttcggcggagggaccaaggtggagatcaaacggtcctccagctaa

SEQ ID NO: 34 - protein, 503 aa, Artificial Sequence
  Fc H8L6 (TSC337) CD3-binding domain
EPKSSDKTHTCPPCPAPEAAGAPSVFLFPPKPKDTLMISRTPEVTCVVVDVSHEDPEVKFNWYVDGVEVHNAKTKPREEQYNSTYRVVSVLTVLHQDWLNGKAYACAVSNKALPAPIEKTISKAKGQPREPQVYTLPPSRDELTKNQVSLTCLVKGFYPSDIAVEWESNGQPENNYKTTPPVLDSDGSFFLYSKLTVDKSRWQQGNVFSCSVMHEALHNHYTQKSLSLSPGQRHNNSSLNTGTQMAGHSPNSQVQLVQSGAEVKKPGASVKVSCKASGYTFTRSTMHWVRQAPGQGLEWMGYINPSSAYTNYNQKFKDRVTMTRDTSTSTVYMELSSLRSEDTAVYYCARPQVHYDYNGFPYWGQGTLVTVSSGGGGSGGGGSGGGGSGGGGSDIQMTQSPSSLSASVGDRVTITCSASSSVSYMNWYQQKPGKAPKRWIYDSSKLASGVPSRFSGSGSGTDFTLTISSLQPEDFATYYCQQWSRNPPTFGGGTKVEIKRSSS

SEQ ID NO: 35 - DNA, 1572 bp, Artificial Sequence
  Fc H8L7 (TSC338) CD3-binding domain
atggaagcaccagcgcagcttctcttcctcctgctactctggctcccagataccaccggtgagcccaaatcttctgacaaaactcacacatgcccaccgtgcccagcacctgaagccgcgggtgcaccgtcagtcttcctcttccccccaaaacccaaggacaccctcatgatctcccggacccctgaggtcacatgcgtggtggtggacgtgagccacgaagaccctgaggtcaagttcaactggtacgtggacggcgtggaggtgcataatgccaagacaaagccgcgggaggagcagtacaacagcacgtaccgtgtggtcagcgtcctcaccgtcctgcaccaggactggctgaatggcaaggcatacgcatgcgcggtctccaacaaagccctcccagcccccatcgagaaaaccatctccaaagccaaagggcagccccgagaaccacaggtgtacaccctgcccccatcccgggatgagctgaccaagaaccaggtcagcctgacctgcctggtcaaaggcttctatccaagcgacatcgccgtggagtgggagagcaatgggcagccggagaacaactacaagaccacgcctcccgtgctggactccgacggctccttcttcctctacagcaagctcaccgtggacaagagcaggtggcagcaggggaacgtcttctcatgctccgtgatgcatgaggctctgcacaaccactacacgcagaagagcctctccctgtctccgggtcagaggcacaacaattcttccctgaatacaggaactcagatggcaggtcattctccgaattctcaggtgcagctggtgcagtctggggctgaggtgaagaagcctggggcctcagtgaaggtttcctgcaaggcatctggatacaccttcaccagatctacgatgcactgggtgcgacaggcccctggacaagggcttgagtggatgggatacattaatcctagcagtgcttatactaattacaatcagaaattcaaggacagagtcaccatgaccagggacacgtccacgagcacagtctacatggagctgagcagcctgagatctgaggacacggccgtgtattactgtgctagaccccaagtccactatgattacaacgggtttccttactggggccaaggaaccctggtcaccgtctcctcaggtggaggcggttcaggcggaggtggatccggcggtggcggatcgggtggcggcggatctgaaattgtgttgacgcagtctccagccaccctgtctttgtctccaggggaaagagccaccctctcctgcagtgccagctcaagtgtaagttacatgaactggtaccagcagaaacctggcctggcgcccaggagatggatttatgactcatccaaactggcttctggcatcccagacaggttcagtggcagtgggtctgggacagacttcactctcaccatcagcagactggagcctgaagattttgcagtgtattactgtcagcagtggagtcgtaacccacccactttcggcggagggaccaaggtggagatcaaacggtcctccagctaa

SEQ ID NO: 36 - protein, 503 aa, Artificial Sequence
  Fc H8L7 (TSC338) CD3-binding domain
EPKSSDKTHTCPPCPAPEAAGAPSVFLFPPKPKDTLMISRTPEVTCVVVDVSHEDPEVKFNWYVDGVEVHNAKTKPREEQYNSTYRVVSVLTVLHQDWLNGKAYACAVSNKALPAPIEKTISKAKGQPREPQVYTLPPSRDELTKNQVSLTCLVKGFYPSDIAVEWESNGQPENNYKTTPPVLDSDGSFFLYSKLTVDKSRWQQGNVFSCSVMHEALHNHYTQKSLSLSPGQRHNNSSLNTGTQMAGHSPNSQVQLVQSGAEVKKPGASVKVSCKASGYTFTRSTMHWVRQAPGQGLEWMGYINPSSAYTNYNQKFKDRVTMTRDTSTSTVYMELSSLRSEDTAVYYCARPQVHYDYNGFPYWGQGTLVTVSSGGGGSGGGGSGGGGSGGGGSEIVLTQSPATLSLSPGERATLSCSASSSVSYMNWYQQKPGLAPRRWIYDSSKLASGIPDRFSGSGSGTDFTLTISRLEPEDFAVYYCQQWSRNPPTFGGGTKVEIKRSSS

SEQ ID NO: 37 - DNA, 1572 bp, Artificial Sequence
  Fc H8L8 (TSC339) CD3-binding domain
atggaagcaccagcgcagcttctcttcctcctgctactctggctcccagataccaccggtgagcccaaatcttctgacaaaactcacacatgcccaccgtgcccagcacctgaagccgcgggtgcaccgtcagtcttcctcttccccccaaaacccaaggacaccctcatgatctcccggacccctgaggtcacatgcgtggtggtggacgtgagccacgaagaccctgaggtcaagttcaactggtacgtggacggcgtggaggtgcataatgccaagacaaagccgcgggaggagcagtacaacagcacgtaccgtgtggtcagcgtcctcaccgtcctgcaccaggactggctgaatggcaaggcatacgcatgcgcggtctccaacaaagccctcccagcccccatcgagaaaaccatctccaaagccaaagggcagccccgagaaccacaggtgtacaccctgcccccatcccgggatgagctgaccaagaaccaggtcagcctgacctgcctggtcaaaggcttctatccaagcgacatcgccgtggagtgggagagcaatgggcagccggagaacaactacaagaccacgcctcccgtgctggactccgacggctccttcttcctctacagcaagctcaccgtggacaagagcaggtggcagcaggggaacgtcttctcatgctccgtgatgcatgaggctctgcacaaccactacacgcagaagagcctctccctgtctccgggtcagaggcacaacaattcttccctgaatacaggaactcagatggcaggtcattctccgaattctcaggtgcagctggtgcagtctggggctgaggtgaagaagcctggggcctcagtgaaggtttcctgcaaggcatctggatacaccttcaccagatctacgatgcactgggtgcgacaggcccctggacaagggcttgagtggatgggatacattaatcctagcagtgcttatactaattacaatcagaaattcaaggacagagtcaccatgaccagggacacgtccacgagcacagtctacatggagctgagcagcctgagatctgaggacacggccgtgtattactgtgctagaccccaagtccactatgattacaacgggtttccttactggggccaaggaaccctggtcaccgtctcctcaggtggaggcggttcaggcggaggtggatccggcggtggcggatcgggtggcggcggatctgacatccagatgacccagtctccttccaccctgtctgcatctgtaggagacagagtcaccatcacttgcagtgccagctcaagtgtaagttacatgaactggtatcagcagaaaccagggaaagcccctaagagatggatttatgactcatccaaactggcttctggggtcccatcaaggttcagcggcagtggatctgggacagaattcactctcaccatcagcagcctgcagcctgatgattttgcaacttattactgccaacagtggagtcgtaacccacccactttcggcggagggaccaaggtggagatcaaacggtcctccagctaa

SEQ ID NO: 38 - protein, 503 aa, Artificial Sequence
  Fc H8L8 (TSC339) CD3-binding domain
EPKSSDKTHTCPPCPAPEAAGAPSVFLFPPKPKDTLMISRTPEVTCVVVDVSHEDPEVKFNWYVDGVEVHNAKTKPREEQYNSTYRVVSVLTVLHQDWLNGKAYACAVSNKALPAPIEKTISKAKGQPREPQVYTLPPSRDELTKNQVSLTCLVKGFYPSDIAVEWESNGQPENNYKTTPPVLDSDGSFFLYSKLTVDKSRWQQGNVFSCSVMHEALHNHYTQKSLSLSPGQRHNNSSLNTGTQMAGHSPNSQVQLVQSGAEVKKPGASVKVSCKASGYTFTRSTMHWVRQAPGQGLEWMGYINPSSAYTNYNQKFKDRVTMTRDTSTSTVYMELSSLRSEDTAVYYCARPQVHYDYNGFPYWGQGTLVTVSSGGGGSGGGGSGGGGSGGGGSDIQMTQSPSTLSASVGDRVTITCSASSSVSYMNWYQQKPGKAPKRWIYDSSKLASGVPSRFSGSGSGTEFTLTISSLQPDDFATYYCQQWSRNPPTFGGGTKVEIKRSSS

SEQ ID NO: 39 - DNA, 1572 bp, Artificial Sequence
  Fc H10L6 (TSC340) CD3-binding domain
atggaagcaccagcgcagcttctcttcctcctgctactctggctcccagataccaccggtgagcccaaatcttctgacaaaactcacacatgcccaccgtgcccagcacctgaagccgcgggtgcaccgtcagtcttcctcttccccccaaaacccaaggacaccctcatgatctcccggacccctgaggtcacatgcgtggtggtggacgtgagccacgaagaccctgaggtcaagttcaactggtacgtggacggcgtggaggtgcataatgccaagacaaagccgcgggaggagcagtacaacagcacgtaccgtgtggtcagcgtcctcaccgtcctgcaccaggactggctgaatggcaaggcatacgcatgcgcggtctccaacaaagccctcccagcccccatcgagaaaaccatctccaaagccaaagggcagccccgagaaccacaggtgtacaccctgcccccatcccgggatgagctgaccaagaaccaggtcagcctgacctgcctggtcaaaggcttctatccaagcgacatcgccgtggagtgggagagcaatgggcagccggagaacaactacaagaccacgcctcccgtgctggactccgacggctccttcttcctctacagcaagctcaccgtggacaagagcaggtggcagcaggggaacgtcttctcatgctccgtgatgcatgaggctctgcacaaccactacacgcagaagagcctctccctgtctccgggtcagaggcacaacaattcttccctgaatacaggaactcagatggcaggtcattctccgaattctcaggtccagctggtgcaatctggggctgaggtgaagaagcctgggtcctcggtgaaggtctcctgcaaggcttctggaggcaccttcagcagatctacgatgcactgggtgcgacaggcccctggacaagggcttgagtggatgggatacattaatcctagcagtgcttatactaattacaatcagaaattcaaggacagagtcacgattaccgcggacaaatccacgagcacagcctacatggagctgagcagcctgagatctgaggacacggccgtgtattactgtgcgagaccccaagtccactatgattacaacgggtttccttactggggccaaggaaccctggtcaccgtctcctcaggtggaggcggttcaggcggaggtggatccggcggtggcggatcgggtggcggcggatctgacatccagatgacccagtctccatcctccctgtctgcatctgtaggagacagagtcaccatcacttgcagtgccagctcaagtgtaagttacatgaactggtatcagcagaaaccagggaaagcccctaagagatggatttatgactcatccaaactggcttctggggtcccatcaaggttcagtggcagtggatctgggacagatttcactctcaccatcagcagtctgcaacctgaagattttgcaacttactactgtcaacagtggagtcgtaacccacccactttcggcggagggaccaaggtggagatcaaacggtcctccagctaa

SEQ ID NO: 40 - protein, 503 aa, Artificial Sequence
  Fc H10L6 (TSC340) CD3-binding domain
EPKSSDKTHTCPPCPAPEAAGAPSVFLFPPKPKDTLMISRTPEVTCVVVDVSHEDPEVKFNWYVDGVEVHNAKTKPREEQYNSTYRVVSVLTVLHQDWLNGKAYACAVSNKALPAPIEKTISKAKGQPREPQVYTLPPSRDELTKNQVSLTCLVKGFYPSDIAVEWESNGQPENNYKTTPPVLDSDGSFFLYSKLTVDKSRWQQGNVFSCSVMHEALHNHYTQKSLSLSPGQRHNNSSLNTGTQMAGHSPNSQVQLVQSGAEVKKPGSSVKVSCKASGGTFSRSTMHWVRQAPGQGLEWMGYINPSSAYTNYNQKFKDRVTITADKSTSTAYMELSSLRSEDTAVYYCARPQVHYDYNGFPYWGQGTLVTVSSGGGGSGGGGSGGGGSGGGGSDIQMTQSPSSLSASVGDRVTITCSASSSVSYMNWYQQKPGKAPKRWIYDSSKLASGVPSRFSGSGSGTDFTLTISSLQPEDFATYYCQQWSRNPPTFGGGTKVEIKRSSS

SEQ ID NO: 41 - DNA, 1572 bp, Artificial Sequence
  Fc H10L7 (TSC341) CD3-binding domain
atggaagcaccagcgcagcttctcttcctcctgctactctggctcccagataccaccggtgagcccaaatcttctgacaaaactcacacatgcccaccgtgcccagcacctgaagccgcgggtgcaccgtcagtcttcctcttccccccaaaacccaaggacaccctcatgatctcccggacccctgaggtcacatgcgtggtggtggacgtgagccacgaagaccctgaggtcaagttcaactggtacgtggacggcgtggaggtgcataatgccaagacaaagccgcgggaggagcagtacaacagcacgtaccgtgtggtcagcgtcctcaccgtcctgcaccaggactggctgaatggcaaggcatacgcatgcgcggtctccaacaaagccctcccagcccccatcgagaaaaccatctccaaagccaaagggcagccccgagaaccacaggtgtacaccctgcccccatcccgggatgagctgaccaagaaccaggtcagcctgacctgcctggtcaaaggcttctatccaagcgacatcgccgtggagtgggagagcaatgggcagccggagaacaactacaagaccacgcctcccgtgctggactccgacggctccttcttcctctacagcaagctcaccgtggacaagagcaggtggcagcaggggaacgtcttctcatgctccgtgatgcatgaggctctgcacaaccactacacgcagaagagcctctccctgtctccgggtcagaggcacaacaattcttccctgaatacaggaactcagatggcaggtcattctccgaattctcaggtccagctggtgcaatctggggctgaggtgaagaagcctgggtcctcggtgaaggtctcctgcaaggcttctggaggcaccttcagcagatctacgatgcactgggtgcgacaggcccctggacaagggcttgagtggatgggatacattaatcctagcagtgcttatactaattacaatcagaaattcaaggacagagtcacgattaccgcggacaaatccacgagcacagcctacatggagctgagcagcctgagatctgaggacacggccgtgtattactgtgcgagaccccaagtccactatgattacaacgggtttccttactggggccaaggaaccctggtcaccgtctcctcaggtggaggcggttcaggcggaggtggatccggcggtggcggatcgggtggcggcggatctgaaattgtgttgacgcagtctccagccaccctgtctttgtctccaggggaaagagccaccctctcctgcagtgccagctcaagtgtaagttacatgaactggtaccagcagaaacctggcctggcgcccaggagatggatttatgactcatccaaactggcttctggcatcccagacaggttcagtggcagtgggtctgggacagacttcactctcaccatcagcagactggagcctgaagattttgcagtgtattactgtcagcagtggagtcgtaacccacccactttcggcggagggaccaaggtggagatcaaacggtcctccagctaa

SEQ ID NO: 42 - protein, 503 aa, Artificial Sequence
  Fc H10L7 (TSC341) CD3-binding domain
EPKSSDKTHTCPPCPAPEAAGAPSVFLFPPKPKDTLMISRTPEVTCVVVDVSHEDPEVKFNWYVDGVEVHNAKTKPREEQYNSTYRVVSVLTVLHQDWLNGKAYACAVSNKALPAPIEKTISKAKGQPREPQVYTLPPSRDELTKNQVSLTCLVKGFYPSDIAVEWESNGQPENNYKTTPPVLDSDGSFFLYSKLTVDKSRWQQGNVFSCSVMHEALHNHYTQKSLSLSPGQRHNNSSLNTGTQMAGHSPNSQVQLVQSGAEVKKPGSSVKVSCKASGGTFSRSTMHWVRQAPGQGLEWMGYINPSSAYTNYNQKFKDRVTITADKSTSTAYMELSSLRSEDTAVYYCARPQVHYDYNGFPYWGQGTLVTVSSGGGGSGGGGSGGGGSGGGGSEIVLTQSPATLSLSPGERATLSCSASSSVSYMNWYQQKPGLAPRRWIYDSSKLASGIPDRFSGSGSGTDFTLTISRLEPEDFAVYYCQQWSRNPPTFGGGTKVEIKRSSS

SEQ ID NO: 43 - DNA, 1572 bp, Artificial Sequence
  Fc H10L8 (TSC342) CD3-binding domain
atggaagcaccagcgcagcttctcttcctcctgctactctggctcccagataccaccggtgagcccaaatcttctgacaaaactcacacatgcccaccgtgcccagcacctgaagccgcgggtgcaccgtcagtcttcctcttccccccaaaacccaaggacaccctcatgatctcccggacccctgaggtcacatgcgtggtggtggacgtgagccacgaagaccctgaggtcaagttcaactggtacgtggacggcgtggaggtgcataatgccaagacaaagccgcgggaggagcagtacaacagcacgtaccgtgtggtcagcgtcctcaccgtcctgcaccaggactggctgaatggcaaggcatacgcatgcgcggtctccaacaaagccctcccagcccccatcgagaaaaccatctccaaagccaaagggcagccccgagaaccacaggtgtacaccctgcccccatcccgggatgagctgaccaagaaccaggtcagcctgacctgcctggtcaaaggcttctatccaagcgacatcgccgtggagtgggagagcaatgggcagccggagaacaactacaagaccacgcctcccgtgctggactccgacggctccttcttcctctacagcaagctcaccgtggacaagagcaggtggcagcaggggaacgtcttctcatgctccgtgatgcatgaggctctgcacaaccactacacgcagaagagcctctccctgtctccgggtcagaggcacaacaattcttccctgaatacaggaactcagatggcaggtcattctccgaattctcaggtccagctggtgcaatctggggctgaggtgaagaagcctgggtcctcggtgaaggtctcctgcaaggcttctggaggcaccttcagcagatctacgatgcactgggtgcgacaggcccctggacaagggcttgagtggatgggatacattaatcctagcagtgcttatactaattacaatcagaaattcaaggacagagtcacgattaccgcggacaaatccacgagcacagcctacatggagctgagcagcctgagatctgaggacacggccgtgtattactgtgcgagaccccaagtccactatgattacaacgggtttccttactggggccaaggaaccctggtcaccgtctcctcaggtggaggcggttcaggcggaggtggatccggcggtggcggatcgggtggcggcggatctgacatccagatgacccagtctccttccaccctgtctgcatctgtaggagacagagtcaccatcacttgcagtgccagctcaagtgtaagttacatgaactggtatcagcagaaaccagggaaagcccctaagagatggatttatgactcatccaaactggcttctggggtcccatcaaggttcagcggcagtggatctgggacagaattcactctcaccatcagcagcctgcagcctgatgattttgcaacttattactgccaacagtggagtcgtaacccacccactttcggcggagggaccaaggtggagatcaaacggtcctccagctaa

SEQ ID NO: 44 - protein, 503 aa, Artificial Sequence
  Fc H10L8 (TSC342) CD3-binding domain
EPKSSDKTHTCPPCPAPEAAGAPSVFLFPPKPKDTLMISRTPEVTCVVVDVSHEDPEVKFNWYVDGVEVHNAKTKPREEQYNSTYRVVSVLTVLHQDWLNGKAYACAVSNKALPAPIEKTISKAKGQPREPQVYTLPPSRDELTKNQVSLTCLVKGFYPSDIAVEWESNGQPENNYKTTPPVLDSDGSFFLYSKLTVDKSRWQQGNVFSCSVMHEALHNHYTQKSLSLSPGQRHNNSSLNTGTQMAGHSPNSQVQLVQSGAEVKKPGSSVKVSCKASGGTFSRSTMHWVRQAPGQGLEWMGYINPSSAYTNYNQKFKDRVTITADKSTSTAYMELSSLRSEDTAVYYCARPQVHYDYNGFPYWGQGTLVTVSSGGGGSGGGGSGGGGSGGGGSDIQMTQSPSTLSASVGDRVTITCSASSSVSYMNWYQQKPGKAPKRWIYDSSKLASGVPSRFSGSGSGTEFTLTISSLQPDDFATYYCQQWSRNPPTFGGGTKVEIKRSSS

SEQ ID NO: 45 - DNA, 1572 bp, Artificial Sequence
  TSC370 CD3-binding domain
atggaagcaccagcgcagcttctcttcctcctgctactctggctcccagataccaccggtgagcccaaatcttctgacaaaactcacacatgcccaccgtgcccagcacctgaagccgcgggtgcaccgtcagtcttcctcttccccccaaaacccaaggacaccctcatgatctcccggacccctgaggtcacatgcgtggtggtggacgtgagccacgaagaccctgaggtcaagttcaactggtacgtggacggcgtggaggtgcataatgccaagacaaagccgcgggaggagcagtacaacagcacgtaccgtgtggtcagcgtcctcaccgtcctgcaccaggactggctgaatggcaaggcatacgcatgcgcggtctccaacaaagccctcccagcccccatcgagaaaaccatctccaaagccaaagggcagccccgagaaccacaggtgtacaccctgcccccatcccgggatgagctgaccaagaaccaggtcagcctgacctgcctggtcaaaggcttctatccaagcgacatcgccgtggagtgggagagcaatgggcagccggagaacaactacaagaccacgcctcccgtgctggactccgacggctccttcttcctctacagcaagctcaccgtggacaagagcaggtggcagcaggggaacgtcttctcatgctccgtgatgcatgaggctctgcacaaccactacacgcagaagagcctctccctgtctccgggtcagaggcacaacaattcttccctgaatacaggaactcagatggcaggtcattctccgaattctcaggtccagctggtgcaatctggggctgaggtgaagaagcctgggtcctcggtgaaggtctcctgcaaggcttctggatataccttcagcagatctacgatgcactgggtgcgacaggcccctggacaagggcttgagtggatgggatacattaatcctagcagtgcttatactaattacaatcagaaattcaaggacagagtcacgattaccgcggacaaatccacgagcacagcctacatggagctgagcagcctgagatctgaggacacggccgtgtattactgtgcgagaccccaagtccactatgattacaacgggtttccttactggggccaaggaaccctggtcaccgtctcctcaggtggaggcggttcaggcggaggtggatccggcggtggcggatcgggtggcggcggatctgacatccagatgacccagtctccttccaccctgtctgcatctgtaggagacagagtcaccatcacttgcagtgccagctcaagtgtaagttacatgaactggtatcagcagaaaccagggaaagcccctaagagatggatttatgactcatccaaactggcttctggggtcccatcaaggttcagcggcagtggatctgggacagaattcactctcaccatcagcagcctgcagcctgatgattttgcaacttattactgccaacagtggagtcgtaacccacccactttcggcggagggaccaaggtggagatcaaacggtcctccagctaa

SEQ ID NO: 46 - protein, 503 aa, Artificial Sequence
  TSC370 CD3-binding domain
EPKSSDKTHTCPPCPAPEAAGAPSVFLFPPKPKDTLMISRTPEVTCVVVDVSHEDPEVKFNWYVDGVEVHNAKTKPREEQYNSTYRVVSVLTVLHQDWLNGKAYACAVSNKALPAPIEKTISKAKGQPREPQVYTLPPSRDELTKNQVSLTCLVKGFYPSDIAVEWESNGQPENNYKTTPPVLDSDGSFFLYSKLTVDKSRWQQGNVFSCSVMHEALHNHYTQKSLSLSPGQRHNNSSLNTGTQMAGHSPNSQVQLVQSGAEVKKPGSSVKVSCKASGYTFSRSTMHWVRQAPGQGLEWMGYINPSSAYTNYNQKFKDRVTITADKSTSTAYMELSSLRSEDTAVYYCARPQVHYDYNGFPYWGQGTLVTVSSGGGGSGGGGSGGGGSGGGGSDIQMTQSPSTLSASVGDRVTITCSASSSVSYMNWYQQKPGKAPKRWIYDSSKLASGVPSRFSGSGSGTEFTLTISSLQPDDFATYYCQQWSRNPPTFGGGTKVEIKRSSS

SEQ ID NO: 47 - DNA, 1572 bp, Artificial Sequence
  TSC371 CD3-binding domain
atggaagcaccagcgcagcttctcttcctcctgctactctggctcccagataccaccggtgagcccaaatcttctgacaaaactcacacatgcccaccgtgcccagcacctgaagccgcgggtgcaccgtcagtcttcctcttccccccaaaacccaaggacaccctcatgatctcccggacccctgaggtcacatgcgtggtggtggacgtgagccacgaagaccctgaggtcaagttcaactggtacgtggacggcgtggaggtgcataatgccaagacaaagccgcgggaggagcagtacaacagcacgtaccgtgtggtcagcgtcctcaccgtcctgcaccaggactggctgaatggcaaggcatacgcatgcgcggtctccaacaaagccctcccagcccccatcgagaaaaccatctccaaagccaaagggcagccccgagaaccacaggtgtacaccctgcccccatcccgggatgagctgaccaagaaccaggtcagcctgacctgcctggtcaaaggcttctatccaagcgacatcgccgtggagtgggagagcaatgggcagccggagaacaactacaagaccacgcctcccgtgctggactccgacggctccttcttcctctacagcaagctcaccgtggacaagagcaggtggcagcaggggaacgtcttctcatgctccgtgatgcatgaggctctgcacaaccactacacgcagaagagcctctccctgtctccgggtcagaggcacaacaattcttccctgaatacaggaactcagatggcaggtcattctccgaattctcaggtccagctggtgcaatctggggctgaggtgaagaagcctgggtcctcggtgaaggtctcctgcaaggcttctggaggcaccttcagcagatctacgatgcactgggtgcgacaggcccctggacaagggcttgagtggataggatacattaatcctagcagtgcttatactaattacaatcagaaattcaaggacagagtcacgattaccgcggacaaatccacgagcacagcctacatggagctgagcagcctgagatctgaggacacggccgtgtattactgtgcgagaccccaagtccactatgattacaacgggtttccttactggggccaaggaaccctggtcaccgtctcctcaggtggaggcggttcaggcggaggtggatccggcggtggcggatcgggtggcggcggatctgacatccagatgacccagtctccttccaccctgtctgcatctgtaggagacagagtcaccatcacttgcagtgccagctcaagtgtaagttacatgaactggtatcagcagaaaccagggaaagcccctaagagatggatttatgactcatccaaactggcttctggggtcccatcaaggttcagcggcagtggatctgggacagaattcactctcaccatcagcagcctgcagcctgatgattttgcaacttattactgccaacagtggagtcgtaacccacccactttcggcggagggaccaaggtggagatcaaacggtcctccagctaa

SEQ ID NO: 48 - protein, 503 aa, Artificial Sequence
  TSC371 CD3-binding domain
EPKSSDKTHTCPPCPAPEAAGAPSVFLFPPKPKDTLMISRTPEVTCVVVDVSHEDPEVKFNWYVDGVEVHNAKTKPREEQYNSTYRVVSVLTVLHQDWLNGKAYACAVSNKALPAPIEKTISKAKGQPREPQVYTLPPSRDELTKNQVSLTCLVKGFYPSDIAVEWESNGQPENNYKTTPPVLDSDGSFFLYSKLTVDKSRWQQGNVFSCSVMHEALHNHYTQKSLSLSPGQRHNNSSLNTGTQMAGHSPNSQVQLVQSGAEVKKPGSSVKVSCKASGGTFSRSTMHWVRQAPGQGLEWIGYINPSSAYTNYNQKFKDRVTITADKSTSTAYMELSSLRSEDTAVYYCARPQVHYDYNGFPYWGQGTLVTVSSGGGGSGGGGSGGGGSGGGGSDIQMTQSPSTLSASVGDRVTITCSASSSVSYMNWYQQKPGKAPKRWIYDSSKLASGVPSRFSGSGSGTEFTLTISSLQPDDFATYYCQQWSRNPPTFGGGTKVEIKRSSS

SEQ ID NO: 49 - DNA, 1572 bp, Artificial Sequence
  TSC372 CD3-binding domain
atggaagcaccagcgcagcttctcttcctcctgctactctggctcccagataccaccggtgagcccaaatcttctgacaaaactcacacatgcccaccgtgcccagcacctgaagccgcgggtgcaccgtcagtcttcctcttccccccaaaacccaaggacaccctcatgatctcccggacccctgaggtcacatgcgtggtggtggacgtgagccacgaagaccctgaggtcaagttcaactggtacgtggacggcgtggaggtgcataatgccaagacaaagccgcgggaggagcagtacaacagcacgtaccgtgtggtcagcgtcctcaccgtcctgcaccaggactggctgaatggcaaggcatacgcatgcgcggtctccaacaaagccctcccagcccccatcgagaaaaccatctccaaagccaaagggcagccccgagaaccacaggtgtacaccctgcccccatcccgggatgagctgaccaagaaccaggtcagcctgacctgcctggtcaaaggcttctatccaagcgacatcgccgtggagtgggagagcaatgggcagccggagaacaactacaagaccacgcctcccgtgctggactccgacggctccttcttcctctacagcaagctcaccgtggacaagagcaggtggcagcaggggaacgtcttctcatgctccgtgatgcatgaggctctgcacaaccactacacgcagaagagcctctccctgtctccgggtcagaggcacaacaattcttccctgaatacaggaactcagatggcaggtcattctccgaattctcaggtccagctggtgcaatctggggctgaggtgaagaagcctgggtcctcggtgaaggtctcctgcaaggcttctggaggcaccttcagcagatctacgatgcactgggtgcgacaggcccctggacaagggcttgagtggatgggatacattaatcctagcagtgcttatactaattacaatcagaaattcaaggacagagtcacgattaccgcggacaaatccacgagcacagcctacatggagctgagcagcctgagatctgaggacacggccgtgtattactgtgcgagaccccaagtccactatgattacaacgggtttccttactggggccaaggaaccctggtcaccgtctcctcaggtggaggcggttcaggcggaggtggatccggcggtggcggatcgggtggcggcggatctgacatccagatgacccagtctccttccaccctgtctgcatctgtaggagacagagtcaccatgacttgcagtgccagctcaagtgtaagttacatgaactggtatcagcagaaaccagggaaagcccctaagagatggatttatgactcatccaaactggcttctggggtcccatcaaggttcagcggcagtggatctgggacagaattcactctcaccatcagcagcctgcagcctgatgattttgcaacttattactgccaacagtggagtcgtaacccacccactttcggcggagggaccaaggtggagatcaaacggtcctccagctaa

SEQ ID NO: 50 - protein, 503 aa, Artificial Sequence
  TSC372 CD3-binding domain
EPKSSDKTHTCPPCPAPEAAGAPSVFLFPPKPKDTLMISRTPEVTCVVVDVSHEDPEVKFNWYVDGVEVHNAKTKPREEQYNSTYRVVSVLTVLHQDWLNGKAYACAVSNKALPAPIEKTISKAKGQPREPQVYTLPPSRDELTKNQVSLTCLVKGFYPSDIAVEWESNGQPENNYKTTPPVLDSDGSFFLYSKLTVDKSRWQQGNVFSCSVMHEALHNHYTQKSLSLSPGQRHNNSSLNTGTQMAGHSPNSQVQLVQSGAEVKKPGSSVKVSCKASGGTFSRSTMHWVRQAPGQGLEWMGYINPSSAYTNYNQKFKDRVTITADKSTSTAYMELSSLRSEDTAVYYCARPQVHYDYNGFPYWGQGTLVTVSSGGGGSGGGGSGGGGSGGGGSDIQMTQSPSTLSASVGDRVTMTCSASSSVSYMNWYQQKPGKAPKRWIYDSSKLASGVPSRFSGSGSGTEFTLTISSLQPDDFATYYCQQWSRNPPTFGGGTKVEIKRSSS

SEQ ID NO: 51 - DNA, 1572 bp, Artificial Sequence
  TSC390 CD3-binding domain
atggaagcaccagcgcagcttctcttcctcctgctactctggctcccagataccaccggtgagcccaaatcttctgacaaaactcacacatgcccaccgtgcccagcacctgaagccgcgggtgcaccgtcagtcttcctcttccccccaaaacccaaggacaccctcatgatctcccggacccctgaggtcacatgcgtggtggtggacgtgagccacgaagaccctgaggtcaagttcaactggtacgtggacggcgtggaggtgcataatgccaagacaaagccgcgggaggagcagtacaacagcacgtaccgtgtggtcagcgtcctcaccgtcctgcaccaggactggctgaatggcaaggcatacgcatgcgcggtctccaacaaagccctcccagcccccatcgagaaaaccatctccaaagccaaagggcagccccgagaaccacaggtgtacaccctgcccccatcccgggatgagctgaccaagaaccaggtcagcctgacctgcctggtcaaaggcttctatccaagcgacatcgccgtggagtgggagagcaatgggcagccggagaacaactacaagaccacgcctcccgtgctggactccgacggctccttcttcctctacagcaagctcaccgtggacaagagcaggtggcagcaggggaacgtcttctcatgctccgtgatgcatgaggctctgcacaaccactacacgcagaagagcctctccctgtctccgggtcagaggcacaacaattcttccctgaatacaggaactcagatggcaggtcattctccgaattctcaggtccagctggtgcaatctgggcctgaggtgaagaagcctgggtcctcggtgaaggtctcctgcaaggcttctggatataccttcagcagatctacgatgcactgggtgcgacaggcccctggacaagggcttgagtggatgggatacattaatcctagcagtgcttatactaattacaatcagaaattcaaggacagagtcacgattaccgcggacaaatccacgagcacagcctacatggagctgagcagcctgagatctgaggacacggccgtgtattactgtgcgagaccccaagtccactatgattacaacgggtttccttactggggccaaggaaccctggtcaccgtctcctcaggtggaggcggttcaggcggaggtggatccggcggtggcggatcgggtggcggcggatctgacatccagatgacccagtctccttccaccctgtctgcatctgtaggagacagagtcaccatcacttgcagtgccagctcaagtgtaagttacatgaactggtatcagcagaaaccagggaaagcccctaagagatggatttatgactcatccaaactggcttctggggtcccatcaaggttcagcggcagtggatctgggacagagttcactctcaccatcagcagcctgcagcctgatgattttgcaacttattactgccaacagtggagtcgtaacccacccactttcggcggagggaccaaggtggagatcaaacggtcctccagctaa

SEQ ID NO: 52 - protein, 503 aa, Artificial Sequence
  TSC390 CD3-binding domain
EPKSSDKTHTCPPCPAPEAAGAPSVFLFPPKPKDTLMISRTPEVTCVVVDVSHEDPEVKFNWYVDGVEVHNAKTKPREEQYNSTYRVVSVLTVLHQDWLNGKAYACAVSNKALPAPIEKTISKAKGQPREPQVYTLPPSRDELTKNQVSLTCLVKGFYPSDIAVEWESNGQPENNYKTTPPVLDSDGSFFLYSKLTVDKSRWQQGNVFSCSVMHEALHNHYTQKSLSLSPGQRHNNSSLNTGTQMAGHSPNSQVQLVQSGPEVKKPGSSVKVSCKASGYTFSRSTMHWVRQAPGQGLEWMGYINPSSAYTNYNQKFKDRVTITADKSTSTAYMELSSLRSEDTAVYYCARPQVHYDYNGFPYWGQGTLVTVSSGGGGSGGGGSGGGGSGGGGSDIQMTQSPSTLSASVGDRVTITCSASSSVSYMNWYQQKPGKAPKRWIYDSSKLASGVPSRFSGSGSGTEFTLTISSLQPDDFATYYCQQWSRNPPTFGGGTKVEIKRSSS

SEQ ID NO: 53 - DNA, 1572 bp, Artificial Sequence
  TSC391 CD3-binding domain
atggaagcaccagcgcagcttctcttcctcctgctactctggctcccagataccaccggtgagcccaaatcttctgacaaaactcacacatgcccaccgtgcccagcacctgaagccgcgggtgcaccgtcagtcttcctcttccccccaaaacccaaggacaccctcatgatctcccggacccctgaggtcacatgcgtggtggtggacgtgagccacgaagaccctgaggtcaagttcaactggtacgtggacggcgtggaggtgcataatgccaagacaaagccgcgggaggagcagtacaacagcacgtaccgtgtggtcagcgtcctcaccgtcctgcaccaggactggctgaatggcaaggcatacgcatgcgcggtctccaacaaagccctcccagcccccatcgagaaaaccatctccaaagccaaagggcagccccgagaaccacaggtgtacaccctgcccccatcccgggatgagctgaccaagaaccaggtcagcctgacctgcctggtcaaaggcttctatccaagcgacatcgccgtggagtgggagagcaatgggcagccggagaacaactacaagaccacgcctcccgtgctggactccgacggctccttcttcctctacagcaagctcaccgtggacaagagcaggtggcagcaggggaacgtcttctcatgctccgtgatgcatgaggctctgcacaaccactacacgcagaagagcctctccctgtctccgggtcagaggcacaacaattcttccctgaatacaggaactcagatggcaggtcattctccgaattctcaggtccagctggtgcaatctgggcctgaggtgaagaagcctgggtcctcggtgaaggtctcctgcaaggcttctggatataccttcagcagatctacgatgcactgggtgcgacaggcccctggacaagggcttgagtggataggatacattaatcctagcagtgcttatactaattacaatcagaaattcaaggacagagtcacgattaccgcggacaaatccacgagcacagcctacatggagctgagcagcctgagatctgaggacacggccgtgtattactgtgcgagaccccaagtccactatgattacaacgggtttccttactggggccaaggaaccctggtcaccgtctcctcaggtggaggcggttcaggcggaggtggatccggcggtggcggatcgggtggcggcggatctgacatccagatgacccagtctccttccaccctgtctgcatctgtaggagacagagtcaccatcacttgcagtgccagctcaagtgtaagttacatgaactggtatcagcagaaaccagggaaagcccctaagagatggatttatgactcatccaaactggcttctggggtcccatcaaggttcagcggcagtggatctgggacagagttcactctcaccatcagcagcctgcagcctgatgattttgcaacttattactgccaacagtggagtcgtaacccacccactttcggcggagggaccaaggtggagatcaaacggtcctccagctaa

SEQ ID NO: 54 - protein, 503 aa, Artificial Sequence
  TSC391 CD3-binding domain
EPKSSDKTHTCPPCPAPEAAGAPSVFLFPPKPKDTLMISRTPEVTCVVVDVSHEDPEVKFNWYVDGVEVHNAKTKPREEQYNSTYRVVSVLTVLHQDWLNGKAYACAVSNKALPAPIEKTISKAKGQPREPQVYTLPPSRDELTKNQVSLTCLVKGFYPSDIAVEWESNGQPENNYKTTPPVLDSDGSFFLYSKLTVDKSRWQQGNVFSCSVMHEALHNHYTQKSLSLSPGQRHNNSSLNTGTQMAGHSPNSQVQLVQSGPEVKKPGSSVKVSCKASGYTFSRSTMHWVRQAPGQGLEWIGYINPSSAYTNYNQKFKDRVTITADKSTSTAYMELSSLRSEDTAVYYCARPQVHYDYNGFPYWGQGTLVTVSSGGGGSGGGGSGGGGSGGGGSDIQMTQSPSTLSASVGDRVTITCSASSSVSYMNWYQQKPGKAPKRWIYDSSKLASGVPSRFSGSGSGTEFTLTISSLQPDDFATYYCQQWSRNPPTFGGGTKVEIKRSSS

SEQ ID NO: 55 - DNA, 1572 bp, Artificial Sequence
  TSC392 CD3-binding domain
atggaagcaccagcgcagcttctcttcctcctgctactctggctcccagataccaccggtgagcccaaatcttctgacaaaactcacacatgcccaccgtgcccagcacctgaagccgcgggtgcaccgtcagtcttcctcttccccccaaaacccaaggacaccctcatgatctcccggacccctgaggtcacatgcgtggtggtggacgtgagccacgaagaccctgaggtcaagttcaactggtacgtggacggcgtggaggtgcataatgccaagacaaagccgcgggaggagcagtacaacagcacgtaccgtgtggtcagcgtcctcaccgtcctgcaccaggactggctgaatggcaaggcatacgcatgcgcggtctccaacaaagccctcccagcccccatcgagaaaaccatctccaaagccaaagggcagccccgagaaccacaggtgtacaccctgcccccatcccgggatgagctgaccaagaaccaggtcagcctgacctgcctggtcaaaggcttctatccaagcgacatcgccgtggagtgggagagcaatgggcagccggagaacaactacaagaccacgcctcccgtgctggactccgacggctccttcttcctctacagcaagctcaccgtggacaagagcaggtggcagcaggggaacgtcttctcatgctccgtgatgcatgaggctctgcacaaccactacacgcagaagagcctctccctgtctccgggtcagaggcacaacaattcttccctgaatacaggaactcagatggcaggtcattctccgaattctcaggtccagctggtgcaatctgggcctgaggtgaagaagcctgggtcctcggtgaaggtctcctgcaaggcttctggatataccttcagcagatctacgatgcactgggtgcgacaggcccctggacaagggcttgagtggatgggatacattaatcctagcagtgcttatactaattacaatcagaaattcaaggacagagtcacgattaccgcggacaaatccacgagcacagcctacatggagctgagcagcctgagatctgaggacacggccgtgtattactgtgcgagaccccaagtccactatgattacaacgggtttccttactggggccaaggaaccctggtcaccgtctcctcaggtggaggcggttcaggcggaggtggatccggcggtggcggatcgggtggcggcggatctgacatccagatgacccagtctccttccaccctgtctgcatctgtaggagacagagtcaccatgacttgcagtgccagctcaagtgtaagttacatgaactggtatcagcagaaaccagggaaagcccctaagagatggatttatgactcatccaaactggcttctggggtcccatcaaggttcagcggcagtggatctgggacagagttcactctcaccatcagcagcctgcagcctgatgattttgcaacttattactgccaacagtggagtcgtaacccacccactttcggcggagggaccaaggtggagatcaaacggtcctccagctaa

SEQ ID NO: 56 - protein, 503 aa, Artificial Sequence
  TSC392 CD3-binding domain
EPKSSDKTHTCPPCPAPEAAGAPSVFLFPPKPKDTLMISRTPEVTCVVVDVSHEDPEVKFNWYVDGVEVHNAKTKPREEQYNSTYRVVSVLTVLHQDWLNGKAYACAVSNKALPAPIEKTISKAKGQPREPQVYTLPPSRDELTKNQVSLTCLVKGFYPSDIAVEWESNGQPENNYKTTPPVLDSDGSFFLYSKLTVDKSRWQQGNVFSCSVMHEALHNHYTQKSLSLSPGQRHNNSSLNTGTQMAGHSPNSQVQLVQSGPEVKKPGSSVKVSCKASGYTFSRSTMHWVRQAPGQGLEWMGYINPSSAYTNYNQKFKDRVTITADKSTSTAYMELSSLRSEDTAVYYCARPQVHYDYNGFPYWGQGTLVTVSSGGGGSGGGGSGGGGSGGGGSDIQMTQSPSTLSASVGDRVTMTCSASSSVSYMNWYQQKPGKAPKRWIYDSSKLASGVPSRFSGSGSGTEFTLTISSLQPDDFATYYCQQWSRNPPTFGGGTKVEIKRSSS

SEQ ID NO: 57 - DNA, 1572 bp, Artificial Sequence
  TSC393 CD3-binding domain
atggaagcaccagcgcagcttctcttcctcctgctactctggctcccagataccaccggtgagcccaaatcttctgacaaaactcacacatgcccaccgtgcccagcacctgaagccgcgggtgcaccgtcagtcttcctcttccccccaaaacccaaggacaccctcatgatctcccggacccctgaggtcacatgcgtggtggtggacgtgagccacgaagaccctgaggtcaagttcaactggtacgtggacggcgtggaggtgcataatgccaagacaaagccgcgggaggagcagtacaacagcacgtaccgtgtggtcagcgtcctcaccgtcctgcaccaggactggctgaatggcaaggcatacgcatgcgcggtctccaacaaagccctcccagcccccatcgagaaaaccatctccaaagccaaagggcagccccgagaaccacaggtgtacaccctgcccccatcccgggatgagctgaccaagaaccaggtcagcctgacctgcctggtcaaaggcttctatccaagcgacatcgccgtggagtgggagagcaatgggcagccggagaacaactacaagaccacgcctcccgtgctggactccgacggctccttcttcctctacagcaagctcaccgtggacaagagcaggtggcagcaggggaacgtcttctcatgctccgtgatgcatgaggctctgcacaaccactacacgcagaagagcctctccctgtctccgggtcagaggcacaacaattcttccctgaatacaggaactcagatggcaggtcattctccgaattctcaggtccagctggtgcaatctggggctgaggtgaagaagcctgggtcctcggtgaaggtctcctgcaaggcttctggatataccttcagcagatctacgatgcactgggtgcgacaggcccctggacaagggcttgagtggataggatacattaatcctagcagtgcttatactaattacaatcagaaattcaaggacagagtcacgattaccgcggacaaatccacgagcacagcctacatggagctgagcagcctgagatctgaggacacggccgtgtattactgtgcgagaccccaagtccactatgattacaacgggtttccttactggggccaaggaaccctggtcaccgtctcctcaggtggaggcggttcaggcggaggtggatccggcggtggcggatcgggtggcggcggatctgacatccagatgacccagtctccttccaccctgtctgcatctgtaggagacagagtcaccatgacttgcagtgccagctcaagtgtaagttacatgaactggtatcagcagaaaccagggaaagcccctaagagatggatttatgactcatccaaactggcttctggggtcccatcaaggttcagcggcagtggatctgggacagagttcactctcaccatcagcagcctgcagcctgatgattttgcaacttattactgccaacagtggagtcgtaacccacccactttcggcggagggaccaaggtggagatcaaacggtcctccagctaa

SEQ ID NO: 58 - protein, 503 aa, Artificial Sequence
  TSC393 CD3-binding domain
EPKSSDKTHTCPPCPAPEAAGAPSVFLFPPKPKDTLMISRTPEVTCVVVDVSHEDPEVKFNWYVDGVEVHNAKTKPREEQYNSTYRVVSVLTVLHQDWLNGKAYACAVSNKALPAPIEKTISKAKGQPREPQVYTLPPSRDELTKNQVSLTCLVKGFYPSDIAVEWESNGQPENNYKTTPPVLDSDGSFFLYSKLTVDKSRWQQGNVFSCSVMHEALHNHYTQKSLSLSPGQRHNNSSLNTGTQMAGHSPNSQVQLVQSGAEVKKPGSSVKVSCKASGYTFSRSTMHWVRQAPGQGLEWIGYINPSSAYTNYNQKFKDRVTITADKSTSTAYMELSSLRSEDTAVYYCARPQVHYDYNGFPYWGQGTLVTVSSGGGGSGGGGSGGGGSGGGGSDIQMTQSPSTLSASVGDRVTMTCSASSSVSYMNWYQQKPGKAPKRWIYDSSKLASGVPSRFSGSGSGTEFTLTISSLQPDDFATYYCQQWSRNPPTFGGGTKVEIKRSSS

SEQ ID NO: 59 - DNA, 1572 bp, Artificial Sequence
  TSC394 CD3-binding domain
atggaagcaccagcgcagcttctcttcctcctgctactctggctcccagataccaccggtgagcccaaatcttctgacaaaactcacacatgcccaccgtgcccagcacctgaagccgcgggtgcaccgtcagtcttcctcttccccccaaaacccaaggacaccctcatgatctcccggacccctgaggtcacatgcgtggtggtggacgtgagccacgaagaccctgaggtcaagttcaactggtacgtggacggcgtggaggtgcataatgccaagacaaagccgcgggaggagcagtacaacagcacgtaccgtgtggtcagcgtcctcaccgtcctgcaccaggactggctgaatggcaaggcatacgcatgcgcggtctccaacaaagccctcccagcccccatcgagaaaaccatctccaaagccaaagggcagccccgagaaccacaggtgtacaccctgcccccatcccgggatgagctgaccaagaaccaggtcagcctgacctgcctggtcaaaggcttctatccaagcgacatcgccgtggagtgggagagcaatgggcagccggagaacaactacaagaccacgcctcccgtgctggactccgacggctccttcttcctctacagcaagctcaccgtggacaagagcaggtggcagcaggggaacgtcttctcatgctccgtgatgcatgaggctctgcacaaccactacacgcagaagagcctctccctgtctccgggtcagaggcacaacaattcttccctgaatacaggaactcagatggcaggtcattctccgaattctcaggtccagctggtgcaatctgggcctgaggtgaagaagcctgggtcctcggtgaaggtctcctgcaaggcttctggatataccttcagcagatctacgatgcactgggtgcgacaggcccctggacaagggcttgagtggataggatacattaatcctagcagtgcttatactaattacaatcagaaattcaaggacagagtcacgattaccgcggacaaatccacgagcacagcctacatggagctgagcagcctgagatctgaggacacggccgtgtattactgtgcgagaccccaagtccactatgattacaacgggtttccttactggggccaaggaaccctggtcaccgtctcctcaggtggaggcggttcaggcggaggtggatccggcggtggcggatcgggtggcggcggatctgacatccagatgacccagtctccttccaccctgtctgcatctgtaggagacagagtcaccatgacttgcagtgccagctcaagtgtaagttacatgaactggtatcagcagaaaccagggaaagcccctaagagatggatttatgactcatccaaactggcttctggggtcccatcaaggttcagcggcagtggatctgggacagagttcactctcaccatcagcagcctgcagcctgatgattttgcaacttattactgccaacagtggagtcgtaacccacccactttcggcggagggaccaaggtggagatcaaacggtcctccagctaa

SEQ ID NO: 60 - protein, 503 aa, Artificial Sequence
  TSC394 CD3-binding domain
EPKSSDKTHTCPPCPAPEAAGAPSVFLFPPKPKDTLMISRTPEVTCVVVDVSHEDPEVKFNWYVDGVEVHNAKTKPREEQYNSTYRVVSVLTVLHQDWLNGKAYACAVSNKALPAPIEKTISKAKGQPREPQVYTLPPSRDELTKNQVSLTCLVKGFYPSDIAVEWESNGQPENNYKTTPPVLDSDGSFFLYSKLTVDKSRWQQGNVFSCSVMHEALHNHYTQKSLSLSPGQRHNNSSLNTGTQMAGHSPNSQVQLVQSGPEVKKPGSSVKVSCKASGYTFSRSTMHWVRQAPGQGLEWIGYINPSSAYTNYNQKFKDRVTITADKSTSTAYMELSSLRSEDTAVYYCARPQVHYDYNGFPYWGQGTLVTVSSGGGGSGGGGSGGGGSGGGGSDIQMTQSPSTLSASVGDRVTMTCSASSSVSYMNWYQQKPGKAPKRWIYDSSKLASGVPSRFSGSGSGTEFTLTISSLQPDDFATYYCQQWSRNPPTFGGGTKVEIKRSSS

SEQ ID NO: 61 - DNA, 2301 bp, Artificial Sequence
  TSC408 Anti-PSMA X anti-CD3 bispecific molecule
atggaagcaccagcgcagcttctcttcctcctgctactctggctcccagataccaccggtgatatccagatgacccagtctccatccgccatgtctgcatctgtaggagacagagtcaccatcacttgccgggcgagtaagagcattagcaaatatttagcctggtttcagcagaaaccagggaaagttcctaagctccgcatccattctggatctactttgcaatcaggggtcccatctcggttcagtggcagtggatctgggacagaatttactctcaccatcagcagcctgcagcctgaagattttgcaacttattactgtcaacagcatattgaatacccgtggacgttcggccaagggaccaaggtggaaatcaaacgaggtggcggagggtctgggggtggcggatccggaggtggtggctctcaggtccagctggtacagtctggggctgaggtgaagaagcctggggcttcagtgaaggtctcctgcaaggcttctggatacacattcactgactactacatgcactgggtgcgacaggcccctggacaagggcttgagtggatgggatattttaatccttataatgattatactagatacgcacagaagttccagggcagagtcaccatgaccagggacacgtctatcagcacagcctacatggagctgagcagcctgagatctgacgacacggccgtgtattactgtgcaagatcggatggttactacgatgctatggactactggggtcaaggaaccacagtcaccgtctcctcgagtgagcccaaatcttctgacaaaactcacacatgcccaccgtgcccagcacctgaagccgcgggtgcaccgtcagtcttcctcttccccccaaaacccaaggacaccctcatgatctcccggacccctgaggtcacatgcgtggtggtggacgtgagccacgaagaccctgaggtcaagttcaactggtacgtggacggcgtggaggtgcataatgccaagacaaagccgcgggaggagcagtacaacagcacgtaccgtgtggtcagcgtcctcaccgtcctgcaccaggactggctgaatggcaaggcgtacgcgtgcgcggtctccaacaaagccctcccagcccccatcgagaaaaccatctccaaagccaaagggcagccccgagaaccacaggtgtacaccctgcccccatcccgggatgagctgaccaagaaccaggtcagcctgacctgcctggtcaaaggcttctatccaagcgacatcgccgtggagtgggagagcaatgggcagccggagaacaactacaagaccacgcctcccgtgctggactccgacggctccttcttcctctacagcaagctcaccgtggacaagagcaggtggcagcaggggaacgtcttctcatgctccgtgatgcatgaggctctgcacaaccactacacgcagaagagcctctccctgtctccgggtcagaggcacaacaattcttccctgaatacaggaactcagatggcaggtcattctccgaattctcaggtccagctggtgcaatctgggcctgaggtgaagaagcctgggtcctcggtgaaggtctcctgcaaggcttctggatataccttcagcagatctacgatgcactgggtgcgacaggcccctggacaagggcttgagtggataggatacattaatcctagcagtgcttatactaattacaatcagaaattcaaggacagagtcacgattaccgcggacaaatccacgagcacagcctacatggagctgagcagcctgagatctgaggacacggccgtgtattactgtgcgagaccccaagtccactatgattacaacgggtttccttactggggccaaggaaccctggtcaccgtctcctcaggtggaggcggttcaggcggaggtggatccggcggtggcggatcgggtggcggcggatctgacatccagatgacccagtctccttccaccctgtctgcatctgtaggagacagagtcaccatcacttgcagtgccagctcaagtgtaagttacatgaactggtatcagcagaaaccagggaaagcccctaagagatggatttatgactcatccaaactggcttctggggtcccatcaaggttcagcggcagtggatctgggacagagttcactctcaccatcagcagcctgcagcctgatgattttgcaacttattactgccaacagtggagtcgtaacccacccactttcggcggagggaccaaggtggagatcaaacggtcctccagctaa

SEQ ID NO: 62 - protein, 746 aa, Artificial Sequence
  TSC408 Anti-PSMA X anti-CD3 bispecific molecule
DIQMTQSPSAMSASVGDRVTITCRASKSISKYLAWFQQKPGKVPKLRIHSGSTLQSGVPSRFSGSGSGTEFTLTISSLQPEDFATYYCQQHIEYPWTFGQGTKVEIKRGGGGSGGGGSGGGGSQVQLVQSGAEVKKPGASVKVSCKASGYTFTDYYMHWVRQAPGQGLEWMGYFNPYNDYTRYAQKFQGRVTMTRDTSISTAYMELSSLRSDDTAVYYCARSDGYYDAMDYWGQGTTVTVSSSEPKSSDKTHTCPPCPAPEAAGAPSVFLFPPKPKDTLMISRTPEVTCVVVDVSHEDPEVKFNWYVDGVEVHNAKTKPREEQYNSTYRVVSVLTVLHQDWLNGKAYACAVSNKALPAPIEKTISKAKGQPREPQVYTLPPSRDELTKNQVSLTCLVKGFYPSDIAVEWESNGQPENNYKTTPPVLDSDGSFFLYSKLTVDKSRWQQGNVFSCSVMHEALHNHYTQKSLSLSPGQRHNNSSLNTGTQMAGHSPNSQVQLVQSGPEVKKPGSSVKVSCKASGYTFSRSTMHWVRQAPGQGLEWIGYINPSSAYTNYNQKFKDRVTITADKSTSTAYMELSSLRSEDTAVYYCARPQVHYDYNGFPYWGQGTLVTVSSGGGGSGGGGSGGGGSGGGGSDIQMTQSPSTLSASVGDRVTITCSASSSVSYMNWYQQKPGKAPKRWIYDSSKLASGVPSRFSGSGSGTEFTLTISSLQPDDFATYYCQQWSRNPPTFGGGTKVEIKRSSS

SEQ ID NO: 63 - DNA, 2301 bp, Artificial Sequence
  TSC409 Anti-PSMA X anti-CD3 bispecific molecule
atggaagcaccagcgcagcttctcttcctcctgctactctggctcccagataccaccggtgatatccagatgacccagtctccatccgccatgtctgcatctgtaggagacagagtcaccatcacttgccgggcgagtaagagcattagcaaatatttagcctggtttcagcagaaaccagggaaagttcctaagctccgcatccattctggatctactttgcaatcaggggtcccatctcggttcagtggcagtggatctgggacagaatttactctcaccatcagcagcctgcagcctgaagattttgcaacttattactgtcaacagcatattgaatacccgtggacgttcggccaagggaccaaggtggaaatcaaacgaggtggcggagggtctgggggtggcggatccggaggtggtggctctcaggtccagctggtacagtctggggctgaggtgaagaagcctggggcttcagtgaaggtctcctgcaaggcttctggatacacattcactgactactacatgcactgggtgcgacaggcccctggacaagggcttgagtggatgggatattttaatccttataatgattatactagatacgcacagaagttccagggcagagtcaccatgaccagggacacgtctatcagcacagcctacatggagctgagcagcctgagatctgacgacacggccgtgtattactgtgcaagatcggatggttactacgatgctatggactactggggtcaaggaaccacagtcaccgtctcctcgagtgagcccaaatcttctgacaaaactcacacatgcccaccgtgcccagcacctgaagccgcgggtgcaccgtcagtcttcctcttccccccaaaacccaaggacaccctcatgatctcccggacccctgaggtcacatgcgtggtggtggacgtgagccacgaagaccctgaggtcaagttcaactggtacgtggacggcgtggaggtgcataatgccaagacaaagccgcgggaggagcagtacaacagcacgtaccgtgtggtcagcgtcctcaccgtcctgcaccaggactggctgaatggcaaggcgtacgcgtgcgcggtctccaacaaagccctcccagcccccatcgagaaaaccatctccaaagccaaagggcagccccgagaaccacaggtgtacaccctgcccccatcccgggatgagctgaccaagaaccaggtcagcctgacctgcctggtcaaaggcttctatccaagcgacatcgccgtggagtgggagagcaatgggcagccggagaacaactacaagaccacgcctcccgtgctggactccgacggctccttcttcctctacagcaagctcaccgtggacaagagcaggtggcagcaggggaacgtcttctcatgctccgtgatgcatgaggctctgcacaaccactacacgcagaagagcctctccctgtctccgggtcagaggcacaacaattcttccctgaatacaggaactcagatggcaggtcattctccgaattctcaggtccagctggtgcaatctgggcctgaggtgaagaagcctgggtcctcggtgaaggtctcctgcaaggcttctggatataccttcagcagatctacgatgcactgggtgcgacaggcccctggacaagggcttgagtggatgggatacattaatcctagcagtgcttatactaattacaatcagaaattcaaggacagagtcacgattaccgcggacaaatccacgagcacagcctacatggagctgagcagcctgagatctgaggacacggccgtgtattactgtgcgagaccccaagtccactatgattacaacgggtttccttactggggccaaggaaccctggtcaccgtctcctcaggtggaggcggttcaggcggaggtggatccggcggtggcggatcgggtggcggcggatctgacatccagatgacccagtctccttccaccctgtctgcatctgtaggagacagagtcaccatgacttgcagtgccagctcaagtgtaagttacatgaactggtatcagcagaaaccagggaaagcccctaagagatggatttatgactcatccaaactggcttctggggtcccatcaaggttcagcggcagtggatctgggacagagttcactctcaccatcagcagcctgcagcctgatgattttgcaacttattactgccaacagtggagtcgtaacccacccactttcggcggagggaccaaggtggagatcaaacggtcctccagctaa

SEQ ID NO: 64 - protein, 746 aa, Artificial Sequence
  TSC409 Anti-PSMA X anti-CD3 bispecific molecule
DIQMTQSPSAMSASVGDRVTITCRASKSISKYLAWFQQKPGKVPKLRIHSGSTLQSGVPSRFSGSGSGTEFTLTISSLQPEDFATYYCQQHIEYPWTFGQGTKVEIKRGGGGSGGGGSGGGGSQVQLVQSGAEVKKPGASVKVSCKASGYTFTDYYMHWVRQAPGQGLEWMGYFNPYNDYTRYAQKFQGRVTMTRDTSISTAYMELSSLRSDDTAVYYCARSDGYYDAMDYWGQGTTVTVSSSEPKSSDKTHTCPPCPAPEAAGAPSVFLFPPKPKDTLMISRTPEVTCVVVDVSHEDPEVKFNWYVDGVEVHNAKTKPREEQYNSTYRVVSVLTVLHQDWLNGKAYACAVSNKALPAPIEKTISKAKGQPREPQVYTLPPSRDELTKNQVSLTCLVKGFYPSDIAVEWESNGQPENNYKTTPPVLDSDGSFFLYSKLTVDKSRWQQGNVFSCSVMHEALHNHYTQKSLSLSPGQRHNNSSLNTGTQMAGHSPNSQVQLVQSGPEVKKPGSSVKVSCKASGYTFSRSTMHWVRQAPGQGLEWMGYINPSSAYTNYNQKFKDRVTITADKSTSTAYMELSSLRSEDTAVYYCARPQVHYDYNGFPYWGQGTLVTVSSGGGGSGGGGSGGGGSGGGGSDIQMTQSPSTLSASVGDRVTMTCSASSSVSYMNWYQQKPGKAPKRWIYDSSKLASGVPSRFSGSGSGTEFTLTISSLQPDDFATYYCQQWSRNPPTFGGGTKVEIKRSSS

SEQ ID NO: 65 - DNA, 2301 bp, Artificial Sequence
  TSC410 Anti-PSMA X anti-CD3 bispecific molecule
atggaagcaccagcgcagcttctcttcctcctgctactctggctcccagataccaccggtgatatccagatgacccagtctccatccgccatgtctgcatctgtaggagacagagtcaccatcacttgccgggcgagtaagagcattagcaaatatttagcctggtttcagcagaaaccagggaaagttcctaagctccgcatccattctggatctactttgcaatcaggggtcccatctcggttcagtggcagtggatctgggacagaatttactctcaccatcagcagcctgcagcctgaagattttgcaacttattactgtcaacagcatattgaatacccgtggacgttcggccaagggaccaaggtggaaatcaaacgaggtggcggagggtctgggggtggcggatccggaggtggtggctctcaggtccagctggtacagtctggggctgaggtgaagaagcctggggcttcagtgaaggtctcctgcaaggcttctggatacacattcactgactactacatgcactgggtgcgacaggcccctggacaagggcttgagtggatgggatattttaatccttataatgattatactagatacgcacagaagttccagggcagagtcaccatgaccagggacacgtctatcagcacagcctacatggagctgagcagcctgagatctgacgacacggccgtgtattactgtgcaagatcggatggttactacgatgctatggactactggggtcaaggaaccacagtcaccgtctcctcgagtgagcccaaatcttctgacaaaactcacacatgcccaccgtgcccagcacctgaagccgcgggtgcaccgtcagtcttcctcttccccccaaaacccaaggacaccctcatgatctcccggacccctgaggtcacatgcgtggtggtggacgtgagccacgaagaccctgaggtcaagttcaactggtacgtggacggcgtggaggtgcataatgccaagacaaagccgcgggaggagcagtacaacagcacgtaccgtgtggtcagcgtcctcaccgtcctgcaccaggactggctgaatggcaaggcgtacgcgtgcgcggtctccaacaaagccctcccagcccccatcgagaaaaccatctccaaagccaaagggcagccccgagaaccacaggtgtacaccctgcccccatcccgggatgagctgaccaagaaccaggtcagcctgacctgcctggtcaaaggcttctatccaagcgacatcgccgtggagtgggagagcaatgggcagccggagaacaactacaagaccacgcctcccgtgctggactccgacggctccttcttcctctacagcaagctcaccgtggacaagagcaggtggcagcaggggaacgtcttctcatgctccgtgatgcatgaggctctgcacaaccactacacgcagaagagcctctccctgtctccgggtcagaggcacaacaattcttccctgaatacaggaactcagatggcaggtcattctccgaattctcaggtccagctggtgcaatctggggctgaggtgaagaagcctgggtcctcggtgaaggtctcctgcaaggcttctggatataccttcagcagatctacgatgcactgggtgcgacaggcccctggacaagggcttgagtggataggatacattaatcctagcagtgcttatactaattacaatcagaaattcaaggacagagtcacgattaccgcggacaaatccacgagcacagcctacatggagctgagcagcctgagatctgaggacacggccgtgtattactgtgcgagaccccaagtccactatgattacaacgggtttccttactggggccaaggaaccctggtcaccgtctcctcaggtggaggcggttcaggcggaggtggatccggcggtggcggatcgggtggcggcggatctgacatccagatgacccagtctccttccaccctgtctgcatctgtaggagacagagtcaccatgacttgcagtgccagctcaagtgtaagttacatgaactggtatcagcagaaaccagggaaagcccctaagagatggatttatgactcatccaaactggcttctggggtcccatcaaggttcagcggcagtggatctgggacagagttcactctcaccatcagcagcctgcagcctgatgattttgcaacttattactgccaacagtggagtcgtaacccacccactttcggcggagggaccaaggtggagatcaaacggtcctccagctaa

SEQ ID NO: 66 - protein, 746 aa, Artificial Sequence
  TSC410 Anti-PSMA X anti-CD3 bispecific molecule
DIQMTQSPSAMSASVGDRVTITCRASKSISKYLAWFQQKPGKVPKLRIHSGSTLQSGVPSRFSGSGSGTEFTLTISSLQPEDFATYYCQQHIEYPWTFGQGTKVEIKRGGGGSGGGGSGGGGSQVQLVQSGAEVKKPGASVKVSCKASGYTFTDYYMHWVRQAPGQGLEWMGYFNPYNDYTRYAQKFQGRVTMTRDTSISTAYMELSSLRSDDTAVYYCARSDGYYDAMDYWGQGTTVTVSSSEPKSSDKTHTCPPCPAPEAAGAPSVFLFPPKPKDTLMISRTPEVTCVVVDVSHEDPEVKFNWYVDGVEVHNAKTKPREEQYNSTYRVVSVLTVLHQDWLNGKAYACAVSNKALPAPIEKTISKAKGQPREPQVYTLPPSRDELTKNQVSLTCLVKGFYPSDIAVEWESNGQPENNYKTTPPVLDSDGSFFLYSKLTVDKSRWQQGNVFSCSVMHEALHNHYTQKSLSLSPGQRHNNSSLNTGTQMAGHSPNSQVQLVQSGAEVKKPGSSVKVSCKASGYTFSRSTMHWVRQAPGQGLEWIGYINPSSAYTNYNQKFKDRVTITADKSTSTAYMELSSLRSEDTAVYYCARPQVHYDYNGFPYWGQGTLVTVSSGGGGSGGGGSGGGGSGGGGSDIQMTQSPSTLSASVGDRVTMTCSASSSVSYMNWYQQKPGKAPKRWIYDSSKLASGVPSRFSGSGSGTEFTLTISSLQPDDFATYYCQQWSRNPPTFGGGTKVEIKRSSS

SEQ ID NO: 67 - DNA, 2301 bp, Artificial Sequence
  TSC411 Anti-PSMA X anti-CD3 bispecific molecule
atggaagcaccagcgcagcttctcttcctcctgctactctggctcccagataccaccggtgatatccagatgacccagtctccatccgccatgtctgcatctgtaggagacagagtcaccatcacttgccgggcgagtaagagcattagcaaatatttagcctggtttcagcagaaaccagggaaagttcctaagctccgcatccattctggatctactttgcaatcaggggtcccatctcggttcagtggcagtggatctgggacagaatttactctcaccatcagcagcctgcagcctgaagattttgcaacttattactgtcaacagcatattgaatacccgtggacgttcggccaagggaccaaggtggaaatcaaacgaggtggcggagggtctgggggtggcggatccggaggtggtggctctcaggtccagctggtacagtctggggctgaggtgaagaagcctggggcttcagtgaaggtctcctgcaaggcttctggatacacattcactgactactacatgcactgggtgcgacaggcccctggacaagggcttgagtggatgggatattttaatccttataatgattatactagatacgcacagaagttccagggcagagtcaccatgaccagggacacgtctatcagcacagcctacatggagctgagcagcctgagatctgacgacacggccgtgtattactgtgcaagatcggatggttactacgatgctatggactactggggtcaaggaaccacagtcaccgtctcctcgagtgagcccaaatcttctgacaaaactcacacatgcccaccgtgcccagcacctgaagccgcgggtgcaccgtcagtcttcctcttccccccaaaacccaaggacaccctcatgatctcccggacccctgaggtcacatgcgtggtggtggacgtgagccacgaagaccctgaggtcaagttcaactggtacgtggacggcgtggaggtgcataatgccaagacaaagccgcgggaggagcagtacaacagcacgtaccgtgtggtcagcgtcctcaccgtcctgcaccaggactggctgaatggcaaggcgtacgcgtgcgcggtctccaacaaagccctcccagcccccatcgagaaaaccatctccaaagccaaagggcagccccgagaaccacaggtgtacaccctgcccccatcccgggatgagctgaccaagaaccaggtcagcctgacctgcctggtcaaaggcttctatccaagcgacatcgccgtggagtgggagagcaatgggcagccggagaacaactacaagaccacgcctcccgtgctggactccgacggctccttcttcctctacagcaagctcaccgtggacaagagcaggtggcagcaggggaacgtcttctcatgctccgtgatgcatgaggctctgcacaaccactacacgcagaagagcctctccctgtctccgggtcagaggcacaacaattcttccctgaatacaggaactcagatggcaggtcattctccgaattctcaggtccagctggtgcaatctgggcctgaggtgaagaagcctgggtcctcggtgaaggtctcctgcaaggcttctggatataccttcagcagatctacgatgcactgggtgcgacaggcccctggacaagggcttgagtggataggatacattaatcctagcagtgcttatactaattacaatcagaaattcaaggacagagtcacgattaccgcggacaaatccacgagcacagcctacatggagctgagcagcctgagatctgaggacacggccgtgtattactgtgcgagaccccaagtccactatgattacaacgggtttccttactggggccaaggaaccctggtcaccgtctcctcaggtggaggcggttcaggcggaggtggatccggcggtggcggatcgggtggcggcggatctgacatccagatgacccagtctccttccaccctgtctgcatctgtaggagacagagtcaccatgacttgcagtgccagctcaagtgtaagttacatgaactggtatcagcagaaaccagggaaagcccctaagagatggatttatgactcatccaaactggcttctggggtcccatcaaggttcagcggcagtggatctgggacagagttcactctcaccatcagcagcctgcagcctgatgattttgcaacttattactgccaacagtggagtcgtaacccacccactttcggcggagggaccaaggtggagatcaaacggtcctccagctaa

SEQ ID NO: 68 - protein, 746 aa, Artificial Sequence
  TSC411 Anti-PSMA X anti-CD3 bispecific molecule
DIQMTQSPSAMSASVGDRVTITCRASKSISKYLAWFQQKPGKVPKLRIHSGSTLQSGVPSRFSGSGSGTEFTLTISSLQPEDFATYYCQQHIEYPWTFGQGTKVEIKRGGGGSGGGGSGGGGSQVQLVQSGAEVKKPGASVKVSCKASGYTFTDYYMHWVRQAPGQGLEWMGYFNPYNDYTRYAQKFQGRVTMTRDTSISTAYMELSSLRSDDTAVYYCARSDGYYDAMDYWGQGTTVTVSSSEPKSSDKTHTCPPCPAPEAAGAPSVFLFPPKPKDTLMISRTPEVTCVVVDVSHEDPEVKFNWYVDGVEVHNAKTKPREEQYNSTYRVVSVLTVLHQDWLNGKAYACAVSNKALPAPIEKTISKAKGQPREPQVYTLPPSRDELTKNQVSLTCLVKGFYPSDIAVEWESNGQPENNYKTTPPVLDSDGSFFLYSKLTVDKSRWQQGNVFSCSVMHEALHNHYTQKSLSLSPGQRHNNSSLNTGTQMAGHSPNSQVQLVQSGPEVKKPGSSVKVSCKASGYTFSRSTMHWVRQAPGQGLEWIGYINPSSAYTNYNQKFKDRVTITADKSTSTAYMELSSLRSEDTAVYYCARPQVHYDYNGFPYWGQGTLVTVSSGGGGSGGGGSGGGGSGGGGSDIQMTQSPSTLSASVGDRVTMTCSASSSVSYMNWYQQKPGKAPKRWIYDSSKLASGVPSRFSGSGSGTEFTLTISSLQPDDFATYYCQQWSRNPPTFGGGTKVEIKRSSS

SEQ ID NO: 69 - DNA, 2313 bp, Artificial Sequence
  CAS105 Anti-CD37 X anti-CD3 bispecific molecule
atggaagcaccagcgcagcttctcttcctcctgctactctggctcccagataccaccggtgaggtgcagctggtgcagtctggagcagaggtgaaaaagcccggagagtctctgaagatttcctgtaagggctccggttactcattcactggctacaatatgaactgggtgcgccagatgcccgggaaaggcctggagtggatgggcaatattgatccttattatggtggtactacctacaaccggaagttcaagggccaggtcactatctccgccgacaagtccatcagcaccgcctacctgcaatggagcagcctgaaggcctcggacaccgccatgtattactgtgcacgctcagtcggccctttcgactcctggggccagggcaccctggtcactgtctcctctgggggtggaggctctggtggcggtggctctggcggaggtggatccggtggcggcggatctggcgggggtggctctgaaattgtgttgacacagtctccagccaccctgtctttgtctccaggcgaaagagccaccctctcctgccgagcaagtgaaaatgtttacagctacttagcctggtaccaacagaaacctggccaggctcctaggctcctcatctattttgcaaaaaccttagcagaaggtattccagccaggttcagtggcagtggctccgggacagacttcactctcaccatcagcagcctagagcctgaagattttgcagtttattactgtcaacatcattccgataatccgtggacattcggccaagggaccaaggtggaaatcaaatcctcgagtgagcccaaatcttctgacaaaactcacacatgcccaccgtgcccagcacctgaagccgcgggtgcaccgtcagtcttcctcttccccccaaaacccaaggacaccctcatgatctcccggacccctgaggtcacatgcgtggtggtggacgtgagccacgaagaccctgaggtcaagttcaactggtacgtggacggcgtggaggtgcataatgccaagacaaagccgcgggaggagcagtacaacagcacgtaccgtgtggtcagcgtcctcaccgtcctgcaccaggactggctgaatggcaaggcatacgcgtgcgcggtctccaacaaagccctcccagcccccatcgagaaaaccatctccaaagccaaagggcagccccgagaaccacaggtgtacaccctgcccccatcccgggatgagctgaccaagaaccaggtcagcctgacctgcctggtcaaaggcttctatccaagcgacatcgccgtggagtgggagagcaatgggcagccggagaacaactacaagaccacgcctcccgtgctggactccgacggctccttcttcctctacagcaagctcaccgtggacaagagcaggtggcagcaggggaacgtcttctcatgctccgtgatgcatgaggctctgcacaaccactacacgcagaagagcctctccctgtctccgggtcagaggcacaacaattcttccctgaatacaggaactcagatggcaggtcattctccgaattctcaggtccagctggtggagtctgggggcggagtggtgcagcctgggcggtcactgaggctgtcctgcaaggcttctggctacacctttactagatctacgatgcactgggtaaggcaggcccctggacaaggtctggaatggattggatacattaatcctagcagtgcttatactaattacaatcagaaattcaaggacaggttcacaatcagcgcagacaaatccaagagcacagccttcctgcagatggacagcctgaggcccgaggacaccggcgtctatttctgtgcacggccccaagtccactatgattacaacgggtttccttactggggccaagggactcccgtcactgtctctagcggtggcggagggtctgggggtggcggatccggaggtggtggctctgcacaagacatccagatgacccagtctccaagcagcctgtctgcaagcgtgggggacagggtcaccatgacctgcagtgccagctcaagtgtaagttacatgaactggtaccagcagaagccgggcaaggcccccaaaagatggatttatgactcatccaaactggcttctggagtccctgctcgcttcagtggcagtgggtctgggaccgactataccctcacaatcagcagcctgcagcccgaagatttcgccacttattactgccagcagtggagtcgtaacccacccacgttcggaggggggaccaagctacaaattacatcctccagctaa

SEQ ID NO: 70 - protein, 750 aa, Artificial Sequence
  CAS105 Anti-CD37 X anti-CD3 bispecific molecule
EVQLVQSGAEVKKPGESLKISCKGSGYSFTGYNMNWVRQMPGKGLEWMGNIDPYYGGTTYNRKFKGQVTISADKSISTAYLQWSSLKASDTAMYYCARSVGPFDSWGQGTLVTVSSGGGGSGGGGSGGGGSGGGGSGGGGSEIVLTQSPATLSLSPGERATLSCRASENVYSYLAWYQQKPGQAPRLLIYFAKTLAEGIPARFSGSGSGTDFTLTISSLEPEDFAVYYCQHHSDNPWTFGQGTKVEIKSSSEPKSSDKTHTCPPCPAPEAAGAPSVFLFPPKPKDTLMISRTPEVTCVVVDVSHEDPEVKFNWYVDGVEVHNAKTKPREEQYNSTYRVVSVLTVLHQDWLNGKAYACAVSNKALPAPIEKTISKAKGQPREPQVYTLPPSRDELTKNQVSLTCLVKGFYPSDIAVEWESNGQPENNYKTTPPVLDSDGSFFLYSKLTVDKSRWQQGNVFSCSVMHEALHNHYTQKSLSLSPGQRHNNSSLNTGTQMAGHSPNSQVQLVESGGGVVQPGRSLRLSCKASGYTFTRSTMHWVRQAPGQGLEWIGYINPSSAYTNYNQKFKDRFTISADKSKSTAFLQMDSLRPEDTGVYFCARPQVHYDYNGFPYWGQGTPVTVSSGGGGSGGGGSGGGGSAQDIQMTQSPSSLSASVGDRVTMTCSASSSVSYMNWYQQKPGKAPKRWIYDSSKLASGVPARFSGSGSGTDYTLTISSLQPEDFATYYCQQWSRNPPTFGGGTKLQITSSS

SEQ ID NO: 71 - DNA, 2325 bp, Artificial Sequence
  Anti-CD37 X TSC445 anti-CD3 bispecific molecule
atggaagcaccagcgcagcttctcttcctcctgctactctggctcccagataccaccggtgaggtgcagctggtgcagtctggagcagaggtgaaaaagcccggagagtctctgaagatttcctgtaagggctccggttactcattcactggctacaatatgaactgggtgcgccagatgcccgggaaaggcctggagtggatgggcaatattgatccttattatggtggtactacctacaaccggaagttcaagggccaggtcactatctccgccgacaagtccatcagcaccgcctacctgcaatggagcagcctgaaggcctcggacaccgccatgtattactgtgcacgctcagtcggccctttcgactcctggggccagggcaccctggtcactgtctcctctgggggtggaggctctggtggcggtggctctggcggaggtggatccggtggcggcggatctggcgggggtggctctgaaattgtgttgacacagtctccagccaccctgtctttgtctccaggcgaaagagccaccctctcctgccgagcaagtgaaaatgtttacagctacttagcctggtaccaacagaaacctggccaggctcctaggctcctcatctattttgcaaaaaccttagcagaaggtattccagccaggttcagtggcagtggctccgggacagacttcactctcaccatcagcagcctagagcctgaagattttgcagtttattactgtcaacatcattccgataatccgtggacattcggccaagggaccaaggtggaaatcaaatcctcgagtgagcccaaatcttctgacaaaactcacacatgcccaccgtgcccagcacctgaagccgcgggtgcaccgtcagtcttcctcttccccccaaaacccaaggacaccctcatgatctcccggacccctgaggtcacatgcgtggtggtggacgtgagccacgaagaccctgaggtcaagttcaactggtacgtggacggcgtggaggtgcataatgccaagacaaagccgcgggaggagcagtacaacagcacgtaccgtgtggtcagcgtcctcaccgtcctgcaccaggactggctgaatggcaaggcatacgcgtgcgcggtctccaacaaagccctcccagcccccatcgagaaaaccatctccaaagccaaagggcagccccgagaaccacaggtgtacaccctgcccccatcccgggatgagctgaccaagaaccaggtcagcctgacctgcctggtcaaaggcttctatccaagcgacatcgccgtggagtgggagagcaatgggcagccggagaacaactacaagaccacgcctcccgtgctggactccgacggctccttcttcctctacagcaagctcaccgtggacaagagcaggtggcagcaggggaacgtcttctcatgctccgtgatgcatgaggctctgcacaaccactacacgcagaagagcctctccctgtctccgggtcagaggcacaacaattcttccctgaatacaggaactcagatggcaggtcattctccgaattctcaggtccagctggtgcaatctgggcctgaggtgaagaagcctgggtcctcggtgaaggtctcctgcaaggcttctggatataccttcagcagatctacgatgcactgggtgcgacaggcccctggacaagggcttgagtggataggatacattaatcctagcagtgcttatactaattacaatcagaaattcaaggacagagtcacgattaccgcggacaaatccacgagcacagcctacatggagctgagcagcctgagatctgaggacacggccgtgtattactgtgcgagaccccaagtccactatgattacaacgggtttccttactggggccaaggaaccctggtcaccgtctcctcaggtggaggcggttcaggcggaggtggatccggcggtggcggatcgggtggcggcggatctgacatccagatgacccagtctccttccaccctgtctgcatctgtaggagacagagtcaccatgacttgcagtgccagctcaagtgtaagttacatgaactggtatcagcagaaaccagggaaagcccctaagagatggatttatgactcatccaaactggcttctggggtcccatcaaggttcagcggcagtggatctgggacagagttcactctcaccatcagcagcctgcagcctgatgattttgcaacttattactgccaacagtggagtcgtaacccacccactttcggcggagggaccaaggtggagatcaaacggtcctccagctaa

SEQ ID NO: 72 - protein, 754 aa, Artificial Sequence
  Anti-CD37 X TSC445 anti-CD3 bispecific molecule
EVQLVQSGAEVKKPGESLKISCKGSGYSFTGYNMNWVRQMPGKGLEWMGNIDPYYGGTTYNRKFKGQVTISADKSISTAYLQWSSLKASDTAMYYCARSVGPFDSWGQGTLVTVSSGGGGSGGGGSGGGGSGGGGSGGGGSEIVLTQSPATLSLSPGERATLSCRASENVYSYLAWYQQKPGQAPRLLIYFAKTLAEGIPARFSGSGSGTDFTLTISSLEPEDFAVYYCQHHSDNPWTFGQGTKVEIKSSSEPKSSDKTHTCPPCPAPEAAGAPSVFLFPPKPKDTLMISRTPEVTCVVVDVSHEDPEVKFNWYVDGVEVHNAKTKPREEQYNSTYRVVSVLTVLHQDWLNGKAYACAVSNKALPAPIEKTISKAKGQPREPQVYTLPPSRDELTKNQVSLTCLVKGFYPSDIAVEWESNGQPENNYKTTPPVLDSDGSFFLYSKLTVDKSRWQQGNVFSCSVMHEALHNHYTQKSLSLSPGQRHNNSSLNTGTQMAGHSPNSQVQLVQSGPEVKKPGSSVKVSCKASGYTFSRSTMHWVRQAPGQGLEWIGYINPSSAYTNYNQKFKDRVTITADKSTSTAYMELSSLRSEDTAVYYCARPQVHYDYNGFPYWGQGTLVTVSSGGGGSGGGGSGGGGSGGGGSDIQMTQSPSTLSASVGDRVTMTCSASSSVSYMNWYQQKPGKAPKRWIYDSSKLASGVPSRFSGSGSGTEFTLTISSLQPDDFATYYCQQWSRNPPTFGGGTKVEIKRSSS

SEQ ID NO: 73 - DNA, 2325 bp, Artificial Sequence
  Anti-CD37 X TSC452 anti-CD3 bispecific molecule
atggaagcaccagcgcagcttctcttcctcctgctactctggctcccagataccaccggtgaggtgcagctggtgcagtctggagcagaggtgaaaaagcccggagagtctctgaagatttcctgtaagggctccggttactcattcactggctacaatatgaactgggtgcgccagatgcccgggaaaggcctggagtggatgggcaatattgatccttattatggtggtactacctacaaccggaagttcaagggccaggtcactatctccgccgacaagtccatcagcaccgcctacctgcaatggagcagcctgaaggcctcggacaccgccatgtattactgtgcacgctcagtcggccctttcgactcctggggccagggcaccctggtcactgtctcctctgggggtggaggctctggtggcggtggctctggcggaggtggatccggtggcggcggatctggcgggggtggctctgaaattgtgttgacacagtctccagccaccctgtctttgtctccaggcgaaagagccaccctctcctgccgagcaagtgaaaatgtttacagctacttagcctggtaccaacagaaacctggccaggctcctaggctcctcatctattttgcaaaaaccttagcagaaggtattccagccaggttcagtggcagtggctccgggacagacttcactctcaccatcagcagcctagagcctgaagattttgcagtttattactgtcaacatcattccgataatccgtggacattcggccaagggaccaaggtggaaatcaaatcctcgagtgagcccaaatcttctgacaaaactcacacatgcccaccgtgcccagcacctgaagccgcgggtgcaccgtcagtcttcctcttccccccaaaacccaaggacaccctcatgatctcccggacccctgaggtcacatgcgtggtggtggacgtgagccacgaagaccctgaggtcaagttcaactggtacgtggacggcgtggaggtgcataatgccaagacaaagccgcgggaggagcagtacaacagcacgtaccgtgtggtcagcgtcctcaccgtcctgcaccaggactggctgaatggcaaggcatacgcgtgcgcggtctccaacaaagccctcccagcccccatcgagaaaaccatctccaaagccaaagggcagccccgagaaccacaggtgtacaccctgcccccatcccgggatgagctgaccaagaaccaggtcagcctgacctgcctggtcaaaggcttctatccaagcgacatcgccgtggagtgggagagcaatgggcagccggagaacaactacaagaccacgcctcccgtgctggactccgacggctccttcttcctctacagcaagctcaccgtggacaagagcaggtggcagcaggggaacgtcttctcatgctccgtgatgcatgaggctctgcacaaccactacacgcagaagagcctctccctgtctccgggtcagaggcacaacaattcttccctgaatacaggaactcagatggcaggtcattctccgaattctcaggtccagctggtggagtctgggggcggagtggtgcagcctgggcggtcactgaggctgtcctgcaaggcttctggctacacctttactagatctacgatgcactgggtaaggcaggcccctggacaaggtctggaatggattggatacattaatcctagcagtgcttatactaattacaatcagaaattcaaggacaggttcacaatcagcgcagacaaatccaagagcacagccttcctgcagatggacagcctgaggcccgaggacaccggcgtctatttctgtgcacggccccaagtccactatgattacaacgggtttccttactggggccaagggactcccgtcactgtctctagcggtggcggagggtctgggggtggcggatccggcggtggcggatcgggtggcggcggatctgacatccagatgacccagtctccttccaccctgtctgcatctgtaggagacagagtcaccatgacttgcagtgccagctcaagtgtaagttacatgaactggtatcagcagaaaccagggaaagcccctaagagatggatttatgactcatccaaactggcttctggggtcccatcaaggttcagcggcagtggatctgggacagagttcactctcaccatcagcagcctgcagcctgatgattttgcaacttattactgccaacagtggagtcgtaacccacccactttcggcggagggaccaaggtggagatcaaacggtcctccagctaa

SEQ ID NO: 74 - protein, 754 aa, Artificial Sequence
  Anti-CD37 X TSC452 anti-CD3 bispecific molecule
EVQLVQSGAEVKKPGESLKISCKGSGYSFTGYNMNWVRQMPGKGLEWMGNIDPYYGGTTYNRKFKGQVTISADKSISTAYLQWSSLKASDTAMYYCARSVGPFDSWGQGTLVTVSSGGGGSGGGGSGGGGSGGGGSGGGGSEIVLTQSPATLSLSPGERATLSCRASENVYSYLAWYQQKPGQAPRLLIYFAKTLAEGIPARFSGSGSGTDFTLTISSLEPEDFAVYYCQHHSDNPWTFGQGTKVEIKSSSEPKSSDKTHTCPPCPAPEAAGAPSVFLFPPKPKDTLMISRTPEVTCVVVDVSHEDPEVKFNWYVDGVEVHNAKTKPREEQYNSTYRVVSVLTVLHQDWLNGKAYACAVSNKALPAPIEKTISKAKGQPREPQVYTLPPSRDELTKNQVSLTCLVKGFYPSDIAVEWESNGQPENNYKTTPPVLDSDGSFFLYSKLTVDKSRWQQGNVFSCSVMHEALHNHYTQKSLSLSPGQRHNNSSLNTGTQMAGHSPNSQVQLVESGGGVVQPGRSLRLSCKASGYTFTRSTMHWVRQAPGQGLEWIGYINPSSAYTNYNQKFKDRFTISADKSKSTAFLQMDSLRPEDTGVYFCARPQVHYDYNGFPYWGQGTPVTVSSGGGGSGGGGSGGGGSGGGGSDIQMTQSPSTLSASVGDRVTMTCSASSSVSYMNWYQQKPGKAPKRWIYDSSKLASGVPSRFSGSGSGTEFTLTISSLQPDDFATYYCQQWSRNPPTFGGGTKVEIKRSSS

SEQ ID NO: 75 - DNA, 2322 bp, Artificial Sequence
  Anti-CD37 X TSC453 anti-CD3 bispecific molecule
atggaagcaccagcgcagcttctcttcctcctgctactctggctcccagataccaccggtgaggtgcagctggtgcagtctggagcagaggtgaaaaagcccggagagtctctgaagatttcctgtaagggctccggttactcattcactggctacaatatgaactgggtgcgccagatgcccgggaaaggcctggagtggatgggcaatattgatccttattatggtggtactacctacaaccggaagttcaagggccaggtcactatctccgccgacaagtccatcagcaccgcctacctgcaatggagcagcctgaaggcctcggacaccgccatgtattactgtgcacgctcagtcggccctttcgactcctggggccagggcaccctggtcactgtctcctctgggggtggaggctctggtggcggtggctctggcggaggtggatccggtggcggcggatctggcgggggtggctctgaaattgtgttgacacagtctccagccaccctgtctttgtctccaggcgaaagagccaccctctcctgccgagcaagtgaaaatgtttacagctacttagcctggtaccaacagaaacctggccaggctcctaggctcctcatctattttgcaaaaaccttagcagaaggtattccagccaggttcagtggcagtggctccgggacagacttcactctcaccatcagcagcctagagcctgaagattttgcagtttattactgtcaacatcattccgataatccgtggacattcggccaagggaccaaggtggaaatcaaatcctcgagtgagcccaaatcttctgacaaaactcacacatgcccaccgtgcccagcacctgaagccgcgggtgcaccgtcagtcttcctcttccccccaaaacccaaggacaccctcatgatctcccggacccctgaggtcacatgcgtggtggtggacgtgagccacgaagaccctgaggtcaagttcaactggtacgtggacggcgtggaggtgcataatgccaagacaaagccgcgggaggagcagtacaacagcacgtaccgtgtggtcagcgtcctcaccgtcctgcaccaggactggctgaatggcaaggcatacgcgtgcgcggtctccaacaaagccctcccagcccccatcgagaaaaccatctccaaagccaaagggcagccccgagaaccacaggtgtacaccctgcccccatcccgggatgagctgaccaagaaccaggtcagcctgacctgcctggtcaaaggcttctatccaagcgacatcgccgtggagtgggagagcaatgggcagccggagaacaactacaagaccacgcctcccgtgctggactccgacggctccttcttcctctacagcaagctcaccgtggacaagagcaggtggcagcaggggaacgtcttctcatgctccgtgatgcatgaggctctgcacaaccactacacgcagaagagcctctccctgtctccgggtcagaggcacaacaattcttccctgaatacaggaactcagatggcaggtcattctccgaattctcaggtccagctggtgcaatctgggcctgaggtgaagaagcctgggtcctcggtgaaggtctcctgcaaggcttctggatataccttcagcagatctacgatgcactgggtgcgacaggcccctggacaagggcttgagtggataggatacattaatcctagcagtgcttatactaattacaatcagaaattcaaggacagagtcacgattaccgcggacaaatccacgagcacagcctacatggagctgagcagcctgagatctgaggacacggccgtgtattactgtgcgagaccccaagtccactatgattacaacgggtttccttactggggccaaggaaccctggtcaccgtctcctcaggtggaggcggttcaggcggaggtggatccggaggtggtggctctggtggcggcggatctgacatccagatgacccagtctccaagcagcctgtctgcaagcgtgggggacagggtcaccatgacctgcagtgccagctcaagtgtaagttacatgaactggtaccagcagaagccgggcaaggcccccaaaagatggatttatgactcatccaaactggcttctggagtccctgctcgcttcagtggcagtgggtctgggaccgactataccctcacaatcagcagcctgcagcccgaagatttcgccacttattactgccagcagtggagtcgtaacccacccacgttcggaggggggaccaagctacaaattacatcctccagctaa

SEQ ID NO: 76 - protein, 753 aa, Artificial Sequence
  Anti-CD37 X TSC453 anti-CD3 bispecific molecule
EVQLVQSGAEVKKPGESLKISCKGSGYSFTGYNMNWVRQMPGKGLEWMGNIDPYYGGTTYNRKFKGQVTISADKSISTAYLQWSSLKASDTAMYYCARSVGPFDSWGQGTLVTVSSGGGGSGGGGSGGGGSGGGGSGGGGSEIVLTQSPATLSLSPGERATLSCRASENVYSYLAWYQQKPGQAPRLLIYFAKTLAEGIPARFSGSGSGTDFTLTISSLEPEDFAVYYCQHHSDNPWTFGQGTKVEIKSSSEPKSSDKTHTCPPCPAPEAAGAPSVFLFPPKPKDTLMISRTPEVTCVVVDVSHEDPEVKFNWYVDGVEVHNAKTKPREEQYNSTYRVVSVLTVLHQDWLNGKAYACAVSNKALPAPIEKTISKAKGQPREPQVYTLPPSRDELTKNQVSLTCLVKGFYPSDIAVEWESNGQPENNYKTTPPVLDSDGSFFLYSKLTVDKSRWQQGNVFSCSVMHEALHNHYTQKSLSLSPGQRHNNSSLNTGTQMAGHSPNSQVQLVQSGPEVKKPGSSVKVSCKASGYTFSRSTMHWVRQAPGQGLEWIGYINPSSAYTNYNQKFKDRVTITADKSTSTAYMELSSLRSEDTAVYYCARPQVHYDYNGFPYWGQGTLVTVSSGGGGSGGGGSGGGGSGGGGSDIQMTQSPSSLSASVGDRVTMTCSASSSVSYMNWYQQKPGKAPKRWIYDSSKLASGVPARFSGSGSGTDYTLTISSLQPEDFATYYCQQWSRNPPTFGGGTKLQITSSS

SEQ ID NO: 77 - DNA, 2325 bp, Artificial Sequence
  Anti-CD37 X TSC454 anti-CD3 bispecific molecule
atggaagcaccagcgcagcttctcttcctcctgctactctggctcccagataccaccggtgaggtgcagctggtgcagtctggagcagaggtgaaaaagcccggagagtctctgaagatttcctgtaagggctccggttactcattcactggctacaatatgaactgggtgcgccagatgcccgggaaaggcctggagtggatgggcaatattgatccttattatggtggtactacctacaaccggaagttcaagggccaggtcactatctccgccgacaagtccatcagcaccgcctacctgcaatggagcagcctgaaggcctcggacaccgccatgtattactgtgcacgctcagtcggccctttcgactcctggggccagggcaccctggtcactgtctcctctgggggtggaggctctggtggcggtggctctggcggaggtggatccggtggcggcggatctggcgggggtggctctgaaattgtgttgacacagtctccagccaccctgtctttgtctccaggcgaaagagccaccctctcctgccgagcaagtgaaaatgtttacagctacttagcctggtaccaacagaaacctggccaggctcctaggctcctcatctattttgcaaaaaccttagcagaaggtattccagccaggttcagtggcagtggctccgggacagacttcactctcaccatcagcagcctagagcctgaagattttgcagtttattactgtcaacatcattccgataatccgtggacattcggccaagggaccaaggtggaaatcaaatcctcgagtgagcccaaatcttctgacaaaactcacacatgcccaccgtgcccagcacctgaagccgcgggtgcaccgtcagtcttcctcttccccccaaaacccaaggacaccctcatgatctcccggacccctgaggtcacatgcgtggtggtggacgtgagccacgaagaccctgaggtcaagttcaactggtacgtggacggcgtggaggtgcataatgccaagacaaagccgcgggaggagcagtacaacagcacgtaccgtgtggtcagcgtcctcaccgtcctgcaccaggactggctgaatggcaaggcatacgcgtgcgcggtctccaacaaagccctcccagcccccatcgagaaaaccatctccaaagccaaagggcagccccgagaaccacaggtgtacaccctgcccccatcccgggatgagctgaccaagaaccaggtcagcctgacctgcctggtcaaaggcttctatccaagcgacatcgccgtggagtgggagagcaatgggcagccggagaacaactacaagaccacgcctcccgtgctggactccgacggctccttcttcctctacagcaagctcaccgtggacaagagcaggtggcagcaggggaacgtcttctcatgctccgtgatgcatgaggctctgcacaaccactacacgcagaagagcctctccctgtctccgggtcagaggcacaacaattcttccctgaatacaggaactcagatggcaggtcattctccgaattctcaggtccagctggtgcaatctgggcctgaggtgaagaagcctgggtcctcggtgaaggtctcctgcaaggcttctggatataccttcagcagatctacgatgcactgggtgcgacaggcccctggacaagggcttgagtggataggatacattaatcctagcagtgcttatactaattacaatcagaaattcaaggacagagtcacgattaccgcggacaaatccacgagcacagcctacatggagctgagcagcctgagatctgaggacacggccgtgtattactgtgcgagaccccaagtccactatgattacaacgggtttccttactggggccaaggaaccctggtcaccgtctcctcaggtggaggcggttcaggcggaggtggatccggcggtggcggatcgggtggcggcggatctgacatccagatgacccagtctccttccaccctgtctgcatctgtaggagacagagtcaccatgacttgcagtgccagctcaagtgtaagttacatgaactggtatcagcagaaaccagggaaagcccctaagagatggatttatgactcatccaaactggcttctggggtcccatcaaggttcagcggcagtggatctgggacagatttcactctcaccatcagcagcctgcagcctgatgattttgcaacttattactgccaacagtggagtcgtaacccacccactttcggcggagggaccaaggtggagatcaaacggtcctccagctaa

SEQ ID NO: 78 - protein, 754 aa, Artificial Sequence
  Anti-CD37 X TSC454 anti-CD3 bispecific molecule
EVQLVQSGAEVKKPGESLKISCKGSGYSFTGYNMNWVRQMPGKGLEWMGNIDPYYGGTTYNRKFKGQVTISADKSISTAYLQWSSLKASDTAMYYCARSVGPFDSWGQGTLVTVSSGGGGSGGGGSGGGGSGGGGSGGGGSEIVLTQSPATLSLSPGERATLSCRASENVYSYLAWYQQKPGQAPRLLIYFAKTLAEGIPARFSGSGSGTDFTLTISSLEPEDFAVYYCQHHSDNPWTFGQGTKVEIKSSSEPKSSDKTHTCPPCPAPEAAGAPSVFLFPPKPKDTLMISRTPEVTCVVVDVSHEDPEVKFNWYVDGVEVHNAKTKPREEQYNSTYRVVSVLTVLHQDWLNGKAYACAVSNKALPAPIEKTISKAKGQPREPQVYTLPPSRDELTKNQVSLTCLVKGFYPSDIAVEWESNGQPENNYKTTPPVLDSDGSFFLYSKLTVDKSRWQQGNVFSCSVMHEALHNHYTQKSLSLSPGQRHNNSSLNTGTQMAGHSPNSQVQLVQSGPEVKKPGSSVKVSCKASGYTFSRSTMHWVRQAPGQGLEWIGYINPSSAYTNYNQKFKDRVTITADKSTSTAYMELSSLRSEDTAVYYCARPQVHYDYNGFPYWGQGTLVTVSSGGGGSGGGGSGGGGSGGGGSDIQMTQSPSTLSASVGDRVTMTCSASSSVSYMNWYQQKPGKAPKRWIYDSSKLASGVPSRFSGSGSGTDFTLTISSLQPDDFATYYCQQWSRNPPTFGGGTKVEIKRSSS

SEQ ID NO: 79 - DNA, 2325 bp, Artificial Sequence
  Anti-CD37 X TSC455 anti-CD3 bispecific molecule
atggaagcaccagcgcagcttctcttcctcctgctactctggctcccagataccaccggtgaggtgcagctggtgcagtctggagcagaggtgaaaaagcccggagagtctctgaagatttcctgtaagggctccggttactcattcactggctacaatatgaactgggtgcgccagatgcccgggaaaggcctggagtggatgggcaatattgatccttattatggtggtactacctacaaccggaagttcaagggccaggtcactatctccgccgacaagtccatcagcaccgcctacctgcaatggagcagcctgaaggcctcggacaccgccatgtattactgtgcacgctcagtcggccctttcgactcctggggccagggcaccctggtcactgtctcctctgggggtggaggctctggtggcggtggctctggcggaggtggatccggtggcggcggatctggcgggggtggctctgaaattgtgttgacacagtctccagccaccctgtctttgtctccaggcgaaagagccaccctctcctgccgagcaagtgaaaatgtttacagctacttagcctggtaccaacagaaacctggccaggctcctaggctcctcatctattttgcaaaaaccttagcagaaggtattccagccaggttcagtggcagtggctccgggacagacttcactctcaccatcagcagcctagagcctgaagattttgcagtttattactgtcaacatcattccgataatccgtggacattcggccaagggaccaaggtggaaatcaaatcctcgagtgagcccaaatcttctgacaaaactcacacatgcccaccgtgcccagcacctgaagccgcgggtgcaccgtcagtcttcctcttccccccaaaacccaaggacaccctcatgatctcccggacccctgaggtcacatgcgtggtggtggacgtgagccacgaagaccctgaggtcaagttcaactggtacgtggacggcgtggaggtgcataatgccaagacaaagccgcgggaggagcagtacaacagcacgtaccgtgtggtcagcgtcctcaccgtcctgcaccaggactggctgaatggcaaggcatacgcgtgcgcggtctccaacaaagccctcccagcccccatcgagaaaaccatctccaaagccaaagggcagccccgagaaccacaggtgtacaccctgcccccatcccgggatgagctgaccaagaaccaggtcagcctgacctgcctggtcaaaggcttctatccaagcgacatcgccgtggagtgggagagcaatgggcagccggagaacaactacaagaccacgcctcccgtgctggactccgacggctccttcttcctctacagcaagctcaccgtggacaagagcaggtggcagcaggggaacgtcttctcatgctccgtgatgcatgaggctctgcacaaccactacacgcagaagagcctctccctgtctccgggtcagaggcacaacaattcttccctgaatacaggaactcagatggcaggtcattctccgaattctcaggtccagctggtgcaatctgggcctgaggtgaagaagcctgggtcctcggtgaaggtctcctgcaaggcttctggatataccttcagcagatctacgatgcactgggtgcgacaggcccctggacaagggcttgagtggataggatacattaatcctagcagtgcttatactaattacaatcagaaattcaaggacagagtcacgattaccgcggacaaatccacgagcacagcctacatggagctgagcagcctgagatctgaggacacggccgtgtattactgtgcgagaccccaagtccactatgattacaacgggtttccttactggggccaaggaaccctggtcaccgtctcctcaggtggaggcggttcaggcggaggtggatccggcggtggcggatcgggtggcggcggatctgacatccagatgacccagtctccttccaccctgtctgcatctgtaggagacagagtcaccatgacttgcagtgccagctcaagtgtaagttacatgaactggtatcagcagaaaccagggaaagcccctaagagatggatttatgactcatccaaactggcttctggggtcccatcaaggttcagcggcagtggatctgggacagagtatactctcaccatcagcagcctgcagcctgatgattttgcaacttattactgccaacagtggagtcgtaacccacccactttcggcggagggaccaaggtggagatcaaacggtcctccagctaa

SEQ ID NO: 80 - protein, 754 aa, Artificial Sequence
  Anti-CD37 X TSC455 anti-CD3 bispecific molecule
EVQLVQSGAEVKKPGESLKISCKGSGYSFTGYNMNWVRQMPGKGLEWMGNIDPYYGGTTYNRKFKGQVTISADKSISTAYLQWSSLKASDTAMYYCARSVGPFDSWGQGTLVTVSSGGGGSGGGGSGGGGSGGGGSGGGGSEIVLTQSPATLSLSPGERATLSCRASENVYSYLAWYQQKPGQAPRLLIYFAKTLAEGIPARFSGSGSGTDFTLTISSLEPEDFAVYYCQHHSDNPWTFGQGTKVEIKSSSEPKSSDKTHTCPPCPAPEAAGAPSVFLFPPKPKDTLMISRTPEVTCVVVDVSHEDPEVKFNWYVDGVEVHNAKTKPREEQYNSTYRVVSVLTVLHQDWLNGKAYACAVSNKALPAPIEKTISKAKGQPREPQVYTLPPSRDELTKNQVSLTCLVKGFYPSDIAVEWESNGQPENNYKTTPPVLDSDGSFFLYSKLTVDKSRWQQGNVFSCSVMHEALHNHYTQKSLSLSPGQRHNNSSLNTGTQMAGHSPNSQVQLVQSGPEVKKPGSSVKVSCKASGYTFSRSTMHWVRQAPGQGLEWIGYINPSSAYTNYNQKFKDRVTITADKSTSTAYMELSSLRSEDTAVYYCARPQVHYDYNGFPYWGQGTLVTVSSGGGGSGGGGSGGGGSGGGGSDIQMTQSPSTLSASVGDRVTMTCSASSSVSYMNWYQQKPGKAPKRWIYDSSKLASGVPSRFSGSGSGTEYTLTISSLQPDDFATYYCQQWSRNPPTFGGGTKVEIKRSSS

SEQ ID NO: 81 - DNA, 2325 bp, Artificial Sequence
  Anti-CD37 X TSC456 anti-CD3 bispecific molecule
atggaagcaccagcgcagcttctcttcctcctgctactctggctcccagataccaccggtgaggtgcagctggtgcagtctggagcagaggtgaaaaagcccggagagtctctgaagatttcctgtaagggctccggttactcattcactggctacaatatgaactgggtgcgccagatgcccgggaaaggcctggagtggatgggcaatattgatccttattatggtggtactacctacaaccggaagttcaagggccaggtcactatctccgccgacaagtccatcagcaccgcctacctgcaatggagcagcctgaaggcctcggacaccgccatgtattactgtgcacgctcagtcggccctttcgactcctggggccagggcaccctggtcactgtctcctctgggggtggaggctctggtggcggtggctctggcggaggtggatccggtggcggcggatctggcgggggtggctctgaaattgtgttgacacagtctccagccaccctgtctttgtctccaggcgaaagagccaccctctcctgccgagcaagtgaaaatgtttacagctacttagcctggtaccaacagaaacctggccaggctcctaggctcctcatctattttgcaaaaaccttagcagaaggtattccagccaggttcagtggcagtggctccgggacagacttcactctcaccatcagcagcctagagcctgaagattttgcagtttattactgtcaacatcattccgataatccgtggacattcggccaagggaccaaggtggaaatcaaatcctcgagtgagcccaaatcttctgacaaaactcacacatgcccaccgtgcccagcacctgaagccgcgggtgcaccgtcagtcttcctcttccccccaaaacccaaggacaccctcatgatctcccggacccctgaggtcacatgcgtggtggtggacgtgagccacgaagaccctgaggtcaagttcaactggtacgtggacggcgtggaggtgcataatgccaagacaaagccgcgggaggagcagtacaacagcacgtaccgtgtggtcagcgtcctcaccgtcctgcaccaggactggctgaatggcaaggcatacgcgtgcgcggtctccaacaaagccctcccagcccccatcgagaaaaccatctccaaagccaaagggcagccccgagaaccacaggtgtacaccctgcccccatcccgggatgagctgaccaagaaccaggtcagcctgacctgcctggtcaaaggcttctatccaagcgacatcgccgtggagtgggagagcaatgggcagccggagaacaactacaagaccacgcctcccgtgctggactccgacggctccttcttcctctacagcaagctcaccgtggacaagagcaggtggcagcaggggaacgtcttctcatgctccgtgatgcatgaggctctgcacaaccactacacgcagaagagcctctccctgtctccgggtcagaggcacaacaattcttccctgaatacaggaactcagatggcaggtcattctccgaattctcaggtccagctggtgcaatctgggcctgaggtgaagaagcctgggtcctcggtgaaggtctcctgcaaggcttctggatataccttcagcagatctacgatgcactgggtgcgacaggcccctggacaagggcttgagtggataggatacattaatcctagcagtgcttatactaattacaatcagaaattcaaggacagagtcacgattaccgcggacaaatccacgagcacagcctacatggagctgagcagcctgagatctgaggacacggccgtgtattactgtgcgagaccccaagtccactatgattacaacgggtttccttactggggccaaggaaccctggtcaccgtctcctcaggtggaggcggttcaggcggaggtggatccggcggtggcggatcgggtggcggcggatctgacatccagatgacccagtctccttccaccctgtctgcatctgtaggagacagagtcaccatgacttgcagtgccagctcaagtgtaagttacatgaactggtatcagcagaaaccagggaaagcccctaagagatggatttatgactcatccaaactggcttctggggtcccatcaaggttcagcggcagtggatctgggacagattatactctcaccatcagcagcctgcagcctgatgattttgcaacttattactgccaacagtggagtcgtaacccacccactttcggcggagggaccaaggtggagatcaaacggtcctccagctaa

SEQ ID NO: 82 - protein, 754 aa, Artificial Sequence
  Anti-CD37 X TSC456 anti-CD3 bispecific molecule
EVQLVQSGAEVKKPGESLKISCKGSGYSFTGYNMNWVRQMPGKGLEWMGNIDPYYGGTTYNRKFKGQVTISADKSISTAYLQWSSLKASDTAMYYCARSVGPFDSWGQGTLVTVSSGGGGSGGGGSGGGGSGGGGSGGGGSEIVLTQSPATLSLSPGERATLSCRASENVYSYLAWYQQKPGQAPRLLIYFAKTLAEGIPARFSGSGSGTDFTLTISSLEPEDFAVYYCQHHSDNPWTFGQGTKVEIKSSSEPKSSDKTHTCPPCPAPEAAGAPSVFLFPPKPKDTLMISRTPEVTCVVVDVSHEDPEVKFNWYVDGVEVHNAKTKPREEQYNSTYRVVSVLTVLHQDWLNGKAYACAVSNKALPAPIEKTISKAKGQPREPQVYTLPPSRDELTKNQVSLTCLVKGFYPSDIAVEWESNGQPENNYKTTPPVLDSDGSFFLYSKLTVDKSRWQQGNVFSCSVMHEALHNHYTQKSLSLSPGQRHNNSSLNTGTQMAGHSPNSQVQLVQSGPEVKKPGSSVKVSCKASGYTFSRSTMHWVRQAPGQGLEWIGYINPSSAYTNYNQKFKDRVTITADKSTSTAYMELSSLRSEDTAVYYCARPQVHYDYNGFPYWGQGTLVTVSSGGGGSGGGGSGGGGSGGGGSDIQMTQSPSTLSASVGDRVTMTCSASSSVSYMNWYQQKPGKAPKRWIYDSSKLASGVPSRFSGSGSGTDYTLTISSLQPDDFATYYCQQWSRNPPTFGGGTKVEIKRSSS

SEQ ID NO: 83 - protein, 251 aa, Artificial Sequence
  TSC455 CD3 scFv CD3-binding domain
QVQLVQSGPEVKKPGSSVKVSCKASGYTFSRSTMHWVRQAPGQGLEWIGYINPSSAYTNYNQKFKDRVTITADKSTSTAYMELSSLRSEDTAVYYCARPQVHYDYNGFPYWGQGTLVTVSSGGGGSGGGGSGGGGSGGGGSDIQMTQSPSTLSASVGDRVTMTCSASSSVSYMNWYQQKPGKAPKRWIYDSSKLASGVPSRFSGSGSGTEYTLTISSLQPDDFATYYCQQWSRNPPTFGGGTKVEIKRSSS

SEQ ID NO: 84 - protein, 251 aa, Artificial Sequence
  TSC456 CD3 scFv CD3-binding domain
QVQLVQSGPEVKKPGSSVKVSCKASGYTFSRSTMHWVRQAPGQGLEWIGYINPSSAYTNYNQKFKDRVTITADKSTSTAYMELSSLRSEDTAVYYCARPQVHYDYNGFPYWGQGTLVTVSSGGGGSGGGGSGGGGSGGGGSDIQMTQSPSTLSASVGDRVTMTCSASSSVSYMNWYQQKPGKAPKRWIYDSSKLASGVPSRFSGSGSGTDYTLTISSLQPDDFATYYCQQWSRNPPTFGGGTKVEIKRSSS

SEQ ID NO: 85 - protein, 247 aa, Artificial Sequence
  DRA222 CD3 scFv CD3-binding domain
QVQLVESGGGVVQPGRSLRLSCKASGYTFTRSTMHWVRQAPGQGLEWIGYINPSSAYTNYNQKFKDRFTISADKSKSTAFLQMDSLRPEDTGVYFCARPQVHYDYNGFPYWGQGTPVTVSSGGGGSGGGGSGGGGSAQDIQMTQSPSSLSASVGDRVTMTCSASSSVSYMNWYQQKPGKAPKRWIYDSSKLASGVPARFSGSGSGTDYTLTISSLQPEDFATYYCQQWSRNPPTFGGGTKLQITSSS

SEQ ID NO: 86 - protein, 121 aa, Artificial Sequence
  TSC455 and TSC456 variable heavy domain CD3-binding domain
QVQLVQSGPEVKKPGSSVKVSCKASGYTFSRSTMHWVRQAPGQGLEWIGYINPSSAYTNYNQKFKDRVTITADKSTSTAYMELSSLRSEDTAVYYCARPQVHYDYNGFPYWGQGTLVTVSS

SEQ ID NO: 87 - protein, 121 aa, Artificial Sequence
  DRA222 variable heavy domain CD3-binding domain
QVQLVESGGGVVQPGRSLRLSCKASGYTFTRSTMHWVRQAPGQGLEWIGYINPSSAYTNYNQKFKDRFTISADKSKSTAFLQMDSLRPEDTGVYFCARPQVHYDYNGFPYWGQGTPVTVSS

SEQ ID NO: 88 - protein, 108 aa, Artificial Sequence
  TSC455 variable light domain CD3-binding domain
DIQMTQSPSTLSASVGDRVTMTCSASSSVSYMNWYQQKPGKAPKRWIYDSSKLASGVPSRFSGSGSGTEYTLTISSLQPDDFATYYCQQWSRNPPTFGGGTKVEIKRS

SEQ ID NO: 89 - protein, 108 aa, Artificial Sequence
  TSC456 variable light domain CD3-binding domain
DIQMTQSPSTLSASVGDRVTMTCSASSSVSYMNWYQQKPGKAPKRWIYDSSKLASGVPSRFSGSGSGTDYTLTISSLQPDDFATYYCQQWSRNPPTFGGGTKVEIKRS

SEQ ID NO: 90 - protein, 107 aa, Artificial Sequence
  DRA222 variable light domain CD3-binding domain
DIQMTQSPSSLSASVGDRVTMTCSASSSVSYMNWYQQKPGKAPKRWIYDSSKLASGVPARFSGSGSGTDYTLTISSLQPEDFATYYCQQWSRNPPTFGGGTKLQITS

SEQ ID NO: 91 - protein, 5 aa, Artificial Sequence
  Cris7 and DRA222 VH CDR1 (Kabat) CD3-binding domain
RSTMH

SEQ ID NO: 92 - protein, 16 aa, Artificial Sequence
  Cris7 and DRA222 VH CDR2 (Kabat) CD3-binding domain
YINPSSAYTNYNQKFK

SEQ ID NO: 93 - protein, 11 aa, Artificial Sequence
  Cris7 and DRA222 VH CDR3 (Kabat) CD3-binding domain
QVHYDYNGFPY

SEQ ID NO: 94 - protein, 10 aa, Artificial Sequence
  Cris7 and DRA222 VL CDR1 (Kabat) CD3-binding domain
SASSSVSYMN

SEQ ID NO: 95 - protein, 7 aa, Artificial Sequence
  Cris7 and DRA222 VL CDR2 (Kabat) CD3-binding domain
DSSKLAS

SEQ ID NO: 96 - protein, 9 aa, Artificial Sequence
  Cris7 and DRA222 VL CDR3 (Kabat) CD3-binding domain
QQWSRNPPT

SEQ ID NO: 97 - DNA, 2304 bp, Artificial Sequence
  ROR133 Anti-ROR1 X anti-CD3 bispecific molecule
atggaagcaccagcgcagcttctcttcctcctgctactctggctcccagataccaccggtgacatccagatgacccagtccccctcctccctgtccgcctccgtgggcgaccgggtgaccatcaactgccaggcctcccagtccatcgactccaacctggcctggttccagcagaagcccggcaagccccccaagctgctgatctaccgggcctccaacctggcctccggcgtgccctcccggttctccggctccggctccggcaccgacttcaccctgaccatctcctccctgcagcccgaggacgtggccacctactactgcctgggcggcgtgggcgccgtgtcctaccggacctccttcggcggcggcaccaaggtggagatcaagggtggaggcggttcaggcggaggtggatccggcggtggcggctccggtggcggcggatctgaggtgcagctggtggagtccggcggcggcctggtgcagcccggccggtccctgcggctgtcctgcaccgcctccggctccgacatcaacgactaccccatctcctgggtgcggcaggcccccggcaagggcctggagtggatcggcttcatcaactccggcggctccacctggtacgcctcctgggtgaagggccggttcaccatctcccgggacgactccaagtccatcgcctacctgcagatgaactccctgaagaccgaggacaccgccgtgtactattgcgcccggggctactccacctactacggcgacttcaacatctggggccagggcaccctggtgaccgtgtcctcgagtgagcccaaatcttctgacaaaactcacacatgcccaccgtgcccagcacctgaagccgcgggtgcaccgtcagtcttcctcttccccccaaaacccaaggacaccctcatgatctcccggacccctgaggtcacatgcgtggtggtggacgtgagccacgaagaccctgaggtcaagttcaactggtacgtggacggcgtggaggtgcataatgccaagacaaagccgcgggaggagcagtacaacagcacgtaccgtgtggtcagcgtcctcaccgtcctgcaccaggactggctgaatggcaaggaatacaagtgcgcggtctccaacaaagccctcccagcccccatcgagaaaaccatctccaaagccaaagggcagccccgagaaccacaggtgtacaccctgcccccatcccgggatgagctgaccaagaaccaggtcagcctgacctgcctggtcaaaggcttctatccaagcgacatcgccgtggagtgggagagcaatgggcagccggagaacaactacaagaccacgcctcccgtgctggactccgacggctccttcttcctctacagcaagctcaccgtggacaagagcaggtggcagcaggggaacgtcttctcatgctccgtgatgcatgaggctctgcacaaccactacacgcagaagagcctctccctgtctccgggttctggtggaggcggttcaggcggaggtggctccggcggtggcggatcgccgggctctcaggtccagctggtggagtctgggggcggagtggtgcagcctgggcggtcactgaggctgtcctgcaaggcttctggctacacctttactagatctacgatgcactgggtaaggcaggcccctggacaaggtctggaatggattggatacattaatcctagcagtgcttatactaattacaatcagaaattcaaggacaggttcacaatcagcgcagacaaatccaagagcacagccttcctgcagatggacagcctgaggcccgaggacaccggcgtctatttctgtgcacggccccaagtccactatgattacaacgggtttccttactggggccaagggactcccgtcactgtctctagcggtggcggagggtctgggggtggcggatccggaggtggtggctctgcacaagacatccagatgacccagtctccaagcagcctgtctgcaagcgtgggggacagggtcaccatgacctgcagtgccagctcaagtgtaagttacatgaactggtaccagcagaagccgggcaaggcccccaaaagatggatttatgactcatccaaactggcttctggagtccctgctcgcttcagtggcagtgggtctgggaccgactataccctcacaatcagcagcctgcagcccgaagatttcgccacttattactgccagcagtggagtcgtaacccacccacgttcggaggggggaccaagctacaaattacatcctccagctaa

SEQ ID NO: 98 - protein, 747 aa, Artificial Sequence
  ROR133 Anti-ROR1 X anti-CD3 bispecific molecule
DIQMTQSPSSLSASVGDRVTINCQASQSIDSNLAWFQQKPGKPPKLLIYRASNLASGVPSRFSGSGSGTDFTLTISSLQPEDVATYYCLGGVGAVSYRTSFGGGTKVEIKGGGGSGGGGSGGGGSGGGGSEVQLVESGGGLVQPGRSLRLSCTASGSDINDYPISWVRQAPGKGLEWIGFINSGGSTWYASWVKGRFTISRDDSKSIAYLQMNSLKTEDTAVYYCARGYSTYYGDFNIWGQGTLVTVSSSEPKSSDKTHTCPPCPAPEAAGAPSVFLFPPKPKDTLMISRTPEVTCVVVDVSHEDPEVKFNWYVDGVEVHNAKTKPREEQYNSTYRVVSVLTVLHQDWLNGKEYKCAVSNKALPAPIEKTISKAKGQPREPQVYTLPPSRDELTKNQVSLTCLVKGFYPSDIAVEWESNGQPENNYKTTPPVLDSDGSFFLYSKLTVDKSRWQQGNVFSCSVMHEALHNHYTQKSLSLSPGSGGGGSGGGGSGGGGSPGSQVQLVESGGGVVQPGRSLRLSCKASGYTFTRSTMHWVRQAPGQGLEWIGYINPSSAYTNYNQKFKDRFTISADKSKSTAFLQMDSLRPEDTGVYFCARPQVHYDYNGFPYWGQGTPVTVSSGGGGSGGGGSGGGGSAQDIQMTQSPSSLSASVGDRVTMTCSASSSVSYMNWYQQKPGKAPKRWIYDSSKLASGVPARFSGSGSGTDYTLTISSLQPEDFATYYCQQWSRNPPTFGGGTKLQITSSS

SEQ ID NO: 99 - DNA, 2316 bp, Artificial Sequence
  ROR193 Anti-ROR1 X anti-CD3 bispecific molecule
atggaagcaccagcgcagcttctcttcctcctgctactctggctcccagataccaccggtgacatccagatgacccagtccccctcctccctgtccgcctccgtgggcgaccgggtgaccatcaactgccaggcctcccagtccatcgactccaacctggcctggttccagcagaagcccggcaagccccccaagctgctgatctaccgggcctccaacctggcctccggcgtgccctcccggttctccggctccggctccggcaccgacttcaccctgaccatctcctccctgcagcccgaggacgtggccacctactactgcctgggcggcgtgggcgccgtgtcctaccggacctccttcggcggcggcaccaaggtggagatcaagggtggaggcggttcaggcggaggtggatccggcggtggcggctccggtggcggcggatctgaggtgcagctggtggagtccggcggcggcctggtgcagcccggccggtccctgcggctgtcctgcaccgcctccggctccgacatcaacgactaccccatctcctgggtgcggcaggcccccggcaagggcctggagtggatcggcttcatcaactccggcggctccacctggtacgcctcctgggtgaagggccggttcaccatctcccgggacgactccaagtccatcgcctacctgcagatgaactccctgaagaccgaggacaccgccgtgtactattgcgcccggggctactccacctactacggcgacttcaacatctggggccagggcaccctggtgaccgtgtcctcgagtgagcccaaatcttctgacaaaactcacacatgcccaccgtgcccagcacctgaagccgcgggtgcaccgtcagtcttcctcttccccccaaaacccaaggacaccctcatgatctcccggacccctgaggtcacatgcgtggtggtggacgtgagccacgaagaccctgaggtcaagttcaactggtacgtggacggcgtggaggtgcataatgccaagacaaagccgcgggaggagcagtacaacagcacgtaccgtgtggtcagcgtcctcaccgtcctgcaccaggactggctgaatggcaaggaatacaagtgcgcggtctccaacaaagccctcccagcccccatcgagaaaaccatctccaaagccaaagggcagccccgagaaccacaggtgtacaccctgcccccatcccgggatgagctgaccaagaaccaggtcagcctgacctgcctggtcaaaggcttctatccaagcgacatcgccgtggagtgggagagcaatgggcagccggagaacaactacaagaccacgcctcccgtgctggactccgacggctccttcttcctctacagcaagctcaccgtggacaagagcaggtggcagcaggggaacgtcttctcatgctccgtgatgcatgaggctctgcacaaccactacacgcagaagagcctctccctgtctccgggttctggtggaggcggttcaggcggaggtggctccggcggtggcggatcgccgggctctcaggtccagctggtgcaatctgggcctgaggtgaagaagcctgggtcctcggtgaaggtctcctgcaaggcttctggatataccttcagcagatctacgatgcactgggtgcgacaggcccctggacaagggcttgagtggataggatacattaatcctagcagtgcttatactaattacaatcagaaattcaaggacagagtcacgattaccgcggacaaatccacgagcacagcctacatggagctgagcagcctgagatctgaggacacggccgtgtattactgtgcgagaccccaagtccactatgattacaacgggtttccttactggggccaaggaaccctggtcaccgtctcctcaggtggaggcggttcaggcggaggtggatccggcggtggcggatcgggtggcggcggatctgacatccagatgacccagtctccttccaccctgtctgcatctgtaggagacagagtcaccatgacttgcagtgccagctcaagtgtaagttacatgaactggtatcagcagaaaccagggaaagcccctaagagatggatttatgactcatccaaactggcttctggggtcccatcaaggttcagcggcagtggatctgggacagagtatactctcaccatcagcagcctgcagcctgatgattttgcaacttattactgccaacagtggagtcgtaacccacccactttcggcggagggaccaaggtggagatcaaacggtcctccagctaa

SEQ ID NO: 100 - protein, 751 aa, Artificial Sequence
  ROR193 Anti-ROR1 X anti-CD3 bispecific molecule
DIQMTQSPSSLSASVGDRVTINCQASQSIDSNLAWFQQKPGKPPKLLIYRASNLASGVPSRFSGSGSGTDFTLTISSLQPEDVATYYCLGGVGAVSYRTSFGGGTKVEIKGGGGSGGGGSGGGGSGGGGSEVQLVESGGGLVQPGRSLRLSCTASGSDINDYPISWVRQAPGKGLEWIGFINSGGSTWYASWVKGRFTISRDDSKSIAYLQMNSLKTEDTAVYYCARGYSTYYGDFNIWGQGTLVTVSSSEPKSSDKTHTCPPCPAPEAAGAPSVFLFPPKPKDTLMISRTPEVTCVVVDVSHEDPEVKFNWYVDGVEVHNAKTKPREEQYNSTYRVVSVLTVLHQDWLNGKEYKCAVSNKALPAPIEKTISKAKGQPREPQVYTLPPSRDELTKNQVSLTCLVKGFYPSDIAVEWESNGQPENNYKTTPPVLDSDGSFFLYSKLTVDKSRWQQGNVFSCSVMHEALHNHYTQKSLSLSPGSGGGGSGGGGSGGGGSPGSQVQLVQSGPEVKKPGSSVKVSCKASGYTFSRSTMHWVRQAPGQGLEWIGYINPSSAYTNYNQKFKDRVTITADKSTSTAYMELSSLRSEDTAVYYCARPQVHYDYNGFPYWGQGTLVTVSSGGGGSGGGGSGGGGSGGGGSDIQMTQSPSTLSASVGDRVTMTCSASSSVSYMNWYQQKPGKAPKRWIYDSSKLASGVPSRFSGSGSGTEYTLTISSLQPDDFATYYCQQWSRNPPTFGGGTKVEIKRSSS

SEQ ID NO: 101 - DNA, 2304 bp, Artificial Sequence
  ROR134 Anti-ROR1 X anti-CD3 bispecific molecule
atggaagcaccagcgcagcttctcttcctcctgctactctggctcccagataccaccggtgacatccagatgacccagtccccctcctccctgtccgcctccgtgggcgaccgggtgaccatcaactgccaggcctcccagtccatcgactccaacctggcctggttccagcagaagcccggcaagccccccaagctgctgatctaccgggcctccaacctggcctccggcgtgccctcccggttctccggctccggctccggcaccgacttcaccctgaccatctcctccctgcagcccgaggacgtggccacctactactgcctgggcggcgtgggcgccgtgtcctaccggacctccttcggcggcggcaccaaggtggagatcaagggtggaggcggttcaggcggaggtggatccggcggtggcggctccggtggcggcggatctgaggtgcagctggtggagtccggcggcggcctggtgcagcccggcggctccctgcggctgtcctgcaccgcctccggctccgacatcaacgactaccccatctcctgggtgcggcaggcccccggcaagggcctggagtggatcggcttcatcaactccggcggctccacctggtacgccgactcggtgaagggccggttcaccatctcccggcactcctccaagaacaccctgtacctgcagatgaactccctgcgggccgaggacaccgccgtgtacttctgcgcccggggctactccacctactacggcgacttcaacatctggggccagggcaccctggtgaccgtgtcctcgagtgagcccaaatcttctgacaaaactcacacatgcccaccgtgcccagcacctgaagccgcgggtgcaccgtcagtcttcctcttccccccaaaacccaaggacaccctcatgatctcccggacccctgaggtcacatgcgtggtggtggacgtgagccacgaagaccctgaggtcaagttcaactggtacgtggacggcgtggaggtgcataatgccaagacaaagccgcgggaggagcagtacaacagcacgtaccgtgtggtcagcgtcctcaccgtcctgcaccaggactggctgaatggcaaggaatacaagtgcgcggtctccaacaaagccctcccagcccccatcgagaaaaccatctccaaagccaaagggcagccccgagaaccacaggtgtacaccctgcccccatcccgggatgagctgaccaagaaccaggtcagcctgacctgcctggtcaaaggcttctatccaagcgacatcgccgtggagtgggagagcaatgggcagccggagaacaactacaagaccacgcctcccgtgctggactccgacggctccttcttcctctacagcaagctcaccgtggacaagagcaggtggcagcaggggaacgtcttctcatgctccgtgatgcatgaggctctgcacaaccactacacgcagaagagcctctccctgtctccgggttctggtggaggcggttcaggcggaggtggctccggcggtggcggatcgccgggctctcaggtccagctggtggagtctgggggcggagtggtgcagcctgggcggtcactgaggctgtcctgcaaggcttctggctacacctttactagatctacgatgcactgggtaaggcaggcccctggacaaggtctggaatggattggatacattaatcctagcagtgcttatactaattacaatcagaaattcaaggacaggttcacaatcagcgcagacaaatccaagagcacagccttcctgcagatggacagcctgaggcccgaggacaccggcgtctatttctgtgcacggccccaagtccactatgattacaacgggtttccttactggggccaagggactcccgtcactgtctctagcggtggcggagggtctgggggtggcggatccggaggtggtggctctgcacaagacatccagatgacccagtctccaagcagcctgtctgcaagcgtgggggacagggtcaccatgacctgcagtgccagctcaagtgtaagttacatgaactggtaccagcagaagccgggcaaggcccccaaaagatggatttatgactcatccaaactggcttctggagtccctgctcgcttcagtggcagtgggtctgggaccgactataccctcacaatcagcagcctgcagcccgaagatttcgccacttattactgccagcagtggagtcgtaacccacccacgttcggaggggggaccaagctacaaattacatcctccagctaa

SEQ ID NO: 102 - protein, 747 aa, Artificial Sequence
  ROR134 Anti-ROR1 X anti-CD3 bispecific molecule
DIQMTQSPSSLSASVGDRVTINCQASQSIDSNLAWFQQKPGKPPKLLIYRASNLASGVPSRFSGSGSGTDFTLTISSLQPEDVATYYCLGGVGAVSYRTSFGGGTKVEIKGGGGSGGGGSGGGGSGGGGSEVQLVESGGGLVQPGGSLRLSCTASGSDINDYPISWVRQAPGKGLEWIGFINSGGSTWYADSVKGRFTISRHSSKNTLYLQMNSLRAEDTAVYFCARGYSTYYGDFNIWGQGTLVTVSSSEPKSSDKTHTCPPCPAPEAAGAPSVFLFPPKPKDTLMISRTPEVTCVVVDVSHEDPEVKFNWYVDGVEVHNAKTKPREEQYNSTYRVVSVLTVLHQDWLNGKEYKCAVSNKALPAPIEKTISKAKGQPREPQVYTLPPSRDELTKNQVSLTCLVKGFYPSDIAVEWESNGQPENNYKTTPPVLDSDGSFFLYSKLTVDKSRWQQGNVFSCSVMHEALHNHYTQKSLSLSPGSGGGGSGGGGSGGGGSPGSQVQLVESGGGVVQPGRSLRLSCKASGYTFTRSTMHWVRQAPGQGLEWIGYINPSSAYTNYNQKFKDRFTISADKSKSTAFLQMDSLRPEDTGVYFCARPQVHYDYNGFPYWGQGTPVTVSSGGGGSGGGGSGGGGSAQDIQMTQSPSSLSASVGDRVTMTCSASSSVSYMNWYQQKPGKAPKRWIYDSSKLASGVPARFSGSGSGTDYTLTISSLQPEDFATYYCQQWSRNPPTFGGGTKLQITSSS

SEQ ID NO: 103 - DNA, 2316 bp, Artificial Sequence
  ROR189 Anti-ROR1 X anti-CD3 bispecific molecule
atggaagcaccagcgcagcttctcttcctcctgctactctggctcccagataccaccggtgacatccagatgacccagtccccctcctccctgtccgcctccgtgggcgaccgggtgaccatcaactgccaggcctcccagtccatcgactccaacctggcctggttccagcagaagcccggcaagccccccaagctgctgatctaccgggcctccaacctggcctccggcgtgccctcccggttctccggctccggctccggcaccgacttcaccctgaccatctcctccctgcagcccgaggacgtggccacctactactgcctgggcggcgtgggcgccgtgtcctaccggacctccttcggcggcggcaccaaggtggagatcaagggtggaggcggttcaggcggaggtggatccggcggtggcggctccggtggcggcggatctgaggtgcagctggtggagtccggcggcggcctggtgcagcccggcggctccctgcggctgtcctgcaccgcctccggctccgacatcaacgactaccccatctcctgggtgcggcaggcccccggcaagggcctggagtggatcggcttcatcaactccggcggctccacctggtacgccgactcggtgaagggccggttcaccatctcccggcactcctccaagaacaccctgtacctgcagatgaactccctgcgggccgaggacaccgccgtgtacttctgcgcccggggctactccacctactacggcgacttcaacatctggggccagggcaccctggtgaccgtgtcctcgagtgagcccaaatcttctgacaaaactcacacatgcccaccgtgcccagcacctgaagccgcgggtgcaccgtcagtcttcctcttccccccaaaacccaaggacaccctcatgatctcccggacccctgaggtcacatgcgtggtggtggacgtgagccacgaagaccctgaggtcaagttcaactggtacgtggacggcgtggaggtgcataatgccaagacaaagccgcgggaggagcagtacaacagcacgtaccgtgtggtcagcgtcctcaccgtcctgcaccaggactggctgaatggcaaggaatacaagtgcgcggtctccaacaaagccctcccagcccccatcgagaaaaccatctccaaagccaaagggcagccccgagaaccacaggtgtacaccctgcccccatcccgggatgagctgaccaagaaccaggtcagcctgacctgcctggtcaaaggcttctatccaagcgacatcgccgtggagtgggagagcaatgggcagccggagaacaactacaagaccacgcctcccgtgctggactccgacggctccttcttcctctacagcaagctcaccgtggacaagagcaggtggcagcaggggaacgtcttctcatgctccgtgatgcatgaggctctgcacaaccactacacgcagaagagcctctccctgtctccgggttctggtggaggcggttcaggcggaggtggctccggcggtggcggatcgccgggctctcaggtccagctggtgcaatctgggcctgaggtgaagaagcctgggtcctcggtgaaggtctcctgcaaggcttctggatataccttcagcagatctacgatgcactgggtgcgacaggcccctggacaagggcttgagtggataggatacattaatcctagcagtgcttatactaattacaatcagaaattcaaggacagagtcacgattaccgcggacaaatccacgagcacagcctacatggagctgagcagcctgagatctgaggacacggccgtgtattactgtgcgagaccccaagtccactatgattacaacgggtttccttactggggccaaggaaccctggtcaccgtctcctcaggtggaggcggttcaggcggaggtggatccggcggtggcggatcgggtggcggcggatctgacatccagatgacccagtctccttccaccctgtctgcatctgtaggagacagagtcaccatgacttgcagtgccagctcaagtgtaagttacatgaactggtatcagcagaaaccagggaaagcccctaagagatggatttatgactcatccaaactggcttctggggtcccatcaaggttcagcggcagtggatctgggacagattatactctcaccatcagcagcctgcagcctgatgattttgcaacttattactgccaacagtggagtcgtaacccacccactttcggcggagggaccaaggtggagatcaaacggtcctccagctaa

SEQ ID NO: 104 - protein, 751 aa, Artificial Sequence
  ROR189 Anti-ROR1 X anti-CD3 bispecific molecule
DIQMTQSPSSLSASVGDRVTINCQASQSIDSNLAWFQQKPGKPPKLLIYRASNLASGVPSRFSGSGSGTDFTLTISSLQPEDVATYYCLGGVGAVSYRTSFGGGTKVEIKGGGGSGGGGSGGGGSGGGGSEVQLVESGGGLVQPGGSLRLSCTASGSDINDYPISWVRQAPGKGLEWIGFINSGGSTWYADSVKGRFTISRHSSKNTLYLQMNSLRAEDTAVYFCARGYSTYYGDFNIWGQGTLVTVSSSEPKSSDKTHTCPPCPAPEAAGAPSVFLFPPKPKDTLMISRTPEVTCVVVDVSHEDPEVKFNWYVDGVEVHNAKTKPREEQYNSTYRVVSVLTVLHQDWLNGKEYKCAVSNKALPAPIEKTISKAKGQPREPQVYTLPPSRDELTKNQVSLTCLVKGFYPSDIAVEWESNGQPENNYKTTPPVLDSDGSFFLYSKLTVDKSRWQQGNVFSCSVMHEALHNHYTQKSLSLSPGSGGGGSGGGGSGGGGSPGSQVQLVQSGPEVKKPGSSVKVSCKASGYTFSRSTMHWVRQAPGQGLEWIGYINPSSAYTNYNQKFKDRVTITADKSTSTAYMELSSLRSEDTAVYYCARPQVHYDYNGFPYWGQGTLVTVSSGGGGSGGGGSGGGGSGGGGSDIQMTQSPSTLSASVGDRVTMTCSASSSVSYMNWYQQKPGKAPKRWIYDSSKLASGVPSRFSGSGSGTDYTLTISSLQPDDFATYYCQQWSRNPPTFGGGTKVEIKRSSS

SEQ ID NO: 105 - DNA, 2304 bp, Artificial Sequence
  ROR154 Anti-ROR1 X anti-CD3 bispecific molecule
atggaagcaccagcgcagcttctcttcctcctgctactctggctcccagataccaccggtgacatccagatgacccagtccccctcctccctgtccgcctccgtgggcgaccgggtgaccatcaactgccaggcctcccagtccatcgactccaacctggcctggttccagcagaagcccggcaagccccccaagctgctgatctaccgggcctccaacctggcctccggcgtgccctcccggttctccggctccggctccggcaccgacttcaccctgaccatctcctccctgcagcccgaggacgtggccacctactactgcctgggcggcgtgggcgccgtgtcctaccggacctccttcggcggcggcaccaaggtggagatcaagggtggaggcggttcaggcggaggtggatccggcggtggcggctccggtggcggcggatctgaggtgcagctggtggagtccggcggcggcctggtgcagcccggccggtccctgcggctgtcctgcaccgcctccggctccgacatcaacgactaccccatcacctgggtgcggcaggcccccggcaagggcctggagtggatcggcttcatcaactccggcggctccacctggtacgcctcctgggtgaagggccggttcaccatctcccgggacgactccaagtccatcgcctacctgcagatgaactccctgaagaccgaggacaccgccgtgtactattgcgcccggggctactccacctactaccgggacttcaacatctggggccagggcaccctggtgaccgtgtcctcgagtgagcccaaatcttctgacaaaactcacacatgcccaccgtgcccagcacctgaagccgcgggtgcaccgtcagtcttcctcttccccccaaaacccaaggacaccctcatgatctcccggacccctgaggtcacatgcgtggtggtggacgtgagccacgaagaccctgaggtcaagttcaactggtacgtggacggcgtggaggtgcataatgccaagacaaagccgcgggaggagcagtacaacagcacgtaccgtgtggtcagcgtcctcaccgtcctgcaccaggactggctgaatggcaaggaatacaagtgcgcggtctccaacaaagccctcccagcccccatcgagaaaaccatctccaaagccaaagggcagccccgagaaccacaggtgtacaccctgcccccatcccgggatgagctgaccaagaaccaggtcagcctgacctgcctggtcaaaggcttctatccaagcgacatcgccgtggagtgggagagcaatgggcagccggagaacaactacaagaccacgcctcccgtgctggactccgacggctccttcttcctctacagcaagctcaccgtggacaagagcaggtggcagcaggggaacgtcttctcatgctccgtgatgcatgaggctctgcacaaccactacacgcagaagagcctctccctgtctccgggttctggtggaggcggttcaggcggaggtggctccggcggtggcggatcgccgggctctcaggtccagctggtggagtctgggggcggagtggtgcagcctgggcggtcactgaggctgtcctgcaaggcttctggctacacctttactagatctacgatgcactgggtaaggcaggcccctggacaaggtctggaatggattggatacattaatcctagcagtgcttatactaattacaatcagaaattcaaggacaggttcacaatcagcgcagacaaatccaagagcacagccttcctgcagatggacagcctgaggcccgaggacaccggcgtctatttctgtgcacggccccaagtccactatgattacaacgggtttccttactggggccaagggactcccgtcactgtctctagcggtggcggagggtctgggggtggcggatccggaggtggtggctctgcacaagacatccagatgacccagtctccaagcagcctgtctgcaagcgtgggggacagggtcaccatgacctgcagtgccagctcaagtgtaagttacatgaactggtaccagcagaagccgggcaaggcccccaaaagatggatttatgactcatccaaactggcttctggagtccctgctcgcttcagtggcagtgggtctgggaccgactataccctcacaatcagcagcctgcagcccgaagatttcgccacttattactgccagcagtggagtcgtaacccacccacgttcggaggggggaccaagctacaaattacatcctccagctaa

SEQ ID NO: 106 - protein, 747 aa, Artificial Sequence
  ROR154 Anti-ROR1 X anti-CD3 bispecific molecule
DIQMTQSPSSLSASVGDRVTINCQASQSIDSNLAWFQQKPGKPPKLLIYRASNLASGVPSRFSGSGSGTDFTLTISSLQPEDVATYYCLGGVGAVSYRTSFGGGTKVEIKGGGGSGGGGSGGGGSGGGGSEVQLVESGGGLVQPGRSLRLSCTASGSDINDYPITWVRQAPGKGLEWIGFINSGGSTWYASWVKGRFTISRDDSKSIAYLQMNSLKTEDTAVYYCARGYSTYYRDFNIWGQGTLVTVSSSEPKSSDKTHTCPPCPAPEAAGAPSVFLFPPKPKDTLMISRTPEVTCVVVDVSHEDPEVKFNWYVDGVEVHNAKTKPREEQYNSTYRVVSVLTVLHQDWLNGKEYKCAVSNKALPAPIEKTISKAKGQPREPQVYTLPPSRDELTKNQVSLTCLVKGFYPSDIAVEWESNGQPENNYKTTPPVLDSDGSFFLYSKLTVDKSRWQQGNVFSCSVMHEALHNHYTQKSLSLSPGSGGGGSGGGGSGGGGSPGSQVQLVESGGGVVQPGRSLRLSCKASGYTFTRSTMHWVRQAPGQGLEWIGYINPSSAYTNYNQKFKDRFTISADKSKSTAFLQMDSLRPEDTGVYFCARPQVHYDYNGFPYWGQGTPVTVSSGGGGSGGGGSGGGGSAQDIQMTQSPSSLSASVGDRVTMTCSASSSVSYMNWYQQKPGKAPKRWIYDSSKLASGVPARFSGSGSGTDYTLTISSLQPEDFATYYCQQWSRNPPTFGGGTKLQITSSS

SEQ ID NO: 107 - DNA, 2316 bp, Artificial Sequence
  ROR185 Anti-ROR1 X anti-CD3 bispecific molecule
atggaagcaccagcgcagcttctcttcctcctgctactctggctcccagataccaccggtgacatccagatgacccagtccccctcctccctgtccgcctccgtgggcgaccgggtgaccatcaactgccaggcctcccagtccatcgactccaacctggcctggttccagcagaagcccggcaagccccccaagctgctgatctaccgggcctccaacctggcctccggcgtgccctcccggttctccggctccggctccggcaccgacttcaccctgaccatctcctccctgcagcccgaggacgtggccacctactactgcctgggcggcgtgggcgccgtgtcctaccggacctccttcggcggcggcaccaaggtggagatcaagggtggaggcggttcaggcggaggtggatccggcggtggcggctccggtggcggcggatctgaggtgcagctggtggagtccggcggcggcctggtgcagcccggccggtccctgcggctgtcctgcaccgcctccggctccgacatcaacgactaccccatcacctgggtgcggcaggcccccggcaagggcctggagtggatcggcttcatcaactccggcggctccacctggtacgcctcctgggtgaagggccggttcaccatctcccgggacgactccaagtccatcgcctacctgcagatgaactccctgaagaccgaggacaccgccgtgtactattgcgcccggggctactccacctactaccgggacttcaacatctggggccagggcaccctggtgaccgtgtcctcgagtgagcccaaatcttctgacaaaactcacacatgcccaccgtgcccagcacctgaagccgcgggtgcaccgtcagtcttcctcttccccccaaaacccaaggacaccctcatgatctcccggacccctgaggtcacatgcgtggtggtggacgtgagccacgaagaccctgaggtcaagttcaactggtacgtggacggcgtggaggtgcataatgccaagacaaagccgcgggaggagcagtacaacagcacgtaccgtgtggtcagcgtcctcaccgtcctgcaccaggactggctgaatggcaaggaatacaagtgcgcggtctccaacaaagccctcccagcccccatcgagaaaaccatctccaaagccaaagggcagccccgagaaccacaggtgtacaccctgcccccatcccgggatgagctgaccaagaaccaggtcagcctgacctgcctggtcaaaggcttctatccaagcgacatcgccgtggagtgggagagcaatgggcagccggagaacaactacaagaccacgcctcccgtgctggactccgacggctccttcttcctctacagcaagctcaccgtggacaagagcaggtggcagcaggggaacgtcttctcatgctccgtgatgcatgaggctctgcacaaccactacacgcagaagagcctctccctgtctccgggttctggtggaggcggttcaggcggaggtggctccggcggtggcggatcgccgggctctcaggtccagctggtgcaatctgggcctgaggtgaagaagcctgggtcctcggtgaaggtctcctgcaaggcttctggatataccttcagcagatctacgatgcactgggtgcgacaggcccctggacaagggcttgagtggataggatacattaatcctagcagtgcttatactaattacaatcagaaattcaaggacagagtcacgattaccgcggacaaatccacgagcacagcctacatggagctgagcagcctgagatctgaggacacggccgtgtattactgtgcgagaccccaagtccactatgattacaacgggtttccttactggggccaaggaaccctggtcaccgtctcctcaggtggaggcggttcaggcggaggtggatccggcggtggcggatcgggtggcggcggatctgacatccagatgacccagtctccttccaccctgtctgcatctgtaggagacagagtcaccatgacttgcagtgccagctcaagtgtaagttacatgaactggtatcagcagaaaccagggaaagcccctaagagatggatttatgactcatccaaactggcttctggggtcccatcaaggttcagcggcagtggatctgggacagattatactctcaccatcagcagcctgcagcctgatgattttgcaacttattactgccaacagtggagtcgtaacccacccactttcggcggagggaccaaggtggagatcaaacggtcctccagctaa

SEQ ID NO: 108 - protein, 751 aa, Artificial Sequence
  ROR185 Anti-ROR1 X anti-CD3 bispecific molecule
DIQMTQSPSSLSASVGDRVTINCQASQSIDSNLAWFQQKPGKPPKLLIYRASNLASGVPSRFSGSGSGTDFTLTISSLQPEDVATYYCLGGVGAVSYRTSFGGGTKVEIKGGGGSGGGGSGGGGSGGGGSEVQLVESGGGLVQPGRSLRLSCTASGSDINDYPITWVRQAPGKGLEWIGFINSGGSTWYASWVKGRFTISRDDSKSIAYLQMNSLKTEDTAVYYCARGYSTYYRDFNIWGQGTLVTVSSSEPKSSDKTHTCPPCPAPEAAGAPSVFLFPPKPKDTLMISRTPEVTCVVVDVSHEDPEVKFNWYVDGVEVHNAKTKPREEQYNSTYRVVSVLTVLHQDWLNGKEYKCAVSNKALPAPIEKTISKAKGQPREPQVYTLPPSRDELTKNQVSLTCLVKGFYPSDIAVEWESNGQPENNYKTTPPVLDSDGSFFLYSKLTVDKSRWQQGNVFSCSVMHEALHNHYTQKSLSLSPGSGGGGSGGGGSGGGGSPGSQVQLVQSGPEVKKPGSSVKVSCKASGYTFSRSTMHWVRQAPGQGLEWIGYINPSSAYTNYNQKFKDRVTITADKSTSTAYMELSSLRSEDTAVYYCARPQVHYDYNGFPYWGQGTLVTVSSGGGGSGGGGSGGGGSGGGGSDIQMTQSPSTLSASVGDRVTMTCSASSSVSYMNWYQQKPGKAPKRWIYDSSKLASGVPSRFSGSGSGTDYTLTISSLQPDDFATYYCQQWSRNPPTFGGGTKVEIKRSSS

SEQ ID NO: 109 - DNA, 2304 bp, Artificial Sequence
  ROR179 Anti-ROR1 X anti-CD3 bispecific molecule
atggaagcaccagcgcagcttctcttcctcctgctactctggctcccagataccaccggtgacatccagatgacccagtccccctcctccctgtccgcctccgtgggcgaccgggtgaccatcaactgccaggcctcccagtccatcgactccaacctggcctggttccagcagaagcccggcaagccccccaagctgctgatctaccgggcctccaacctggcctccggcgtgccctcccggttctccggctccggctccggcaccgacttcaccctgaccatctcctccctgcagcccgaggacgtggccacctactactgcctgggcggcgtgggcgccgtgtcctactggacctccttcggcggcggcaccaaggtggagatcaagggtggaggcggttcaggcggaggtggatccggcggtggcggctccggtggcggcggatctgaggtgcagctggtggagtccggcggcggcctggtgcagcccggccggtccctgcggctgtcctgcaccgcctccggctccgacatcaacgactaccccatcacctgggtgcggcaggcccccggcaagggcctggagtggatcggcttcatcaactccggcggctccacctggtacgcctcctgggtgaagggccggttcaccatctcccgggacgactccaagtccatcgcctacctgcagatgaactccctgaagaccgaggacaccgccgtgtactattgcgcccggggctactccacctactaccgggacttcaacatctggggccagggcaccctggtgaccgtgtcctcgagtgagcccaaatcttctgacaaaactcacacatgcccaccgtgcccagcacctgaagccgcgggtgcaccgtcagtcttcctcttccccccaaaacccaaggacaccctcatgatctcccggacccctgaggtcacatgcgtggtggtggacgtgagccacgaagaccctgaggtcaagttcaactggtacgtggacggcgtggaggtgcataatgccaagacaaagccgcgggaggagcagtacaacagcacgtaccgtgtggtcagcgtcctcaccgtcctgcaccaggactggctgaatggcaaggaatacaagtgcgcggtctccaacaaagccctcccagcccccatcgagaaaaccatctccaaagccaaagggcagccccgagaaccacaggtgtacaccctgcccccatcccgggatgagctgaccaagaaccaggtcagcctgacctgcctggtcaaaggcttctatccaagcgacatcgccgtggagtgggagagcaatgggcagccggagaacaactacaagaccacgcctcccgtgctggactccgacggctccttcttcctctacagcaagctcaccgtggacaagagcaggtggcagcaggggaacgtcttctcatgctccgtgatgcatgaggctctgcacaaccactacacgcagaagagcctctccctgtctccgggttctggtggaggcggttcaggcggaggtggctccggcggtggcggatcgccgggctctcaggtccagctggtggagtctgggggcggagtggtgcagcctgggcggtcactgaggctgtcctgcaaggcttctggctacacctttactagatctacgatgcactgggtaaggcaggcccctggacaaggtctggaatggattggatacattaatcctagcagtgcttatactaattacaatcagaaattcaaggacaggttcacaatcagcgcagacaaatccaagagcacagccttcctgcagatggacagcctgaggcccgaggacaccggcgtctatttctgtgcacggccccaagtccactatgattacaacgggtttccttactggggccaagggactcccgtcactgtctctagcggtggcggagggtctgggggtggcggatccggaggtggtggctctgcacaagacatccagatgacccagtctccaagcagcctgtctgcaagcgtgggggacagggtcaccatgacctgcagtgccagctcaagtgtaagttacatgaactggtaccagcagaagccgggcaaggcccccaaaagatggatttatgactcatccaaactggcttctggagtccctgctcgcttcagtggcagtgggtctgggaccgactataccctcacaatcagcagcctgcagcccgaagatttcgccacttattactgccagcagtggagtcgtaacccacccacgttcggaggggggaccaagctacaaattacatcctccagctaa

SEQ ID NO: 110 - protein, 747 aa, Artificial Sequence
  ROR179 Anti-ROR1 X anti-CD3 bispecific molecule
DIQMTQSPSSLSASVGDRVTINCQASQSIDSNLAWFQQKPGKPPKLLIYRASNLASGVPSRFSGSGSGTDFTLTISSLQPEDVATYYCLGGVGAVSYWTSFGGGTKVEIKGGGGSGGGGSGGGGSGGGGSEVQLVESGGGLVQPGRSLRLSCTASGSDINDYPITWVRQAPGKGLEWIGFINSGGSTWYASWVKGRFTISRDDSKSIAYLQMNSLKTEDTAVYYCARGYSTYYRDFNIWGQGTLVTVSSSEPKSSDKTHTCPPCPAPEAAGAPSVFLFPPKPKDTLMISRTPEVTCVVVDVSHEDPEVKFNWYVDGVEVHNAKTKPREEQYNSTYRVVSVLTVLHQDWLNGKEYKCAVSNKALPAPIEKTISKAKGQPREPQVYTLPPSRDELTKNQVSLTCLVKGFYPSDIAVEWESNGQPENNYKTTPPVLDSDGSFFLYSKLTVDKSRWQQGNVFSCSVMHEALHNHYTQKSLSLSPGSGGGGSGGGGSGGGGSPGSQVQLVESGGGVVQPGRSLRLSCKASGYTFTRSTMHWVRQAPGQGLEWIGYINPSSAYTNYNQKFKDRFTISADKSKSTAFLQMDSLRPEDTGVYFCARPQVHYDYNGFPYWGQGTPVTVSSGGGGSGGGGSGGGGSAQDIQMTQSPSSLSASVGDRVTMTCSASSSVSYMNWYQQKPGKAPKRWIYDSSKLASGVPARFSGSGSGTDYTLTISSLQPEDFATYYCQQWSRNPPTFGGGTKLQITSSS

SEQ ID NO: 111 - DNA, 2316 bp, Artificial Sequence
  ROR186 Anti-ROR1 X anti-CD3 bispecific molecule
atggaagcaccagcgcagcttctcttcctcctgctactctggctcccagataccaccggtgacatccagatgacccagtccccctcctccctgtccgcctccgtgggcgaccgggtgaccatcaactgccaggcctcccagtccatcgactccaacctggcctggttccagcagaagcccggcaagccccccaagctgctgatctaccgggcctccaacctggcctccggcgtgccctcccggttctccggctccggctccggcaccgacttcaccctgaccatctcctccctgcagcccgaggacgtggccacctactactgcctgggcggcgtgggcgccgtgtcctactggacctccttcggcggcggcaccaaggtggagatcaagggtggaggcggttcaggcggaggtggatccggcggtggcggctccggtggcggcggatctgaggtgcagctggtggagtccggcggcggcctggtgcagcccggccggtccctgcggctgtcctgcaccgcctccggctccgacatcaacgactaccccatcacctgggtgcggcaggcccccggcaagggcctggagtggatcggcttcatcaactccggcggctccacctggtacgcctcctgggtgaagggccggttcaccatctcccgggacgactccaagtccatcgcctacctgcagatgaactccctgaagaccgaggacaccgccgtgtactattgcgcccggggctactccacctactaccgggacttcaacatctggggccagggcaccctggtgaccgtgtcctcgagtgagcccaaatcttctgacaaaactcacacatgcccaccgtgcccagcacctgaagccgcgggtgcaccgtcagtcttcctcttccccccaaaacccaaggacaccctcatgatctcccggacccctgaggtcacatgcgtggtggtggacgtgagccacgaagaccctgaggtcaagttcaactggtacgtggacggcgtggaggtgcataatgccaagacaaagccgcgggaggagcagtacaacagcacgtaccgtgtggtcagcgtcctcaccgtcctgcaccaggactggctgaatggcaaggaatacaagtgcgcggtctccaacaaagccctcccagcccccatcgagaaaaccatctccaaagccaaagggcagccccgagaaccacaggtgtacaccctgcccccatcccgggatgagctgaccaagaaccaggtcagcctgacctgcctggtcaaaggcttctatccaagcgacatcgccgtggagtgggagagcaatgggcagccggagaacaactacaagaccacgcctcccgtgctggactccgacggctccttcttcctctacagcaagctcaccgtggacaagagcaggtggcagcaggggaacgtcttctcatgctccgtgatgcatgaggctctgcacaaccactacacgcagaagagcctctccctgtctccgggttctggtggaggcggttcaggcggaggtggctccggcggtggcggatcgccgggctctcaggtccagctggtgcaatctgggcctgaggtgaagaagcctgggtcctcggtgaaggtctcctgcaaggcttctggatataccttcagcagatctacgatgcactgggtgcgacaggcccctggacaagggcttgagtggataggatacattaatcctagcagtgcttatactaattacaatcagaaattcaaggacagagtcacgattaccgcggacaaatccacgagcacagcctacatggagctgagcagcctgagatctgaggacacggccgtgtattactgtgcgagaccccaagtccactatgattacaacgggtttccttactggggccaaggaaccctggtcaccgtctcctcaggtggaggcggttcaggcggaggtggatccggcggtggcggatcgggtggcggcggatctgacatccagatgacccagtctccttccaccctgtctgcatctgtaggagacagagtcaccatgacttgcagtgccagctcaagtgtaagttacatgaactggtatcagcagaaaccagggaaagcccctaagagatggatttatgactcatccaaactggcttctggggtcccatcaaggttcagcggcagtggatctgggacagattatactctcaccatcagcagcctgcagcctgatgattttgcaacttattactgccaacagtggagtcgtaacccacccactttcggcggagggaccaaggtggagatcaaacggtcctccagctaa

SEQ ID NO: 112 - protein, 751 aa, Artificial Sequence
  ROR186 Anti-ROR1 X anti-CD3 bispecific molecule
DIQMTQSPSSLSASVGDRVTINCQASQSIDSNLAWFQQKPGKPPKLLIYRASNLASGVPSRFSGSGSGTDFTLTISSLQPEDVATYYCLGGVGAVSYWTSFGGGTKVEIKGGGGSGGGGSGGGGSGGGGSEVQLVESGGGLVQPGRSLRLSCTASGSDINDYPITWVRQAPGKGLEWIGFINSGGSTWYASWVKGRFTISRDDSKSIAYLQMNSLKTEDTAVYYCARGYSTYYRDFNIWGQGTLVTVSSSEPKSSDKTHTCPPCPAPEAAGAPSVFLFPPKPKDTLMISRTPEVTCVVVDVSHEDPEVKFNWYVDGVEVHNAKTKPREEQYNSTYRVVSVLTVLHQDWLNGKEYKCAVSNKALPAPIEKTISKAKGQPREPQVYTLPPSRDELTKNQVSLTCLVKGFYPSDIAVEWESNGQPENNYKTTPPVLDSDGSFFLYSKLTVDKSRWQQGNVFSCSVMHEALHNHYTQKSLSLSPGSGGGGSGGGGSGGGGSPGSQVQLVQSGPEVKKPGSSVKVSCKASGYTFSRSTMHWVRQAPGQGLEWIGYINPSSAYTNYNQKFKDRVTITADKSTSTAYMELSSLRSEDTAVYYCARPQVHYDYNGFPYWGQGTLVTVSSGGGGSGGGGSGGGGSGGGGSDIQMTQSPSTLSASVGDRVTMTCSASSSVSYMNWYQQKPGKAPKRWIYDSSKLASGVPSRFSGSGSGTDYTLTISSLQPDDFATYYCQQWSRNPPTFGGGTKVEIKRSSS

SEQ ID NO: 113 - DNA, 2304 bp, Artificial Sequence
  ROR181 Anti-ROR1 X anti-CD3 bispecific molecule
atggaagcaccagcgcagcttctcttcctcctgctactctggctcccagataccaccggtgacatccagatgacccagtccccctcctccctgtccgcctccgtgggcgaccgggtgaccatcaactgccaggcctcccagtccatcgactccaacctggcctggttccagcagaagcccggcaagccccccaagctgctgatctaccgggcctccaacctggcctccggcgtgccctcccggttctccggctccggctccggcaccgacttcaccctgaccatctcctccctgcagcccgaggacgtggccacctactactgcctgggcggcgtgggcgccgtgtcctaccggacctccttcggcggcggcaccaaggtggagatcaagggtggaggcggttcaggcggaggtggatccggcggtggcggctccggtggcggcggatctgaggtgcagctggtggagtccggcggcggcctggtgcagcccggcggctccctgcggctgtcctgcaccgtgtccggcaccgacatcaacgactaccccatctcctgggtgcggcaggcccccggcaagggcctggagtggatcggcttcatcaactccggcggctccacctggtacgccgactcggtgaagggccggttcaccatctcccggcactcctccaagaacaccctgtacctgcagatgaactccctgcgggccgaggacaccgccgtgtacttctgcgcccggggctactccacctactaccgggacttcaacatctggggccagggcaccctggtgaccgtgtcctcgagtgagcccaaatcttctgacaaaactcacacatgcccaccgtgcccagcacctgaagccgcgggtgcaccgtcagtcttcctcttccccccaaaacccaaggacaccctcatgatctcccggacccctgaggtcacatgcgtggtggtggacgtgagccacgaagaccctgaggtcaagttcaactggtacgtggacggcgtggaggtgcataatgccaagacaaagccgcgggaggagcagtacaacagcacgtaccgtgtggtcagcgtcctcaccgtcctgcaccaggactggctgaatggcaaggaatacaagtgcgcggtctccaacaaagccctcccagcccccatcgagaaaaccatctccaaagccaaagggcagccccgagaaccacaggtgtacaccctgcccccatcccgggatgagctgaccaagaaccaggtcagcctgacctgcctggtcaaaggcttctatccaagcgacatcgccgtggagtgggagagcaatgggcagccggagaacaactacaagaccacgcctcccgtgctggactccgacggctccttcttcctctacagcaagctcaccgtggacaagagcaggtggcagcaggggaacgtcttctcatgctccgtgatgcatgaggctctgcacaaccactacacgcagaagagcctctccctgtctccgggttctggtggaggcggttcaggcggaggtggctccggcggtggcggatcgccgggctctcaggtccagctggtggagtctgggggcggagtggtgcagcctgggcggtcactgaggctgtcctgcaaggcttctggctacacctttactagatctacgatgcactgggtaaggcaggcccctggacaaggtctggaatggattggatacattaatcctagcagtgcttatactaattacaatcagaaattcaaggacaggttcacaatcagcgcagacaaatccaagagcacagccttcctgcagatggacagcctgaggcccgaggacaccggcgtctatttctgtgcacggccccaagtccactatgattacaacgggtttccttactggggccaagggactcccgtcactgtctctagcggtggcggagggtctgggggtggcggatccggaggtggtggctctgcacaagacatccagatgacccagtctccaagcagcctgtctgcaagcgtgggggacagggtcaccatgacctgcagtgccagctcaagtgtaagttacatgaactggtaccagcagaagccgggcaaggcccccaaaagatggatttatgactcatccaaactggcttctggagtccctgctcgcttcagtggcagtgggtctgggaccgactataccctcacaatcagcagcctgcagcccgaagatttcgccacttattactgccagcagtggagtcgtaacccacccacgttcggaggggggaccaagctacaaattacatcctccagctaa

SEQ ID NO: 114 - protein, 747 aa, Artificial Sequence
  ROR181 Anti-ROR1 X anti-CD3 bispecific molecule
DIQMTQSPSSLSASVGDRVTINCQASQSIDSNLAWFQQKPGKPPKLLIYRASNLASGVPSRFSGSGSGTDFTLTISSLQPEDVATYYCLGGVGAVSYRTSFGGGTKVEIKGGGGSGGGGSGGGGSGGGGSEVQLVESGGGLVQPGGSLRLSCTVSGTDINDYPISWVRQAPGKGLEWIGFINSGGSTWYADSVKGRFTISRHSSKNTLYLQMNSLRAEDTAVYFCARGYSTYYRDFNIWGQGTLVTVSSSEPKSSDKTHTCPPCPAPEAAGAPSVFLFPPKPKDTLMISRTPEVTCVVVDVSHEDPEVKFNWYVDGVEVHNAKTKPREEQYNSTYRVVSVLTVLHQDWLNGKEYKCAVSNKALPAPIEKTISKAKGQPREPQVYTLPPSRDELTKNQVSLTCLVKGFYPSDIAVEWESNGQPENNYKTTPPVLDSDGSFFLYSKLTVDKSRWQQGNVFSCSVMHEALHNHYTQKSLSLSPGSGGGGSGGGGSGGGGSPGSQVQLVESGGGVVQPGRSLRLSCKASGYTFTRSTMHWVRQAPGQGLEWIGYINPSSAYTNYNQKFKDRFTISADKSKSTAFLQMDSLRPEDTGVYFCARPQVHYDYNGFPYWGQGTPVTVSSGGGGSGGGGSGGGGSAQDIQMTQSPSSLSASVGDRVTMTCSASSSVSYMNWYQQKPGKAPKRWIYDSSKLASGVPARFSGSGSGTDYTLTISSLQPEDFATYYCQQWSRNPPTFGGGTKLQITSSS

SEQ ID NO: 115 - DNA, 2316 bp, Artificial Sequence
  ROR191 Anti-ROR1 X anti-CD3 bispecific molecule
atggaagcaccagcgcagcttctcttcctcctgctactctggctcccagataccaccggtgacatccagatgacccagtccccctcctccctgtccgcctccgtgggcgaccgggtgaccatcaactgccaggcctcccagtccatcgactccaacctggcctggttccagcagaagcccggcaagccccccaagctgctgatctaccgggcctccaacctggcctccggcgtgccctcccggttctccggctccggctccggcaccgacttcaccctgaccatctcctccctgcagcccgaggacgtggccacctactactgcctgggcggcgtgggcgccgtgtcctaccggacctccttcggcggcggcaccaaggtggagatcaagggtggaggcggttcaggcggaggtggatccggcggtggcggctccggtggcggcggatctgaggtgcagctggtggagtccggcggcggcctggtgcagcccggcggctccctgcggctgtcctgcaccgtgtccggcaccgacatcaacgactaccccatctcctgggtgcggcaggcccccggcaagggcctggagtggatcggcttcatcaactccggcggctccacctggtacgccgactcggtgaagggccggttcaccatctcccggcactcctccaagaacaccctgtacctgcagatgaactccctgcgggccgaggacaccgccgtgtacttctgcgcccggggctactccacctactaccgggacttcaacatctggggccagggcaccctggtgaccgtgtcctcgagtgagcccaaatcttctgacaaaactcacacatgcccaccgtgcccagcacctgaagccgcgggtgcaccgtcagtcttcctcttccccccaaaacccaaggacaccctcatgatctcccggacccctgaggtcacatgcgtggtggtggacgtgagccacgaagaccctgaggtcaagttcaactggtacgtggacggcgtggaggtgcataatgccaagacaaagccgcgggaggagcagtacaacagcacgtaccgtgtggtcagcgtcctcaccgtcctgcaccaggactggctgaatggcaaggaatacaagtgcgcggtctccaacaaagccctcccagcccccatcgagaaaaccatctccaaagccaaagggcagccccgagaaccacaggtgtacaccctgcccccatcccgggatgagctgaccaagaaccaggtcagcctgacctgcctggtcaaaggcttctatccaagcgacatcgccgtggagtgggagagcaatgggcagccggagaacaactacaagaccacgcctcccgtgctggactccgacggctccttcttcctctacagcaagctcaccgtggacaagagcaggtggcagcaggggaacgtcttctcatgctccgtgatgcatgaggctctgcacaaccactacacgcagaagagcctctccctgtctccgggttctggtggaggcggttcaggcggaggtggctccggcggtggcggatcgccgggctctcaggtccagctggtgcaatctgggcctgaggtgaagaagcctgggtcctcggtgaaggtctcctgcaaggcttctggatataccttcagcagatctacgatgcactgggtgcgacaggcccctggacaagggcttgagtggataggatacattaatcctagcagtgcttatactaattacaatcagaaattcaaggacagagtcacgattaccgcggacaaatccacgagcacagcctacatggagctgagcagcctgagatctgaggacacggccgtgtattactgtgcgagaccccaagtccactatgattacaacgggtttccttactggggccaaggaaccctggtcaccgtctcctcaggtggaggcggttcaggcggaggtggatccggcggtggcggatcgggtggcggcggatctgacatccagatgacccagtctccttccaccctgtctgcatctgtaggagacagagtcaccatgacttgcagtgccagctcaagtgtaagttacatgaactggtatcagcagaaaccagggaaagcccctaagagatggatttatgactcatccaaactggcttctggggtcccatcaaggttcagcggcagtggatctgggacagattatactctcaccatcagcagcctgcagcctgatgattttgcaacttattactgccaacagtggagtcgtaacccacccactttcggcggagggaccaaggtggagatcaaacggtcctccagctaa

SEQ ID NO: 116 - protein, 751 aa, Artificial Sequence
  ROR191 Anti-ROR1 X anti-CD3 bispecific molecule
DIQMTQSPSSLSASVGDRVTINCQASQSIDSNLAWFQQKPGKPPKLLIYRASNLASGVPSRFSGSGSGTDFTLTISSLQPEDVATYYCLGGVGAVSYRTSFGGGTKVEIKGGGGSGGGGSGGGGSGGGGSEVQLVESGGGLVQPGGSLRLSCTVSGTDINDYPISWVRQAPGKGLEWIGFINSGGSTWYADSVKGRFTISRHSSKNTLYLQMNSLRAEDTAVYFCARGYSTYYRDFNIWGQGTLVTVSSSEPKSSDKTHTCPPCPAPEAAGAPSVFLFPPKPKDTLMISRTPEVTCVVVDVSHEDPEVKFNWYVDGVEVHNAKTKPREEQYNSTYRVVSVLTVLHQDWLNGKEYKCAVSNKALPAPIEKTISKAKGQPREPQVYTLPPSRDELTKNQVSLTCLVKGFYPSDIAVEWESNGQPENNYKTTPPVLDSDGSFFLYSKLTVDKSRWQQGNVFSCSVMHEALHNHYTQKSLSLSPGSGGGGSGGGGSGGGGSPGSQVQLVQSGPEVKKPGSSVKVSCKASGYTFSRSTMHWVRQAPGQGLEWIGYINPSSAYTNYNQKFKDRVTITADKSTSTAYMELSSLRSEDTAVYYCARPQVHYDYNGFPYWGQGTLVTVSSGGGGSGGGGSGGGGSGGGGSDIQMTQSPSTLSASVGDRVTMTCSASSSVSYMNWYQQKPGKAPKRWIYDSSKLASGVPSRFSGSGSGTDYTLTISSLQPDDFATYYCQQWSRNPPTFGGGTKVEIKRSSS

SEQ ID NO: 117 - DNA, 2304 bp, Artificial Sequence
  ROR182 Anti-ROR1 X anti-CD3 bispecific molecule
atggaagcaccagcgcagcttctcttcctcctgctactctggctcccagataccaccggtgacatccagatgacccagtccccctcctccctgtccgcctccgtgggcgaccgggtgaccatcaactgccaggcctcccagtccatcgactccaacctggcctggttccagcagaagcccggccagccccccaagctgctgatctaccgggcctccaacctggcctccggcgtgcccgaccggttctccggctccggctccggcaccgacttcaccctgaccatctcctccctggaggccgaggacgtggccacctactactgcctgggcggcgtgggcgccgtgtcctaccggacctccttcggcggcggcaccaaggtggagatcaagggtggaggcggttcaggcggaggtggatccggcggtggcggctccggtggcggcggatctgaggtgcagctggtggagtccggcggcggcctggtgcagcccggccggtccctgcggctgtcctgcaccgcctccggctccgacatcaacgactaccccatcacctgggtgcggcaggcccccggccagggcctggagtggatcggcttcatcaactccggcggctccacctggtacgcctcctgggtgaagggccggttcaccatctcccgggacgactccaagtccatcgcctacctgcagatgaactccctgaagaccgaggacaccgccgtgtactattgcgcccggggctactccacctactaccgggacttcaacatctggggccagggcaccctggtgaccgtgtcctcgagtgagcccaaatcttctgacaaaactcacacatgcccaccgtgcccagcacctgaagccgcgggtgcaccgtcagtcttcctcttccccccaaaacccaaggacaccctcatgatctcccggacccctgaggtcacatgcgtggtggtggacgtgagccacgaagaccctgaggtcaagttcaactggtacgtggacggcgtggaggtgcataatgccaagacaaagccgcgggaggagcagtacaacagcacgtaccgtgtggtcagcgtcctcaccgtcctgcaccaggactggctgaatggcaaggaatacaagtgcgcggtctccaacaaagccctcccagcccccatcgagaaaaccatctccaaagccaaagggcagccccgagaaccacaggtgtacaccctgcccccatcccgggatgagctgaccaagaaccaggtcagcctgacctgcctggtcaaaggcttctatccaagcgacatcgccgtggagtgggagagcaatgggcagccggagaacaactacaagaccacgcctcccgtgctggactccgacggctccttcttcctctacagcaagctcaccgtggacaagagcaggtggcagcaggggaacgtcttctcatgctccgtgatgcatgaggctctgcacaaccactacacgcagaagagcctctccctgtctccgggttctggtggaggcggttcaggcggaggtggctccggcggtggcggatcgccgggctctcaggtccagctggtggagtctgggggcggagtggtgcagcctgggcggtcactgaggctgtcctgcaaggcttctggctacacctttactagatctacgatgcactgggtaaggcaggcccctggacaaggtctggaatggattggatacattaatcctagcagtgcttatactaattacaatcagaaattcaaggacaggttcacaatcagcgcagacaaatccaagagcacagccttcctgcagatggacagcctgaggcccgaggacaccggcgtctatttctgtgcacggccccaagtccactatgattacaacgggtttccttactggggccaagggactcccgtcactgtctctagcggtggcggagggtctgggggtggcggatccggaggtggtggctctgcacaagacatccagatgacccagtctccaagcagcctgtctgcaagcgtgggggacagggtcaccatgacctgcagtgccagctcaagtgtaagttacatgaactggtaccagcagaagccgggcaaggcccccaaaagatggatttatgactcatccaaactggcttctggagtccctgctcgcttcagtggcagtgggtctgggaccgactataccctcacaatcagcagcctgcagcccgaagatttcgccacttattactgccagcagtggagtcgtaacccacccacgttcggaggggggaccaagctacaaattacatcctccagctaa

SEQ ID NO: 118 - protein, 747 aa, Artificial Sequence
  ROR182 Anti-ROR1 X anti-CD3 bispecific molecule
DIQMTQSPSSLSASVGDRVTINCQASQSIDSNLAWFQQKPGQPPKLLIYRASNLASGVPDRFSGSGSGTDFTLTISSLEAEDVATYYCLGGVGAVSYRTSFGGGTKVEIKGGGGSGGGGSGGGGSGGGGSEVQLVESGGGLVQPGRSLRLSCTASGSDINDYPITWVRQAPGQGLEWIGFINSGGSTWYASWVKGRFTISRDDSKSIAYLQMNSLKTEDTAVYYCARGYSTYYRDFNIWGQGTLVTVSSSEPKSSDKTHTCPPCPAPEAAGAPSVFLFPPKPKDTLMISRTPEVTCVVVDVSHEDPEVKFNWYVDGVEVHNAKTKPREEQYNSTYRVVSVLTVLHQDWLNGKEYKCAVSNKALPAPIEKTISKAKGQPREPQVYTLPPSRDELTKNQVSLTCLVKGFYPSDIAVEWESNGQPENNYKTTPPVLDSDGSFFLYSKLTVDKSRWQQGNVFSCSVMHEALHNHYTQKSLSLSPGSGGGGSGGGGSGGGGSPGSQVQLVESGGGVVQPGRSLRLSCKASGYTFTRSTMHWVRQAPGQGLEWIGYINPSSAYTNYNQKFKDRFTISADKSKSTAFLQMDSLRPEDTGVYFCARPQVHYDYNGFPYWGQGTPVTVSSGGGGSGGGGSGGGGSAQDIQMTQSPSSLSASVGDRVTMTCSASSSVSYMNWYQQKPGKAPKRWIYDSSKLASGVPARFSGSGSGTDYTLTISSLQPEDFATYYCQQWSRNPPTFGGGTKLQITSSS

SEQ ID NO: 119 - DNA, 2316 bp, Artificial Sequence
  ROR192 Anti-ROR1 X anti-CD3 bispecific molecule
atggaagcaccagcgcagcttctcttcctcctgctactctggctcccagataccaccggtgacatccagatgacccagtccccctcctccctgtccgcctccgtgggcgaccgggtgaccatcaactgccaggcctcccagtccatcgactccaacctggcctggttccagcagaagcccggccagccccccaagctgctgatctaccgggcctccaacctggcctccggcgtgcccgaccggttctccggctccggctccggcaccgacttcaccctgaccatctcctccctggaggccgaggacgtggccacctactactgcctgggcggcgtgggcgccgtgtcctaccggacctccttcggcggcggcaccaaggtggagatcaagggtggaggcggttcaggcggaggtggatccggcggtggcggctccggtggcggcggatctgaggtgcagctggtggagtccggcggcggcctggtgcagcccggccggtccctgcggctgtcctgcaccgcctccggctccgacatcaacgactaccccatcacctgggtgcggcaggcccccggccagggcctggagtggatcggcttcatcaactccggcggctccacctggtacgcctcctgggtgaagggccggttcaccatctcccgggacgactccaagtccatcgcctacctgcagatgaactccctgaagaccgaggacaccgccgtgtactattgcgcccggggctactccacctactaccgggacttcaacatctggggccagggcaccctggtgaccgtgtcctcgagtgagcccaaatcttctgacaaaactcacacatgcccaccgtgcccagcacctgaagccgcgggtgcaccgtcagtcttcctcttccccccaaaacccaaggacaccctcatgatctcccggacccctgaggtcacatgcgtggtggtggacgtgagccacgaagaccctgaggtcaagttcaactggtacgtggacggcgtggaggtgcataatgccaagacaaagccgcgggaggagcagtacaacagcacgtaccgtgtggtcagcgtcctcaccgtcctgcaccaggactggctgaatggcaaggaatacaagtgcgcggtctccaacaaagccctcccagcccccatcgagaaaaccatctccaaagccaaagggcagccccgagaaccacaggtgtacaccctgcccccatcccgggatgagctgaccaagaaccaggtcagcctgacctgcctggtcaaaggcttctatccaagcgacatcgccgtggagtgggagagcaatgggcagccggagaacaactacaagaccacgcctcccgtgctggactccgacggctccttcttcctctacagcaagctcaccgtggacaagagcaggtggcagcaggggaacgtcttctcatgctccgtgatgcatgaggctctgcacaaccactacacgcagaagagcctctccctgtctccgggttctggtggaggcggttcaggcggaggtggctccggcggtggcggatcgccgggctctcaggtccagctggtgcaatctgggcctgaggtgaagaagcctgggtcctcggtgaaggtctcctgcaaggcttctggatataccttcagcagatctacgatgcactgggtgcgacaggcccctggacaagggcttgagtggataggatacattaatcctagcagtgcttatactaattacaatcagaaattcaaggacagagtcacgattaccgcggacaaatccacgagcacagcctacatggagctgagcagcctgagatctgaggacacggccgtgtattactgtgcgagaccccaagtccactatgattacaacgggtttccttactggggccaaggaaccctggtcaccgtctcctcaggtggaggcggttcaggcggaggtggatccggcggtggcggatcgggtggcggcggatctgacatccagatgacccagtctccttccaccctgtctgcatctgtaggagacagagtcaccatgacttgcagtgccagctcaagtgtaagttacatgaactggtatcagcagaaaccagggaaagcccctaagagatggatttatgactcatccaaactggcttctggggtcccatcaaggttcagcggcagtggatctgggacagattatactctcaccatcagcagcctgcagcctgatgattttgcaacttattactgccaacagtggagtcgtaacccacccactttcggcggagggaccaaggtggagatcaaacggtcctccagctaa

SEQ ID NO: 120 - protein, 751 aa, Artificial Sequence
  ROR192 Anti-ROR1 X anti-CD3 bispecific molecule
DIQMTQSPSSLSASVGDRVTINCQASQSIDSNLAWFQQKPGQPPKLLIYRASNLASGVPDRFSGSGSGTDFTLTISSLEAEDVATYYCLGGVGAVSYRTSFGGGTKVEIKGGGGSGGGGSGGGGSGGGGSEVQLVESGGGLVQPGRSLRLSCTASGSDINDYPITWVRQAPGQGLEWIGFINSGGSTWYASWVKGRFTISRDDSKSIAYLQMNSLKTEDTAVYYCARGYSTYYRDFNIWGQGTLVTVSSSEPKSSDKTHTCPPCPAPEAAGAPSVFLFPPKPKDTLMISRTPEVTCVVVDVSHEDPEVKFNWYVDGVEVHNAKTKPREEQYNSTYRVVSVLTVLHQDWLNGKEYKCAVSNKALPAPIEKTISKAKGQPREPQVYTLPPSRDELTKNQVSLTCLVKGFYPSDIAVEWESNGQPENNYKTTPPVLDSDGSFFLYSKLTVDKSRWQQGNVFSCSVMHEALHNHYTQKSLSLSPGSGGGGSGGGGSGGGGSPGSQVQLVQSGPEVKKPGSSVKVSCKASGYTFSRSTMHWVRQAPGQGLEWIGYINPSSAYTNYNQKFKDRVTITADKSTSTAYMELSSLRSEDTAVYYCARPQVHYDYNGFPYWGQGTLVTVSSGGGGSGGGGSGGGGSGGGGSDIQMTQSPSTLSASVGDRVTMTCSASSSVSYMNWYQQKPGKAPKRWIYDSSKLASGVPSRFSGSGSGTDYTLTISSLQPDDFATYYCQQWSRNPPTFGGGTKVEIKRSSS

SEQ ID NO: 121 - protein, 15 aa, Artificial Sequence
  sss(s)-hIgG1 hinge
EPKSSDKTHTSPPSS

SEQ ID NO: 122 - protein, 15 aa, Artificial Sequence
  csc(s)-hIgG1 hinge
EPKSCDKTHTSPPCS

SEQ ID NO: 123 - protein, 15 aa, Artificial Sequence
  ssc(s)-hIgG1 hinge
EPKSSDKTHTSPPCS

SEQ ID NO: 124 - protein, 15 aa, Artificial Sequence
  scc(s)-hIgG1 hinge
EPKSSDKTHTCPPCS

SEQ ID NO: 125 - protein, 15 aa, Artificial Sequence
  css(s)-hIgG1 hinge
EPKSCDKTHTSPPSS

SEQ ID NO: 126 - protein, 15 aa, Artificial Sequence
  scs(s)-hIgG1 hinge
EPKSSDKTHTCPPSS

SEQ ID NO: 127 - protein, 15 aa, Artificial Sequence
  ccc(s)-hIgG1 hinge
EPKSCDKTHTSPPCS

SEQ ID NO: 128 - protein, 15 aa, Artificial Sequence
  ccc(p)-hIgG1 hinge
EPKSCDKTHTSPPCP

SEQ ID NO: 129 - protein, 15 aa, Artificial Sequence
  sss(p)-hIgG1 hinge
EPKSSDKTHTSPPSP

SEQ ID NO: 130 - protein, 15 aa, Artificial Sequence
  csc(p)-hIgG1 hinge
EPKSCDKTHTSPPCP

SEQ ID NO: 131 - protein, 15 aa, Artificial Sequence
  ssc(p)-hIgG1 hinge
EPKSSDKTHTSPPCP

SEQ ID NO: 132 - protein, 15 aa, Artificial Sequence
  scc(p)-hIgG1 hinge
EPKSSDKTHTCPPCP

SEQ ID NO: 133 - protein, 15 aa, Artificial Sequence
  css(p)-hIgG1 hinge
EPKSCDKTHTSPPSP

SEQ ID NO: 134 - protein, 15 aa, Artificial Sequence
  scs(p)-hIgG1 hinge
EPKSSDKTHTCPPSP

SEQ ID NO: 135 - protein, 6 aa, Artificial Sequence
  Scppcp linker
SCPPCP

SEQ ID NO: 136 - protein, 20 aa, Artificial Sequence
  STD1 linker
NYGGGGSGGGGSGGGGSGNS

SEQ ID NO: 137 - protein, 38 aa, Artificial Sequence
  STD2 linker
NYGGGGSGGGGSGGGGSGNYGGGGSGGGGSGGGGSGNS

SEQ ID NO: 138 - protein, 2 aa, Artificial Sequence
  H1 linker
NS

SEQ ID NO: 139 - protein, 8 aa, Artificial Sequence
  H2 linker
GGGGSGNS

SEQ ID NO: 140 - protein, 10 aa, Artificial Sequence
  H3 linker
NYGGGGSGNS

SEQ ID NO: 141 - protein, 13 aa, Artificial Sequence
  H4 linker
GGGGSGGGGSGNS

SEQ ID NO: 142 - protein, 15 aa, Artificial Sequence
  H5 linker
NYGGGGSGGGGSGNS

SEQ ID NO: 143 - protein, 18 aa, Artificial Sequence
  H6 linker
GGGGSGGGGSGGGGSGNS

SEQ ID NO: 144 - protein, 8 aa, Artificial Sequence
  H7 linker
GCPPCPNS

SEQ ID NO: 145 - protein, 15 aa, Artificial Sequence
  (G4S)3 linker
GGGGSGGGGSGGGGS

SEQ ID NO: 146 - protein, 16 aa, Artificial Sequence
  H105 linker
SGGGGSGGGGSGGGGS

SEQ ID NO: 147 - protein, 20 aa, Artificial Sequence
  (G4S)4 linker
GGGGSGGGGSGGGGSGGGGS

SEQ ID NO: 148 - protein, 21 aa, Artificial Sequence
  H75 (NKG2A quadruple mutant) linker
QRHNNSSLNTGTQMAGHSPNS

SEQ ID NO: 149 - protein, 16 aa, Artificial Sequence
  H83 (NKG2A derived) linker
SSLNTGTQMAGHSPNS

SEQ ID NO: 150 - protein, 18 aa, Artificial Sequence
  H106 (NKG2A derived) linker
QRHNNSSLNTGTQMAGHS

SEQ ID NO: 151 - protein, 14 aa, Artificial Sequence
  H81 (NKG2D derived) linker
EVQIPLTESYSPNS

SEQ ID NO: 152 - protein, 20 aa, Artificial Sequence
  H91 (NKG2D derived) linker
NSLANQEVQIPLTESYSPNS

SEQ ID NO: 153 - protein, 19 aa, Artificial Sequence
  H94 linker
SGGGGSGGGGSGGGGSPNS

SEQ ID NO: 154 - protein, 15 aa, Artificial Sequence
  H16 hinge
LSVKADFLTPSIGNS

SEQ ID NO: 155 - protein, 20 aa, Artificial Sequence
  H17 hinge
LSVKADFLTPSISCPPCPNS

SEQ ID NO: 156 - protein, 15 aa, Artificial Sequence
  H18 hinge
LSVLANFSQPEIGNS

SEQ ID NO: 157 - protein, 20 aa, Artificial Sequence
  H19 hinge
LSVLANFSQPEISCPPCPNS

SEQ ID NO: 158 - protein, 15 aa, Artificial Sequence
  H20 hinge
LKIQERVSKPKISNS

SEQ ID NO: 159 - protein, 20 aa, Artificial Sequence
  H21 hinge
LKIQERVSKPKISCPPCPNS

SEQ ID NO: 160 - protein, 15 aa, Artificial Sequence
  H22 hinge
LNVSERPFPPHIQNS

SEQ ID NO: 161 - protein, 21 aa, Artificial Sequence
  H23 hinge
LDVSERPFPPHIQSCPPCPNS

SEQ ID NO: 162 - protein, 15 aa, Artificial Sequence
  H24 hinge
REQLAEVTLSLKANS

SEQ ID NO: 163 - protein, 20 aa, Artificial Sequence
  H25 hinge
REQLAEVTLSLKACPPCPNS

SEQ ID NO: 164 - protein, 15 aa, Artificial Sequence
  H26 hinge
RIHQMNSELSVLANS

SEQ ID NO: 165 - protein, 20 aa, Artificial Sequence
  H27 hinge
RIHQMNSELSVLACPPCPNS

SEQ ID NO: 166 - protein, 15 aa, Artificial Sequence
  H28 hinge
DTKGKNVLEKIFSNS

SEQ ID NO: 167 - protein, 15 aa, Artificial Sequence
  H30 hinge
LPPETQESQEVTLNS

SEQ ID NO: 168 - protein, 15 aa, Artificial Sequence
  H32 hinge
RIHLNVSERPFPPNS

SEQ ID NO: 169 - protein, 20 aa, Artificial Sequence
  H33 hinge
RIHLNVSERPFPPCPPCPNS

SEQ ID NO: 170 - protein, 13 aa, Artificial Sequence
  H36 hinge
GCPPCPGGGGSNS

SEQ ID NO: 171 - protein, 9 aa, Artificial Sequence
  H40 hinge
GCPPCPANS

SEQ ID NO: 172 - protein, 9 aa, Artificial Sequence
  H41 hinge
GCPPCPANS

SEQ ID NO: 173 - protein, 8 aa, Artificial Sequence
  H42 hinge
GCPPCPNS

SEQ ID NO: 174 - protein, 13 aa, Artificial Sequence
  H44 hinge
GGGASCPPCPGNS

SEQ ID NO: 175 - protein, 13 aa, Artificial Sequence
  H45 hinge
GGGASCPPCAGNS

SEQ ID NO: 176 - protein, 12 aa, Artificial Sequence
  H46 hinge
GGGASCPPCANS

SEQ ID NO: 177 - protein, 15 aa, Artificial Sequence
  H47 hinge
LSVKADFLTPSIGNS

SEQ ID NO: 178 - protein, 11 aa, Artificial Sequence
  H48 hinge
ADFLTPSIGNS

SEQ ID NO: 179 - protein, 15 aa, Artificial Sequence
  H50 hinge
LSVLANFSQPEIGNS

SEQ ID NO: 180 - protein, 15 aa, Artificial Sequence
  H51 hinge
LSVLANFSQPEIGNS

SEQ ID NO: 181 - protein, 11 aa, Artificial Sequence
  H52 hinge
SQPEIVPISNS

SEQ ID NO: 182 - protein, 16 aa, Artificial Sequence
  H53 hinge
SQPEIVPISCPPCPNS

SEQ ID NO: 183 - protein, 19 aa, Artificial Sequence
  H54 hinge
SVLANFSQPEISCPPCPNS

SEQ ID NO: 184 - protein, 15 aa, Artificial Sequence
  H55 hinge
RIHQMNSELSVLANS

SEQ ID NO: 185 - protein, 12 aa, Artificial Sequence
  H56 hinge
QMNSELSVLANS

SEQ ID NO: 186 - protein, 10 aa, Artificial Sequence
  H57 hinge
VSERPFPPNS

SEQ ID NO: 187 - protein, 15 aa, Artificial Sequence
  H58 hinge
KPFFTCGSADTCPNS

SEQ ID NO: 188 - protein, 15 aa, Artificial Sequence
  H59 hinge
KPFFTCGSADTCPNS

SEQ ID NO: 189 - protein, 15 aa, Artificial Sequence
  H60 hinge
QYNCPGQYTFSMPNS

SEQ ID NO: 190 - protein, 21 aa, Artificial Sequence
  H61 hinge
EPAFTPGPNIELQKDSDCPNS

SEQ ID NO: 191 - protein, 21 aa, Artificial Sequence
  H62 hinge
QRHNNSSLNTRTQKARHCPNS

SEQ ID NO: 192 - protein, 20 aa, Artificial Sequence
  H63 hinge
NSLFNQEVQIPLTESYCPNS

SEQ ID NO: 193 - protein, 15 aa, Artificial Sequence
  ((Gly4Ser)3) linker
GGGGSGGGGSGGGGS

SEQ ID NO: 194 - protein, 25 aa, Artificial Sequence
  (Gly4Ser)n linker
  MISC_FEATURE (6)..(25): amino acid residues may be absent
GGGGSGGGGSGGGGSGGGGSGGGGS

SEQ ID NO: 195 - protein, 20 aa, Artificial Sequence
  secretory signal sequence
MEAPAQLLFLLLLWLPDTTG

SEQ ID NO: 196 - protein, 19 aa, Artificial Sequence
  H111 linker
SGGGGSGGGGSGGGGSPGS

SEQ ID NO: 197 - protein, 751 aa, Artificial Sequence
  Chimeric bispecific anti-CD123 (VLVH) x anti-CD3 (TSC456) scFv-Fc-scFv CD3-binding domain
DIMMSQSPSSLAVSVGEKFTMTCKSSQSLFFGSTQKNYLAWYQQKPGQSPKLLIYWASTRESGVPDRFTGSGSGTDFTLAISSVMPEDLAVYYCQQYYNYPWTFGGGTKLEIKGGGGSGGGGSGGGGSGGGGSVQLQESGPGLVKPSQSLSLTCSVTDYSITSGYYWNWIRQFPGNKLEWMGYISYDGSNNYNPSLKNRISITRDTSKNQFFLKLSSVTTEDTATYYCSRGEGFYFDSWGQGTTLTVSSSEPKSSDKTHTCPPCPAPEAAGAPSVFLFPPKPKDTLMISRTPEVTCVVVDVSHEDPEVKFNWYVDGVEVHNAKTKPREEQYNSTYRVVSVLTVLHQDWLNGKEYKCAVSNKALPAPIEKTISKAKGQPREPQVYTLPPSRDELTKNQVSLTCLVKGFYPSDIAVEWESNGQPENNYKTTPPVLDSDGSFFLYSKLTVDKSRWQQGNVFSCSVMHEALHNHYTQKSLSLSPGSGGGGSGGGGSGGGGSPGSQVQLVQSGPEVKKPGSSVKVSCKASGYTFSRSTMHWVRQAPGQGLEWIGYINPSSAYTNYNQKFKDRVTITADKSTSTAYMELSSLRSEDTAVYYCARPQVHYDYNGFPYWGQGTLVTVSSGGGGSGGGGSGGGGSGGGGSDIQMTQSPSTLSASVGDRVTMTCSASSSVSYMNWYQQKPGKAPKRWIYDSSKLASGVPSRFSGSGSGTDYTLTISSLQPDDFATYYCQQWSRNPPTFGGGTKVEIKRSSS

SEQ ID NO: 198 - protein, 753 aa, Artificial Sequence
  Chimeric bispecific anti-CD123 (VHVL) x anti-CD3 (TSC456) scFv-Fc-scFv CD3-binding domain
VQLQESGPGLVKPSQSLSLTCSVTDYSITSGYYWNWIRQFPGNKLEWMGYISYDGSNNYNPSLKNRISITRDTSKNQFFLKLSSVTTEDTATYYCSRGEGFYFDSWGQGTTLTVSSGGGGSGGGGSGGGGSGGGGSDIMMSQSPSSLAVSVGEKFTMTCKSSQSLFFGSTQKNYLAWYQQKPGQSPKLLIYWASTRESGVPDRFTGSGSGTDFTLAISSVMPEDLAVYYCQQYYNYPWTFGGGTKLEIKSSSEPKSSDKTHTCPPCPAPEAAGAPSVFLFPPKPKDTLMISRTPEVTCVVVDVSHEDPEVKFNWYVDGVEVHNAKTKPREEQYNSTYRVVSVLTVLHQDWLNGKEYKCAVSNKALPAPIEKTISKAKGQPREPQVYTLPPSRDELTKNQVSLTCLVKGFYPSDIAVEWESNGQPENNYKTTPPVLDSDGSFFLYSKLTVDKSRWQQGNVFSCSVMHEALHNHYTQKSLSLSPGSGGGGSGGGGSGGGGSPGSQVQLVQSGPEVKKPGSSVKVSCKASGYTFSRSTMHWVRQAPGQGLEWIGYINPSSAYTNYNQKFKDRVTITADKSTSTAYMELSSLRSEDTAVYYCARPQVHYDYNGFPYWGQGTLVTVSSGGGGSGGGGSGGGGSGGGGSDIQMTQSPSTLSASVGDRVTMTCSASSSVSYMNWYQQKPGKAPKRWIYDSSKLASGVPSRFSGSGSGTDYTLTISSLQPDDFATYYCQQWSRNPPTFGGGTKVEIKRSSS

SEQ ID NO: 199 - protein, 8 aa, Artificial Sequence
  Cris7 and DRA222 VH CDR1 (IMGT) CD3-binding domain
GYTFTRST

SEQ ID NO: 200 - protein, 8 aa, Artificial Sequence
  Cris7 and DRA222 VH CDR2 (IMGT) CD3-binding domain
INPSSAYT

SEQ ID NO: 201 - protein, 9 aa, Artificial Sequence
  Cris7 and DRA222 VH CDR3 (IMGT) CD3-binding domain
QQWSRNPPT

SEQ ID NO: 202 - protein, 7 aa, Artificial Sequence
  Cris7 and DRA222 VL CDR1 (IMGT) CD3-binding domain
ASSSVSY

SEQ ID NO: 203 - protein, 3 aa, Artificial Sequence
  Cris7 and DRA222 VL CDR2 (IMGT) CD3-binding domain
DSS

SEQ ID NO: 204 - protein, 9 aa, Artificial Sequence
  Cris7 and DRA222 VL CDR3 (IMGT) CD3-binding domain
QQWSRNPPT

SEQ ID NO: 205 - DNA, 2286 bp, Artificial Sequence
  TSC471 Anti-PSMA X anti-CD3 bispecific molecule
atggaagcaccagcgcagcttctcttcctcctgctactctggctcccagataccaccggtgatatccagatgacccagtctccatccgccatgtctgcatctgtaggagacagagtcaccatcacttgccgggcgagtaagagcattagcaaatatttagcctggtttcagcagaaaccagggaaagttcctaagctccgcatccattctggatctactttgcaatcaggggtcccatctcggttcagtggcagtggatctgggacagaatttactctcaccatcagcagcctgcagcctgaagattttgcaacttattactgtcaacagcatattgaatacccgtggacgttcggccaagggaccaaggtggaaatcaaacgaggtggcggagggtctgggggtggcggatccggaggtggtggctctcaggtccagctggtacagtctggggctgaggtgaagaagcctggggcttcagtgaaggtctcctgcaaggcttctggatacacattcactgactactacatgcactgggtgcgacaggcccctggacaagggcttgagtggatgggatattttaatccttataatgattatactagatacgcacagaagttccagggcagagtcaccatgaccagggacacgtctatcagcacagcctacatggagctgagcagcctgagatctgacgacacggccgtgtattactgtgcaagatcggatggttactacgatgctatggactactggggtcaaggaaccacagtcaccgtctcctcgagtgagcccaaatcttctgacaaaactcacacatgcccaccgtgcccagcacctgaagccgcgggtgcaccgtcagtcttcctcttccccccaaaacccaaggacaccctcatgatctcccggacccctgaggtcacatgcgtggtggtggacgtgagccacgaagaccctgaggtcaagttcaactggtacgtggacggcgtggaggtgcataatgccaagacaaagccgcgggaggagcagtacaacagcacgtaccgtgtggtcagcgtcctcaccgtcctgcaccaggactggctgaatggcaaggaatacaagtgcgcggtctccaacaaagccctcccagcccccatcgagaaaaccatctccaaagccaaagggcagccccgagaaccacaggtgtacaccctgcccccatcccgggatgagctgaccaagaaccaggtcagcctgacctgcctggtcaaaggcttctatccaagcgacatcgccgtggagtgggagagcaatgggcagccggagaacaactacaagaccacgcctcccgtgctggactccgacggctccttcttcctctacagcaagctcaccgtggacaagagcaggtggcagcaggggaacgtcttctcatgctccgtgatgcatgaggctctgcacaaccactacacgcagaagagcctctccctgtctccgggttccggaggtggcggttcgggaggtggcgggtcaggaggtgggggctctccttcacaggtgcagctggtgcagtctggtcctgaggtgaaaaagcctggctccagcgtgaaggtgtcctgcaaggccagcggatacacctttagccggtccaccatgcattgggtgaggcaggctcctggacagggcctggagtggatcggctacatcaaccccagcagcgcttataccaactacaatcagaagtttaaggaccgggtgaccatcaccgccgataagtccaccagcaccgcctacatggagctgtccagcctgaggagcgaggataccgccgtgtactattgcgcccggccccaggtccattacgactacaacggcttcccctattggggccagggaaccctggtgaccgtgtccagcggtggcggtggcagcggcggcggcggctctggcggaggtggcagcggcggagggggctccgacattcagatgacccagtccccctccaccctgtccgctagcgtgggcgatcgggtgaccatgacctgcagcgccagcagctccgtgtcctacatgaactggtaccagcagaagcccggcaaggctcccaagaggtggatttacgactccagcaagctggcctctggtgtccccagcaggttctctggtagcggcagcggcacagactacaccctgaccatctcctccctgcagcccgacgatttcgccacctactattgccagcagtggtcccggaatccccctacctttggcggcggcaccaaggtggagatcaagaggagctaa

SEQ ID NO: 206 - protein, 741 aa, Artificial Sequence
  TSC471 Anti-PSMA X anti-CD3 bispecific molecule
DIQMTQSPSAMSASVGDRVTITCRASKSISKYLAWFQQKPGKVPKLRIHSGSTLQSGVPSRFSGSGSGTEFTLTISSLQPEDFATYYCQQHIEYPWTFGQGTKVEIKRGGGGSGGGGSGGGGSQVQLVQSGAEVKKPGASVKVSCKASGYTFTDYYMHWVRQAPGQGLEWMGYFNPYNDYTRYAQKFQGRVTMTRDTSISTAYMELSSLRSDDTAVYYCARSDGYYDAMDYWGQGTTVTVSSSEPKSSDKTHTCPPCPAPEAAGAPSVFLFPPKPKDTLMISRTPEVTCVVVDVSHEDPEVKFNWYVDGVEVHNAKTKPREEQYNSTYRVVSVLTVLHQDWLNGKEYKCAVSNKALPAPIEKTISKAKGQPREPQVYTLPPSRDELTKNQVSLTCLVKGFYPSDIAVEWESNGQPENNYKTTPPVLDSDGSFFLYSKLTVDKSRWQQGNVFSCSVMHEALHNHYTQKSLSLSPGSGGGGSGGGGSGGGGSPSQVQLVQSGPEVKKPGSSVKVSCKASGYTFSRSTMHWVRQAPGQGLEWIGYINPSSAYTNYNQKFKDRVTITADKSTSTAYMELSSLRSEDTAVYYCARPQVHYDYNGFPYWGQGTLVTVSSGGGGSGGGGSGGGGSGGGGSDIQMTQSPSTLSASVGDRVTMTCSASSSVSYMNWYQQKPGKAPKRWIYDSSKLASGVPSRFSGSGSGTDYTLTISSLQPDDFATYYCQQWSRNPPTFGGGTKVEIKRS

SEQ ID NO: 207 - DNA, 2307 bp, Artificial Sequence
  ROR243 Anti-ROR1 X anti-CD3 bispecific molecule
atggaggctcccgctcagctgctgttcctcctgctgctctggctgcccgacaccacaggcgacatccagatgacccagtccccttcctccctgtccgctagcgtgggcgatagggtgaccatcaactgccaggcctcccagtccattgactccaatctggcctggttccagcagaagcccggacagccccccaagctgctgatttacagggcctccaacctggcttccggcgtgcctgacaggttctccggatccggcagcggcaccgacttcaccctgaccatctcctccctggaggccgaggatgtcgccacctactactgtctgggcggcgtgggcgctgtgagctatcggacctccttcggcggcggcaccaaggtggagatcaagggcggcggcggcagcggcggcggcggcagcggcggcggaggctccggcggcggcggcagcgaggtgcagctggtggaaagcggaggaggcctggtgcagcctggaaggtccctgaggctgtcctgcacagccagcggctccgacatcaacgactaccccatcacctgggtgaggcaggctcctggccagggcctggaatggatcggctttatcaacagcggcggcagcacctggtatgcttcctgggtgaagggccggttcaccattagcagggacgactccaagtccattgcctacctgcagatgaactccctgaagaccgaggacaccgccgtgtactactgcgccaggggctacagcacctattaccgggactttaacatctggggccagggcacactggtcaccgtgtcctcgagtgagcccaaatcttctgacaaaactcacacatgcccaccgtgcccagcacctgaagccgcgggtgcaccgtcagtcttcctcttccccccaaaacccaaggacaccctcatgatctcccggacccctgaggtcacatgcgtggtggtggacgtgagccacgaagaccctgaggtcaagttcaactggtacgtggacggcgtggaggtgcataatgccaagacaaagccgcgggaggagcagtacaacagcacgtaccgtgtggtcagcgtcctcaccgtcctgcaccaggactggctgaatggcaaggaatacaagtgcgcggtctccaacaaagccctcccagcccccatcgagaaaaccatctccaaagccaaagggcagccccgagaaccacaggtgtacaccctgcccccatcccgggatgagctgaccaagaaccaggtcagcctgacctgcctggtcaaaggcttctatccaagcgacatcgccgtggagtgggagagcaatgggcagccggagaacaactacaagaccacgcctcccgtgctggactccgacggctccttcttcctctacagcaagctcaccgtggacaagagcaggtggcagcaggggaacgtcttctcatgctccgtgatgcatgaggctctgcacaaccactacacgcagaagagcctctccctgtctccgggttccggaggagggggttcaggtgggggaggttctggcggcgggggaagcccttcacaggtgcaactggtgcagagtggacccgaggttaaaaaaccagggtcctccgttaaggttagctgcaaagcctctggctacacattttccaggagtacaatgcactgggtgaggcaggctcctggacagggactcgagtggatcgggtatatcaacccatctagcgcctataccaattacaaccaaaagtttaaggaccgagttaccattaccgctgacaaatccaccagtacagcttatatggagctgtcatctcttaggtccgaggacactgctgtttattactgcgctcgtcctcaggttcactatgactataatggttttccctactggggtcagggaaccctggtgactgtctcttctggcggtggaggcagcggtgggggtgggtctggaggcggtggcagtggcggcggaggctctgatattcagatgactcagtctcctagcactctcagcgccagcgtgggggatcgtgtgacaatgacttgctccgctagcagtagtgtgtcttacatgaattggtatcagcagaagcccgggaaagcacctaagcgctggatctatgactcttccaagctggcaagtggtgtcccctcacggttctctggctcaggttctggtactgactatactttgactatctcctccctccagcccgatgatttcgctacctattattgtcagcagtggagccgtaacccacccactttcggaggcggtaccaaagtggagatcaagaggtcatga

SEQ ID NO: 208 - protein, 748 aa, Artificial Sequence
  ROR243 Anti-ROR1 X anti-CD3 bispecific molecule
DIQMTQSPSSLSASVGDRVTINCQASQSIDSNLAWFQQKPGQPPKLLIYRASNLASGVPDRFSGSGSGTDFTLTISSLEAEDVATYYCLGGVGAVSYRTSFGGGTKVEIKGGGGSGGGGSGGGGSGGGGSEVQLVESGGGLVQPGRSLRLSCTASGSDINDYPITWVRQAPGQGLEWIGFINSGGSTWYASWVKGRFTISRDDSKSIAYLQMNSLKTEDTAVYYCARGYSTYYRDFNIWGQGTLVTVSSSEPKSSDKTHTCPPCPAPEAAGAPSVFLFPPKPKDTLMISRTPEVTCVVVDVSHEDPEVKFNWYVDGVEVHNAKTKPREEQYNSTYRVVSVLTVLHQDWLNGKEYKCAVSNKALPAPIEKTISKAKGQPREPQVYTLPPSRDELTKNQVSLTCLVKGFYPSDIAVEWESNGQPENNYKTTPPVLDSDGSFFLYSKLTVDKSRWQQGNVFSCSVMHEALHNHYTQKSLSLSPGSGGGGSGGGGSGGGGSPSQVQLVQSGPEVKKPGSSVKVSCKASGYTFSRSTMHWVRQAPGQGLEWIGYINPSSAYTNYNQKFKDRVTITADKSTSTAYMELSSLRSEDTAVYYCARPQVHYDYNGFPYWGQGTLVTVSSGGGGSGGGGSGGGGSGGGGSDIQMTQSPSTLSASVGDRVTMTCSASSSVSYMNWYQQKPGKAPKRWIYDSSKLASGVPSRFSGSGSGTDYTLTISSLQPDDFATYYCQQWSRNPPTFGGGTKVEIKRS

SEQ ID NO: 209 - DNA, 2289 bp, Artificial Sequence
  TSC266 Anti-PSMA X anti-CD3 bispecific molecule
atggaagcaccagcgcagcttctcttcctcctgctactctggctcccagataccaccggtgatatccagatgacccagtctccatccgccatgtctgcatctgtaggagacagagtcaccatcacttgccgggcgagtaagagcattagcaaatatttagcctggtttcagcagaaaccagggaaagttcctaagctccgcatccattctggatctactttgcaatcaggggtcccatctcggttcagtggcagtggatctgggacagaatttactctcaccatcagcagcctgcagcctgaagattttgcaacttattactgtcaacagcatattgaatacccgtggacgttcggccaagggaccaaggtggaaatcaaacgaggtggcggagggtctgggggtggcggatccggaggtggtggctctcaggtccagctggtacagtctggggctgaggtgaagaagcctggggcttcagtgaaggtctcctgcaaggcttctggatacacattcactgactactacatgcactgggtgcgacaggcccctggacaagggcttgagtggatgggatattttaatccttataatgattatactagatacgcacagaagttccagggcagagtcaccatgaccagggacacgtctatcagcacagcctacatggagctgagcagcctgagatctgacgacacggccgtgtattactgtgcaagatcggatggttactacgatgctatggactactggggtcaaggaaccacagtcaccgtctcctcgagtgagcccaaatcttctgacaaaactcacacatgcccaccgtgcccagcacctgaagccgcgggtgcaccgtcagtcttcctcttccccccaaaacccaaggacaccctcatgatctcccggacccctgaggtcacatgcgtggtggtggacgtgagccacgaagaccctgaggtcaagttcaactggtacgtggacggcgtggaggtgcataatgccaagacaaagccgcgggaggagcagtacaacagcacgtaccgtgtggtcagcgtcctcaccgtcctgcaccaggactggctgaatggcaaggcgtacgcgtgcgcggtctccaacaaagccctcccagcccccatcgagaaaaccatctccaaagccaaagggcagccccgagaaccacaggtgtacaccctgcccccatcccgggatgagctgaccaagaaccaggtcagcctgacctgcctggtcaaaggcttctatccaagcgacatcgccgtggagtgggagagcaatgggcagccggagaacaactacaagaccacgcctcccgtgctggactccgacggctccttcttcctctacagcaagctcaccgtggacaagagcaggtggcagcaggggaacgtcttctcatgctccgtgatgcatgaggctctgcacaaccactacacgcagaagagcctctccctgtctccgggtcagaggcacaacaattcttccctgaatacaggaactcagatggcaggtcattctccgaattctcaggtccagctggtggagtctgggggcggagtggtgcagcctgggcggtcactgaggctgtcctgcaaggcttctggctacacctttactagatctacgatgcactgggtaaggcaggcccctggacaaggtctggaatggattggatacattaatcctagcagtgcttatactaattacaatcagaaattcaaggacaggttcacaatcagcgcagacaaatccaagagcacagccttcctgcagatggacagcctgaggcccgaggacaccggcgtctatttctgtgcacggccccaagtccactatgattacaacgggtttccttactggggccaagggactcccgtcactgtctctagcggtggcggagggtctgggggtggcggatccggaggtggtggctctgcacaagacatccagatgacccagtctccaagcagcctgtctgcaagcgtgggggacagggtcaccatgacctgcagtgccagctcaagtgtaagttacatgaactggtaccagcagaagccgggcaaggcccccaaaagatggatttatgactcatccaaactggcttctggagtccctgctcgcttcagtggcagtgggtctgggaccgactataccctcacaatcagcagcctgcagcccgaagatttcgccacttattactgccagcagtggagtcgtaacccacccacgttcggaggggggaccaagctacaaattacatcctccagctaa

SEQ ID NO: 210 - protein, 742 aa, Artificial Sequence
  TSC266 Anti-PSMA X anti-CD3 bispecific molecule
DIQMTQSPSAMSASVGDRVTITCRASKSISKYLAWFQQKPGKVPKLRIHSGSTLQSGVPSRFSGSGSGTEFTLTISSLQPEDFATYYCQQHIEYPWTFGQGTKVEIKRGGGGSGGGGSGGGGSQVQLVQSGAEVKKPGASVKVSCKASGYTFTDYYMHWVRQAPGQGLEWMGYFNPYNDYTRYAQKFQGRVTMTRDTSISTAYMELSSLRSDDTAVYYCARSDGYYDAMDYWGQGTTVTVSSSEPKSSDKTHTCPPCPAPEAAGAPSVFLFPPKPKDTLMISRTPEVTCVVVDVSHEDPEVKFNWYVDGVEVHNAKTKPREEQYNSTYRVVSVLTVLHQDWLNGKAYACAVSNKALPAPIEKTISKAKGQPREPQVYTLPPSRDELTKNQVSLTCLVKGFYPSDIAVEWESNGQPENNYKTTPPVLDSDGSFFLYSKLTVDKSRWQQGNVFSCSVMHEALHNHYTQKSLSLSPGQRHNNSSLNTGTQMAGHSPNSQVQLVESGGGVVQPGRSLRLSCKASGYTFTRSTMHWVRQAPGQGLEWIGYINPSSAYTNYNQKFKDRFTISADKSKSTAFLQMDSLRPEDTGVYFCARPQVHYDYNGFPYWGQGTPVTVSSGGGGSGGGGSGGGGSAQDIQMTQSPSSLSASVGDRVTMTCSASSSVSYMNWYQQKPGKAPKRWIYDSSKLASGVPARFSGSGSGTDYTLTISSLQPEDFATYYCQQWSRNPPTFGGGTKLQITSSS

SEQ ID NO: 211 - DNA, 2301 bp, Artificial Sequence
  ROR206 Anti-ROR1 X anti-CD3 bispecific molecule
atggaagcaccagcgcagcttctcttcctcctgctactctggctcccagataccaccggtgacatccagatgacccagtccccctcctccctgtccgcctccgtgggcgaccgggtgaccatcaactgccaggcctcccagtccatcgactccaacctggcctggttccagcagaagcccggcaagccccccaagctgctgatctaccgggcctccaacctggcctccggcgtgccctcccggttctccggctccggctccggcaccgacttcaccctgaccatctcctccctgcagcccgaggacgtggccacctactactgcctgggcggcgtgggcgccgtgtcctaccggacctccttcggcggcggcaccaaggtggagatcaagggtggaggcggttcaggcggaggtggatccggcggtggcggctccggtggcggcggatctgaggtgcagctggtggagtccggcggcggcctggtgcagcccggccggtccctgcggctgtcctgcaccgcctccggctccgacatcaacgactaccccatcacctgggtgcggcaggcccccggcaagggcctggagtggatcggcttcatcaactccggcggctccacctggtacgcctcctgggtgaagggccggttcaccatctcccgggacgactccaagtccatcgcctacctgcagatgaactccctgaagaccgaggacaccgccgtgtactattgcgcccggggctactccacctactaccgggacttcaacatctggggccagggcaccctggtgaccgtgtcctcgagtgagcccaaatcttctgacaaaactcacacatgcccaccgtgcccagcacctgaagccgcgggtgcaccgtcagtcttcctcttccccccaaaacccaaggacaccctcatgatctcccggacccctgaggtcacatgcgtggtggtggacgtgagccacgaagaccctgaggtcaagttcaactggtacgtggacggcgtggaggtgcataatgccaagacaaagccgcgggaggagcagtacaacagcacgtaccgtgtggtcagcgtcctcaccgtcctgcaccaggactggctgaatggcaaggaatacaagtgcgcggtctccaacaaagccctcccagcccccatcgagaaaaccatctccaaagccaaagggcagccccgagaaccacaggtgtacaccctgcccccatcccgggatgagctgaccaagaaccaggtcagcctgacctgcctggtcaaaggcttctatccaagcgacatcgccgtggagtgggagagcaatgggcagccggagaacaactacaagaccacgcctcccgtgctggactccgacggctccttcttcctctacagcaagctcaccgtggacaagagcaggtggcagcaggggaacgtcttctcatgctccgtgatgcatgaggctctgcacaaccactacacgcagaagagcctctccctgtctccgggttctggtggaggcggttcaggcggaggtggctccggcggtggcggatcgccgggctctcaggtccagctggtggagtctgggggcggagtggtgcagcctgggcggtcactgaggctgtcctgcaaggcttctggctacacctttactagatctacgatgcactgggtaaggcaggcccctggacaaggtctggaatggattggatacattaatcctagcagtgcttatactaattacaatcagaaattcaaggacaggttcacaatcagcgcagacaaatccaagagcacagccttcctgcagatggacagcctgaggcccgaggacaccggcgtctatttctgtgcacggccccaagtccactatgattacaacgggtttccttactggggccaagggactcccgtcactgtctctagcggtggcggagggtctgggggtggcggatccggaggtggtggctctgcacaagacatccagatgacccagtctccaagcagcctgtctgcaagcgtgggggacagggtcaccatgacctgcagtgccagctcaagtgtaagttacatgaactggtaccagcagaagccgggcaaggcccccaaaagatggatttatgactcatccaaactggcttctggagtccctgctcgcttcagtggcagtgggtctgggaccgactataccctcacaatcagcagcctgcagcccgaagatttcgccacttattactgccagcagtggagtcgtaacccacccacgttcggaggggggaccaagctacaaattacatcctccagc

SEQ ID NO: 212 - protein, 767 aa, Artificial Sequence
  ROR206 Anti-ROR1 X anti-CD3 bispecific molecule
MEAPAQLLFLLLLWLPDTTGDIQMTQSPSSLSASVGDRVTINCQASQSIDSNLAWFQQKPGKPPKLLIYRASNLASGVPSRFSGSGSGTDFTLTISSLQPEDVATYYCLGGVGAVSYRTSFGGGTKVEIKGGGGSGGGGSGGGGSGGGGSEVQLVESGGGLVQPGRSLRLSCTASGSDINDYPITWVRQAPGKGLEWIGFINSGGSTWYASWVKGRFTISRDDSKSIAYLQMNSLKTEDTAVYYCARGYSTYYRDFNIWGQGTLVTVSSSEPKSSDKTHTCPPCPAPEAAGAPSVFLFPPKPKDTLMISRTPEVTCVVVDVSHEDPEVKFNWYVDGVEVHNAKTKPREEQYNSTYRVVSVLTVLHQDWLNGKEYKCAVSNKALPAPIEKTISKAKGQPREPQVYTLPPSRDELTKNQVSLTCLVKGFYPSDIAVEWESNGQPENNYKTTPPVLDSDGSFFLYSKLTVDKSRWQQGNVFSCSVMHEALHNHYTQKSLSLSPGSGGGGSGGGGSGGGGSPGSQVQLVESGGGVVQPGRSLRLSCKASGYTFTRSTMHWVRQAPGQGLEWIGYINPSSAYTNYNQKFKDRFTISADKSKSTAFLQMDSLRPEDTGVYFCARPQVHYDYNGFPYWGQGTPVTVSSGGGGSGGGGSGGGGSAQDIQMTQSPSSLSASVGDRVTMTCSASSSVSYMNWYQQKPGKAPKRWIYDSSKLASGVPARFSGSGSGTDYTLTISSLQPEDFATYYCQQWSRNPPTFGGGTKLQITSSS

SEQ ID NO: 213 - DNA, 2313 bp, Artificial Sequence
  ROR207 Anti-ROR1 X anti-CD3 bispecific molecule
atggaagcaccagcgcagcttctcttcctcctgctactctggctcccagataccaccggtgacatccagatgacccagtccccctcctccctgtccgcctccgtgggcgaccgggtgaccatcaactgccaggcctcccagtccatcgactccaacctggcctggttccagcagaagcccggcaagccccccaagctgctgatctaccgggcctccaacctggcctccggcgtgccctcccggttctccggctccggctccggcaccgacttcaccctgaccatctcctccctgcagcccgaggacgtggccacctactactgcctgggcggcgtgggcgccgtgtcctaccggacctccttcggcggcggcaccaaggtggagatcaagggtggaggcggttcaggcggaggtggatccggcggtggcggctccggtggcggcggatctgaggtgcagctggtggagtccggcggcggcctggtgcagcccggccggtccctgcggctgtcctgcaccgcctccggctccgacatcaacgactaccccatcacctgggtgcggcaggcccccggcaagggcctggagtggatcggcttcatcaactccggcggctccacctggtacgcctcctgggtgaagggccggttcaccatctcccgggacgactccaagtccatcgcctacctgcagatgaactccctgaagaccgaggacaccgccgtgtactattgcgcccggggctactccacctactaccgggacttcaacatctggggccagggcaccctggtgaccgtgtcctcgagtgagcccaaatcttctgacaaaactcacacatgcccaccgtgcccagcacctgaagccgcgggtgcaccgtcagtcttcctcttccccccaaaacccaaggacaccctcatgatctcccggacccctgaggtcacatgcgtggtggtggacgtgagccacgaagaccctgaggtcaagttcaactggtacgtggacggcgtggaggtgcataatgccaagacaaagccgcgggaggagcagtacaacagcacgtaccgtgtggtcagcgtcctcaccgtcctgcaccaggactggctgaatggcaaggaatacaagtgcgcggtctccaacaaagccctcccagcccccatcgagaaaaccatctccaaagccaaagggcagccccgagaaccacaggtgtacaccctgcccccatcccgggatgagctgaccaagaaccaggtcagcctgacctgcctggtcaaaggcttctatccaagcgacatcgccgtggagtgggagagcaatgggcagccggagaacaactacaagaccacgcctcccgtgctggactccgacggctccttcttcctctacagcaagctcaccgtggacaagagcaggtggcagcaggggaacgtcttctcatgctccgtgatgcatgaggctctgcacaaccactacacgcagaagagcctctccctgtctccgggttctggtggaggcggttcaggcggaggtggctccggcggtggcggatcgccgggctctcaggtccagctggtgcaatctgggcctgaggtgaagaagcctgggtcctcggtgaaggtctcctgcaaggcttctggatataccttcagcagatctacgatgcactgggtgcgacaggcccctggacaagggcttgagtggataggatacattaatcctagcagtgcttatactaattacaatcagaaattcaaggacagagtcacgattaccgcggacaaatccacgagcacagcctacatggagctgagcagcctgagatctgaggacacggccgtgtattactgtgcgagaccccaagtccactatgattacaacgggtttccttactggggccaaggaaccctggtcaccgtctcctcaggtggaggcggttcaggcggaggtggatccggcggtggcggatcgggtggcggcggatctgacatccagatgacccagtctccttccaccctgtctgcatctgtaggagacagagtcaccatgacttgcagtgccagctcaagtgtaagttacatgaactggtatcagcagaaaccagggaaagcccctaagagatggatttatgactcatccaaactggcttctggggtcccatcaaggttcagcggcagtggatctgggacagattatactctcaccatcagcagcctgcagcctgatgattttgcaacttattactgccaacagtggagtcgtaacccacccactttcggcggagggaccaaggtggagatcaaacggtcctccagc

SEQ ID NO: 214 - protein, 771 aa, Artificial Sequence
  ROR207 Anti-ROR1 X anti-CD3 bispecific molecule
MEAPAQLLFLLLLWLPDTTGDIQMTQSPSSLSASVGDRVTINCQASQSIDSNLAWFQQKPGKPPKLLIYRASNLASGVPSRFSGSGSGTDFTLTISSLQPEDVATYYCLGGVGAVSYRTSFGGGTKVEIKGGGGSGGGGSGGGGSGGGGSEVQLVESGGGLVQPGRSLRLSCTASGSDINDYPITWVRQAPGKGLEWIGFINSGGSTWYASWVKGRFTISRDDSKSIAYLQMNSLKTEDTAVYYCARGYSTYYRDFNIWGQGTLVTVSSSEPKSSDKTHTCPPCPAPEAAGAPSVFLFPPKPKDTLMISRTPEVTCVVVDVSHEDPEVKFNWYVDGVEVHNAKTKPREEQYNSTYRVVSVLTVLHQDWLNGKEYKCAVSNKALPAPIEKTISKAKGQPREPQVYTLPPSRDELTKNQVSLTCLVKGFYPSDIAVEWESNGQPENNYKTTPPVLDSDGSFFLYSKLTVDKSRWQQGNVFSCSVMHEALHNHYTQKSLSLSPGSGGGGSGGGGSGGGGSPGSQVQLVQSGPEVKKPGSSVKVSCKASGYTFSRSTMHWVRQAPGQGLEWIGYINPSSAYTNYNQKFKDRVTITADKSTSTAYMELSSLRSEDTAVYYCARPQVHYDYNGFPYWGQGTLVTVSSGGGGSGGGGSGGGGSGGGGSDIQMTQSPSTLSASVGDRVTMTCSASSSVSYMNWYQQKPGKAPKRWIYDSSKLASGVPSRFSGSGSGTDYTLTISSLQPDDFATYYCQQWSRNPPTFGGGTKVEIKRSSS

SEQ ID NO: 215 - DNA, 2301 bp, Artificial Sequence
  ROR208 Anti-ROR1 X anti-CD3 bispecific molecule
atggaagcaccagcgcagcttctcttcctcctgctactctggctcccagataccaccggtgacatccagatgacccagtccccctcctccctgtccgcctccgtgggcgaccgggtgaccatcaactgccaggcctcccagtccatcgactccaacctggcctggttccagcagaagcccggccagccccccaagctgctgatctaccgggcctccaacctggcctccggcgtgcccgaccggttctccggctccggctccggcaccgacttcaccctgaccatctcctccctggaggccgaggacgtggccacctactactgcctgggcggcgtgggcgccgtgtcctaccggacctccttcggcggcggcaccaaggtggagatcaagggtggaggcggttcaggcggaggtggatccggcggtggcggctccggtggcggcggatctgaggtgcagctggtggagtccggcggcggcctggtgcagcccggccggtccctgcggctgtcctgcaccgcctccggctccgacatcaacgactaccccatcacctgggtgcggcaggcccccggccagggcctggagtggatcggcttcatcaactccggcggctccacctggtacgcctcctgggtgaagggccggttcaccatctcccgggacgactccaagtccatcgcctacctgcagatgaactccctgaagaccgaggacaccgccgtgtactattgcgcccggggctactccacctactaccgggacttcaacatctggggccagggcaccctggtgaccgtgtcctcgagtgagcccaaatcttctgacaaaactcacacatgcccaccgtgcccagcacctgaagccgcgggtgcaccgtcagtcttcctcttccccccaaaacccaaggacaccctcatgatctcccggacccctgaggtcacatgcgtggtggtggacgtgagccacgaagaccctgaggtcaagttcaactggtacgtggacggcgtggaggtgcataatgccaagacaaagccgcgggaggagcagtacaacagcacgtaccgtgtggtcagcgtcctcaccgtcctgcaccaggactggctgaatggcaaggaatacaagtgcgcggtctccaacaaagccctcccagcccccatcgagaaaaccatctccaaagccaaagggcagccccgagaaccacaggtgtacaccctgcccccatcccgggatgagctgaccaagaaccaggtcagcctgacctgcctggtcaaaggcttctatccaagcgacatcgccgtggagtgggagagcaatgggcagccggagaacaactacaagaccacgcctcccgtgctggactccgacggctccttcttcctctacagcaagctcaccgtggacaagagcaggtggcagcaggggaacgtcttctcatgctccgtgatgcatgaggctctgcacaaccactacacgcagaagagcctctccctgtctccgggttctggtggaggcggttcaggcggaggtggctccggcggtggcggatcgccgggctctcaggtccagctggtggagtctgggggcggagtggtgcagcctgggcggtcactgaggctgtcctgcaaggcttctggctacacctttactagatctacgatgcactgggtaaggcaggcccctggacaaggtctggaatggattggatacattaatcctagcagtgcttatactaattacaatcagaaattcaaggacaggttcacaatcagcgcagacaaatccaagagcacagccttcctgcagatggacagcctgaggcccgaggacaccggcgtctatttctgtgcacggccccaagtccactatgattacaacgggtttccttactggggccaagggactcccgtcactgtctctagcggtggcggagggtctgggggtggcggatccggaggtggtggctctgcacaagacatccagatgacccagtctccaagcagcctgtctgcaagcgtgggggacagggtcaccatgacctgcagtgccagctcaagtgtaagttacatgaactggtaccagcagaagccgggcaaggcccccaaaagatggatttatgactcatccaaactggcttctggagtccctgctcgcttcagtggcagtgggtctgggaccgactataccctcacaatcagcagcctgcagcccgaagatttcgccacttattactgccagcagtggagtcgtaacccacccacgttcggaggggggaccaagctacaaattacatcctccagc

SEQ ID NO: 216 - protein, 767 aa, Artificial Sequence
  ROR208 Anti-ROR1 X anti-CD3 bispecific molecule
MEAPAQLLFLLLLWLPDTTGDIQMTQSPSSLSASVGDRVTINCQASQSIDSNLAWFQQKPGQPPKLLIYRASNLASGVPDRFSGSGSGTDFTLTISSLEAEDVATYYCLGGVGAVSYRTSFGGGTKVEIKGGGGSGGGGSGGGGSGGGGSEVQLVESGGGLVQPGRSLRLSCTASGSDINDYPITWVRQAPGQGLEWIGFINSGGSTWYASWVKGRFTISRDDSKSIAYLQMNSLKTEDTAVYYCARGYSTYYRDFNIWGQGTLVTVSSSEPKSSDKTHTCPPCPAPEAAGAPSVFLFPPKPKDTLMISRTPEVTCVVVDVSHEDPEVKFNWYVDGVEVHNAKTKPREEQYNSTYRVVSVLTVLHQDWLNGKEYKCAVSNKALPAPIEKTISKAKGQPREPQVYTLPPSRDELTKNQVSLTCLVKGFYPSDIAVEWESNGQPENNYKTTPPVLDSDGSFFLYSKLTVDKSRWQQGNVFSCSVMHEALHNHYTQKSLSLSPGSGGGGSGGGGSGGGGSPGSQVQLVESGGGVVQPGRSLRLSCKASGYTFTRSTMHWVRQAPGQGLEWIGYINPSSAYTNYNQKFKDRFTISADKSKSTAFLQMDSLRPEDTGVYFCARPQVHYDYNGFPYWGQGTPVTVSSGGGGSGGGGSGGGGSAQDIQMTQSPSSLSASVGDRVTMTCSASSSVSYMNWYQQKPGKAPKRWIYDSSKLASGVPARFSGSGSGTDYTLTISSLQPEDFATYYCQQWSRNPPTFGGGTKLQITSSS

SEQ ID NO: 217 - DNA, 2313 bp, Artificial Sequence
  ROR209 Anti-ROR1 X anti-CD3 bispecific molecule
atggaagcaccagcgcagcttctcttcctcctgctactctggctcccagataccaccggtgacatccagatgacccagtccccctcctccctgtccgcctccgtgggcgaccgggtgaccatcaactgccaggcctcccagtccatcgactccaacctggcctggttccagcagaagcccggccagccccccaagctgctgatctaccgggcctccaacctggcctccggcgtgcccgaccggttctccggctccggctccggcaccgacttcaccctgaccatctcctccctggaggccgaggacgtggccacctactactgcctgggcggcgtgggcgccgtgtcctaccggacctccttcggcggcggcaccaaggtggagatcaagggtggaggcggttcaggcggaggtggatccggcggtggcggctccggtggcggcggatctgaggtgcagctggtggagtccggcggcggcctggtgcagcccggccggtccctgcggctgtcctgcaccgcctccggctccgacatcaacgactaccccatcacctgggtgcggcaggcccccggccagggcctggagtggatcggcttcatcaactccggcggctccacctggtacgcctcctgggtgaagggccggttcaccatctcccgggacgactccaagtccatcgcctacctgcagatgaactccctgaagaccgaggacaccgccgtgtactattgcgcccggggctactccacctactaccgggacttcaacatctggggccagggcaccctggtgaccgtgtcctcgagtgagcccaaatcttctgacaaaactcacacatgcccaccgtgcccagcacctgaagccgcgggtgcaccgtcagtcttcctcttccccccaaaacccaaggacaccctcatgatctcccggacccctgaggtcacatgcgtggtggtggacgtgagccacgaagaccctgaggtcaagttcaactggtacgtggacggcgtggaggtgcataatgccaagacaaagccgcgggaggagcagtacaacagcacgtaccgtgtggtcagcgtcctcaccgtcctgcaccaggactggctgaatggcaaggaatacaagtgcgcggtctccaacaaagccctcccagcccccatcgagaaaaccatctccaaagccaaagggcagccccgagaaccacaggtgtacaccctgcccccatcccgggatgagctgaccaagaaccaggtcagcctgacctgcctggtcaaaggcttctatccaagcgacatcgccgtggagtgggagagcaatgggcagccggagaacaactacaagaccacgcctcccgtgctggactccgacggctccttcttcctctacagcaagctcaccgtggacaagagcaggtggcagcaggggaacgtcttctcatgctccgtgatgcatgaggctctgcacaaccactacacgcagaagagcctctccctgtctccgggttctggtggaggcggttcaggcggaggtggctccggcggtggcggatcgccgggctctcaggtccagctggtgcaatctgggcctgaggtgaagaagcctgggtcctcggtgaaggtctcctgcaaggcttctggatataccttcagcagatctacgatgcactgggtgcgacaggcccctggacaagggcttgagtggataggatacattaatcctagcagtgcttatactaattacaatcagaaattcaaggacagagtcacgattaccgcggacaaatccacgagcacagcctacatggagctgagcagcctgagatctgaggacacggccgtgtattactgtgcgagaccccaagtccactatgattacaacgggtttccttactggggccaaggaaccctggtcaccgtctcctcaggtggaggcggttcaggcggaggtggatccggcggtggcggatcgggtggcggcggatctgacatccagatgacccagtctccttccaccctgtctgcatctgtaggagacagagtcaccatgacttgcagtgccagctcaagtgtaagttacatgaactggtatcagcagaaaccagggaaagcccctaagagatggatttatgactcatccaaactggcttctggggtcccatcaaggttcagcggcagtggatctgggacagattatactctcaccatcagcagcctgcagcctgatgattttgcaacttattactgccaacagtggagtcgtaacccacccactttcggcggagggaccaaggtggagatcaaacggtcctccagc

SEQ ID NO: 218 - protein, 771 aa, Artificial Sequence
  ROR209 Anti-ROR1 X anti-CD3 bispecific molecule
MEAPAQLLFLLLLWLPDTTGDIQMTQSPSSLSASVGDRVTINCQASQSIDSNLAWFQQKPGQPPKLLIYRASNLASGVPDRFSGSGSGTDFTLTISSLEAEDVATYYCLGGVGAVSYRTSFGGGTKVEIKGGGGSGGGGSGGGGSGGGGSEVQLVESGGGLVQPGRSLRLSCTASGSDINDYPITWVRQAPGQGLEWIGFINSGGSTWYASWVKGRFTISRDDSKSIAYLQMNSLKTEDTAVYYCARGYSTYYRDFNIWGQGTLVTVSSSEPKSSDKTHTCPPCPAPEAAGAPSVFLFPPKPKDTLMISRTPEVTCVVVDVSHEDPEVKFNWYVDGVEVHNAKTKPREEQYNSTYRVVSVLTVLHQDWLNGKEYKCAVSNKALPAPIEKTISKAKGQPREPQVYTLPPSRDELTKNQVSLTCLVKGFYPSDIAVEWESNGQPENNYKTTPPVLDSDGSFFLYSKLTVDKSRWQQGNVFSCSVMHEALHNHYTQKSLSLSPGSGGGGSGGGGSGGGGSPGSQVQLVQSGPEVKKPGSSVKVSCKASGYTFSRSTMHWVRQAPGQGLEWIGYINPSSAYTNYNQKFKDRVTITADKSTSTAYMELSSLRSEDTAVYYCARPQVHYDYNGFPYWGQGTLVTVSSGGGGSGGGGSGGGGSGGGGSDIQMTQSPSTLSASVGDRVTMTCSASSSVSYMNWYQQKPGKAPKRWIYDSSKLASGVPSRFSGSGSGTDYTLTISSLQPDDFATYYCQQWSRNPPTFGGGTKVEIKRSSS

SEQ ID NO: 219 - DNA, 2313 bp, Artificial Sequence
  ROR231 Anti-ROR1 X anti-CD3 bispecific molecule
atggaggcacccgcccagctgctgttcttgttgctgctgtggctccctgataccaccggagacatccagatgacccaatccccttctagtctctccgctagcgtcggagaccgcgtgaccatcaattgtcaagcatctcagagtattgacagcaatctcgcctggtttcagcagaagccaggaaagccacccaagctcctgatttatagggctagcaacctggcttctggtgtccctagtaggttcagcggctctgggagtggcacagacttcaccctgaccattagtagtctgcagcccgaagatgtcgctacctattactgcctcggaggagtgggtgccgtttcttatcgcacctcatttggaggtggcaccaaagtggagatcaaaggtggtggcggctccgggggtggcgggtcaggggggggagggtctggaggcggcggatcagaagttcagctggtggaatctggaggaggtctggtgcagccaggcaggtccctccggctgagctgcactgcatccggctctgacattaatgactaccctatcacctgggtgaggcaggcccccggtaaaggcctggagtggatcgggttcatcaattctggtggatctacttggtacgcaagctgggtgaaaggacgcttcacaattagtagagacgactctaagtctatcgcatatctgcagatgaatagcttgaagacagaggacaccgccgtgtactattgtgcaagaggatactccacttactaccgcgatttcaatatctggggccagggaaccctggtgacagtgtcctcgagtgagcccaaatcttctgacaaaactcacacatgcccaccgtgcccagcacctgaagccgcgggtgcaccgtcagtcttcctcttccccccaaaacccaaggacaccctcatgatctcccggacccctgaggtcacatgcgtggtggtggacgtgagccacgaagaccctgaggtcaagttcaactggtacgtggacggcgtggaggtgcataatgccaagacaaagccgcgggaggagcagtacaacagcacgtaccgtgtggtcagcgtcctcaccgtcctgcaccaggactggctgaatggcaaggaatacaagtgcgcggtctccaacaaagccctcccagcccccatcgagaaaaccatctccaaagccaaagggcagccccgagaaccacaggtgtacaccctgcccccatcccgggatgagctgaccaagaaccaggtcagcctgacctgcctggtcaaaggcttctatccaagcgacatcgccgtggagtgggagagcaatgggcagccggagaacaactacaagaccacgcctcccgtgctggactccgacggctccttcttcctctacagcaagctcaccgtggacaagagcaggtggcagcaggggaacgtcttctcatgctccgtgatgcatgaggctctgcacaaccactacacgcagaagagcctctccctgtctccgggttccggaggcggcggctccggcggcggcggcagcggcggcggcggcagccccggatcccaggtgcagctggtgcagtctggtcctgaggtgaaaaagcctggctccagcgtgaaggtgtcctgcaaggccagcggatacacctttagccggtccaccatgcattgggtgaggcaggctcctggacagggcctggagtggatcggctacatcaaccccagcagcgcttataccaactacaatcagaagtttaaggaccgggtgaccatcaccgccgataagtccaccagcaccgcctacatggagctgtccagcctgaggagcgaggataccgccgtgtactattgcgcccggccccaggtccattacgactacaacggcttcccctattggggccagggaaccctggtgaccgtgtccagcggaggcggcggcagcggcggcggcggcagcggcggaggaggcagcggcggaggaggctccgacattcagatgacccagtccccctccaccctgtccgctagcgtgggcgatcgggtgaccatgacctgcagcgccagcagctccgtgtcctacatgaactggtaccagcagaagcccggcaaggctcccaagaggtggatttacgactccagcaagctggcctctggtgtccccagcaggttctctggtagcggcagcggcacagactacaccctgaccatctcctccctgcagcccgacgatttcgccacctactattgccagcagtggtcccggaatccccctacctttggcggcggcaccaaggtggagatcaagaggagctccagc

SEQ ID NO: 220 - protein, 771 aa, Artificial Sequence; identical to SEQ ID NO: 214
  ROR231 Anti-ROR1 X anti-CD3 bispecific molecule

SEQ ID NO: 221 - DNA, 2313 bp, Artificial Sequence
  ROR233 Anti-ROR1 X anti-CD3 bispecific molecule
atggaggctcccgctcagctgctgttcctcctgctgctctggctgcccgacaccacaggcgacatccagatgacccagtccccttcctccctgtccgctagcgtgggcgatagggtgaccatcaactgccaggcctcccagtccattgactccaatctggcctggttccagcagaagcccggacagccccccaagctgctgatttacagggcctccaacctggcttccggcgtgcctgacaggttctccggatccggcagcggcaccgacttcaccctgaccatctcctccctggaggccgaggatgtcgccacctactactgtctgggcggcgtgggcgctgtgagctatcggacctccttcggcggcggcaccaaggtggagatcaagggcggcggcggcagcggcggcggcggcagcggcggcggaggctccggcggcggcggcagcgaggtgcagctggtggaaagcggaggaggcctggtgcagcctggaaggtccctgaggctgtcctgcacagccagcggctccgacatcaacgactaccccatcacctgggtgaggcaggctcctggccagggcctggaatggatcggctttatcaacagcggcggcagcacctggtatgcttcctgggtgaagggccggttcaccattagcagggacgactccaagtccattgcctacctgcagatgaactccctgaagaccgaggacaccgccgtgtactactgcgccaggggctacagcacctattaccgggactttaacatctggggccagggcacactggtcaccgtgtcctcgagtgagcccaaatcttctgacaaaactcacacatgcccaccgtgcccagcacctgaagccgcgggtgcaccgtcagtcttcctcttccccccaaaacccaaggacaccctcatgatctcccggacccctgaggtcacatgcgtggtggtggacgtgagccacgaagaccctgaggtcaagttcaactggtacgtggacggcgtggaggtgcataatgccaagacaaagccgcgggaggagcagtacaacagcacgtaccgtgtggtcagcgtcctcaccgtcctgcaccaggactggctgaatggcaaggaatacaagtgcgcggtctccaacaaagccctcccagcccccatcgagaaaaccatctccaaagccaaagggcagccccgagaaccacaggtgtacaccctgcccccatcccgggatgagctgaccaagaaccaggtcagcctgacctgcctggtcaaaggcttctatccaagcgacatcgccgtggagtgggagagcaatgggcagccggagaacaactacaagaccacgcctcccgtgctggactccgacggctccttcttcctctacagcaagctcaccgtggacaagagcaggtggcagcaggggaacgtcttctcatgctccgtgatgcatgaggctctgcacaaccactacacgcagaagagcctctccctgtctccgggttccggaggcggcggctccggcggcggcggcagcggcggcggcggcagccccggatcccaggtgcagctggtgcagtctggtcctgaggtgaaaaagcctggctccagcgtgaaggtgtcctgcaaggccagcggatacacctttagccggtccaccatgcattgggtgaggcaggctcctggacagggcctggagtggatcggctacatcaaccccagcagcgcttataccaactacaatcagaagtttaaggaccgggtgaccatcaccgccgataagtccaccagcaccgcctacatggagctgtccagcctgaggagcgaggataccgccgtgtactattgcgcccggccccaggtccattacgactacaacggcttcccctattggggccagggaaccctggtgaccgtgtccagcggaggcggcggcagcggcggcggcggcagcggcggaggaggcagcggcggaggaggctccgacattcagatgacccagtccccctccaccctgtccgctagcgtgggcgatcgggtgaccatgacctgcagcgccagcagctccgtgtcctacatgaactggtaccagcagaagcccggcaaggctcccaagaggtggatttacgactccagcaagctggcctctggtgtccccagcaggttctctggtagcggcagcggcacagactacaccctgaccatctcctccctgcagcccgacgatttcgccacctactattgccagcagtggtcccggaatccccctacctttggcggcggcaccaaggtggagatcaagaggagctccagc

SEQ ID NO: 222 - protein, 771 aa, Artificial Sequence; identical to SEQ ID NO: 218
  ROR233 Anti-ROR1 X anti-CD3 bispecific molecule